European Patent Application EP 4 495 246 A2, published January 22, 2025. Title: TECHNIQUES FOR GENERATING CELL-BASED THERAPEUTICS USING RECOMBINANT T CELL RECEPTOR GENES. Applicant: UNIVERSITY OF KANSAS. Application EP. The sequence listing filed with the application follows.

SEQUENCE LISTING (79 sequences)

SEQ ID NO: 1 - protein, 9 aa, Human immunodeficiency virus
RPQVPLRPM

SEQ ID NO: 2 - protein, 142 aa, Homo sapiens
PNIQNPDPAVYQLRDSKSSDKSVCLFTDFDSQTNVSQSKDSDVYITDKTVLDMRSMDFKSNSAVAWSNKSDFACANAFNNSIIPEDTFFPSPESSCDVKLVEKSFETDTNLNFQNLSVIGFRILLLKVAGFNLLMTLRLWSS

SEQ ID NO: 3 - protein, 177 aa, Homo sapiens
EDLNKVFPPEVAVFEPSEAEISHTQKATLVCLATGFFPDHVELSWWVNGKEVHSGVSTDPQPLKEQPALNDSRYCLSSRLRVSATFWQNPRNHFRCQVQFYGLSENDEWTQDRAKPVTQIVSAEAWGRADCGFTSVSYQQGVLSATILYEILLGKATLYAVLVSALVLMAMVKRKDF

SEQ ID NO: 4 - protein, 178 aa, Homo sapiens
DLKNVFPPEVAVFEPSEAEISHTQKATLVCLATGFYPDHVELSWWVNGKEVHSGVSTDPQPLKEQPALNDSRYCLSSRLRVSATFWQNPRNHFRCQVQFYGLSENDEWTQDRAKPVTQIVSAEAWGRADCGFTSESYQQGVLSATILYEILLGKATLYAVLVSALVLMAMVKRKDSRG

SEQ ID NO: 5 - protein, 173 aa, Homo sapiens
DKQLDADVSPKPTIFLPSIAETKLQKAGTYLCLLEKFFPDVIKIHWQEKKSNTILGSQEGNTMKTNDTYMKFSWLTVPEKSLDKEHRCIVRHENNKNGVDQEIIFPPIKTDVITMDPKDNCSKDANDTLLLQLTNTSAYYMYLLLLLKSVVYFAIITCCLLRRTAFCCNGEKS

SEQ ID NO: 6 - protein, 189 aa, Homo sapiens
DKQLDADVSPKPTIFLPSIAETKLQKAGTYLCLLEKFFPDIIKIHWQEKKSNTILGSQEGNTMKTNDTYMKFSWLTVPEESLDKEHRCIVRHENNKNGIDQEIIFPPIKTDVTTVDPKDSYSKDANDVITMDPKDNWSKDANDTLLLQLTNTSAYYMYLLLLLKSVVYFAIITCCLLGRTAFCCNGEKS

SEQ ID NO: 7 - protein, 153 aa, Homo sapiens
SQPHTKPSVFVMKNGTNVACLVKEFYPKDIRINLVSSKKITEFDPAIVISPSGKYNAVKLGKYEDSNSVTCSVQHDNKTVHSTDFEVKTDSTDHVKPKETENTKQPSKSCHKPKAIVHTEKVNMMSLTVLGLRMLFAKTVAVNFLLTAKLFFL

SEQ ID NO: 8 - protein, 15 aa, synthetic construct
  REGION 1..15: note = Description of Artificial Sequence: Synthetic peptide
GGGGSGGGGSGGGGS

SEQ ID NO: 9 - protein, 5 aa, synthetic construct
  REGION 1..5: note = Description of Artificial Sequence: Synthetic peptide
GGGGS

SEQ ID NO: 10 - protein, 14 aa, synthetic construct
  REGION 1..14: note = Description of Artificial Sequence: Synthetic peptide
GGGGSGGGGSGGGG

SEQ ID NO: 11 - protein, 13 aa, synthetic construct
  REGION 1..13: note = Description of Artificial Sequence: Synthetic peptide
EFGAGLVLGGQFM

SEQ ID NO: 12 - protein, 21 aa, synthetic construct
  REGION 1..21: note = Description of Artificial Sequence: Synthetic peptide
  REGION 1..3: note = MISC_FEATURE - This region may or may not be present
GSGEGRGSLLTCGDVEENPGP

SEQ ID NO: 13 - protein, 22 aa, synthetic construct
  REGION 1..22: note = Description of Artificial Sequence: Synthetic peptide
  REGION 1..3: note = MISC_FEATURE - This region may or may not be present
GSGATNFSLLKQAGDVEENPGP

SEQ ID NO: 14 - protein, 23 aa, synthetic construct
  REGION 1..23: note = Description of Artificial Sequence: Synthetic peptide
  REGION 1..3: note = MISC_FEATURE - This region may or may not be present
GSGQCTNYALLKLAGDVESNPGP

SEQ ID NO: 15 - protein, 24 aa, synthetic construct
  REGION 1..24: note = Description of Artificial Sequence: Synthetic peptide
  REGION 1..3: note = MISC_FEATURE - This region may or may not be present
GSGVKQTLNFDLLKLAGDVESNPG

SEQ ID NO: 16 - DNA, 355 bp, synthetic construct
  misc_feature 1..355: note = Description of Artificial Sequence: Synthetic polynucleotide
  source 1..355: mol_type = other DNA
tatgctagtacgtctctcaaggataagtaagtaatattaaggtacgggaggtattggacaggccgcaataaaatatctttattttcattacatctgtgtgttggttttttgtgtgaatcgatagtactaacatacgctctccatcaaaacaaaacgaaacaaaacaaactagcaaaataggctgtccccagtgcaagtgcaggtgccagaacatttctctggcctaactggccggtacctgagctctagtttcactttccctagtttcactttccctagtttcactttccctagtttcactttccctagtttcactttcccctcgaggatatcaagatctggcctcggcggccag

SEQ ID NO: 17 - DNA, 80 bp, Woodchuck hepatitis virus
  source 1..80: mol_type = other DNA
gccacggcggaactcatcgccgcctgccttgcccgctgctggacaggggctcggctgttgggcactgacaattccgtggt

SEQ ID NO: 18 - DNA, 592 bp, Woodchuck hepatitis virus
  source 1..592: mol_type = other DNA
aatcaacctctggattacaaaatttgtgaaagattgactggtattcttaactatgttgctccttttacgctatgtggatacgctgctttaatgcctttgtatcatgctattgcttcccgtatggctttcattttctcctccttgtataaatcctggttgctgtctctttatgaggagttgtggcccgttgtcaggcaacgtggcgtggtgtgcactgtgtttgctgacgcaacccccactggttggggcattgccaccacctgtcagctcctttccgggactttcgctttccccctccctattgccacggcggaactcatcgccgcctgccttgcccgctgctggacaggggctcggctgttgggcactgacaattccgtggtgttgtcggggaagctgacgtcctttccatggctgctcgcctgtgttgccacctggattctgcgcgggacgtccttctgctacgtcccttcggccctcaatccagcggaccttccttcccgcggcctgctgccggctctgcggcctcttccgcgtcttcgccttcgccctcagacgagtcggatctccctttgggccgcctccccgcctg

SEQ ID NO: 19 - DNA, 8904 bp, synthetic construct
  misc_feature 1..8904: note = Description of Artificial Sequence: Synthetic polynucleotide
  source 1..8904: mol_type = other DNA
tggaagggctaattcactcccaaagaagacaagatatccttgatctgtggatctaccacacacaaggctacttccctgattagcagaactacacaccagggccaggggtcagatatccactgacctttggatggtgctacaagctagtaccagttgagccagataaggtagaagaggccaataaaggagagaacaccagcttgttacaccctgtgagcctgcatgggatggatgacccggagagagaagtgttagagtggaggtttgacagccgcctagcatttcatcacgtggcccgagagctgcatccggagtacttcaagaactgctgatatcgagcttgctacaagggactttccgctggggactttccagggaggcgtggcctgggcgggactggggagtggcgagccctcagatcctgcatataagcagctgctttttgcctgtactgggtctctctggttagaccagatctgagcctgggagctctctggctaactagggaacccactgcttaagcctcaataaagcttgccttgagtgcttcaagtagtgtgtgcccgtctgttgtgtgactctggtaactagagatccctcagacccttttagtcagtgtggaaaatctctagcagtggcgcccgaacagggacttgaaagcgaaagggaaaccagaggagctctctcgacgcaggactcggcttgctgaagcgcgcacggcaagaggcgaggggcggcgactggtgagtacgccaaaaattttgactagcggaggctagaaggagagagatgggtgcgagagcgtcagtattaagcgggggagaattagatcgcgatgggaaaaaattcggttaaggccagggggaaagaaaaaatataaattaaaacatatagtatgggcaagcagggagctagaacgattcgcagttaatcctggcctgttagaaacatcagaaggctgtagacaaatactgggacagctacaaccatcccttcagacaggatcagaagaacttagatcattatataatacagtagcaaccctctattgtgtgcatcaaaggatagagataaaagacaccaaggaagctttagacaagatagaggaagagcaaaacaaaagtaagaccaccgcacagcaagcggccggccgctgatcttcagacctggaggaggagatatgagggacaattggagaagtgaattatataaatataaagtagtaaaaattgaaccattaggagtagcacccaccaaggcaaagagaagagtggtgcagagagaaaaaagagcagtgggaataggagctttgttccttgggttcttgggagcagcaggaagcactatgggcgcagcgtcaatgacgctgacggtacaggccagacaattattgtctggtatagtgcagcagcagaacaatttgctgagggctattgaggcgcaacagcatctgttgcaactcacagtctggggcatcaagcagctccaggcaagaatcctggctgtggaaagatacctaaaggatcaacagctcctggggatttggggttgctctggaaaactcatttgcaccactgctgtgccttggaatgctagttggagtaataaatctctggaacagatttggaatcacacgacctggatggagtgggacagagaaattaacaattacacaagcttaatacactccttaattgaagaatcgcaaaaccagcaagaaaagaatgaacaagaattattggaattagataaatgggcaagtttgtggaattggtttaacataacaaattggctgtggtatataaaattattcataatgatagtaggaggcttggtaggtttaagaatagtttttgctgtactttctatagtgaatagagttaggcagggatattcaccattatcgtttcagacccacctcccaaccccgaggggacccgacaggcccgaaggaatagaagaagaaggtggagagagagacagagacagatccattcgattagtgaacggatctcgacggtatcgcctttaaaagaaaaggggggattggggggtacagtgcaggggaaagaatagtagacataatagcaacagacatacaaactaaagaattacaaaaacaaattacaaaaattcaaaattttcgggtttattacagggacagcagagatccagtttatcgatgagtaattcatacaaaaggactcgcccctgccttggggaatcccagggaccgtcgttaaactcccactaacgtagaacccagagatcgctgcgttcccgccccctcacccgcccgctctcgtcatcactgaggtggagaagagcatgcgtgaggctccggtgcccgtcagtgggcagagcgcacatcgcccacagtccccgagaagttggggggaggggtcggcaattgaaccggtgcctagagaaggtggcgcggggtaaactgggaaagtgatgtcgtgtactggctccgcctttttcccgagggtgggggagaaccgtatataagtgcagtagtcgccgtgaacgttctttttcgcaacgggtttgccgccagaacacaggtaagtgccgtgtgtggttcccgcgggcctggcctctttacgggttatggcccttgcgtgccttgaattacttccacgcccctggctgcagtacgtgattcttgatcccgagcttcgggttggaagtgggtgggagagttcgaggccttgcgcttaaggagccccttcgcctcgtgcttgagttgaggcctggcttgggcgctggggccgccgcgtgcgaatctggtggcaccttcgcgcctgtctcgctgctttcgataagtctctagccatttaaaatttttgatgacctgctgcgacgctttttttctggcaagatagtcttgtaaatgcgggccaagatctgcacactggtatttcggtttttggggccgcgggcggcgacggggcccgtgcgtcccagcgcacatgttcggcgaggcggggcctgcgagcgcggccaccgagaatcggacgggggtagtctcaagctggccggcctgctctggtgcctggcctcgcgccgccgtgtatcgccccgccctgggcggcaaggctggcccggtcggcaccagttgcgtgagcggaaagatggccgcttcccggccctgctgcagggagctcaaaatggaggacgcggcgctcgggagagcgggcgggtgagtcacccacacaaaggaaaagggcctttccgtcctcagccgtcgcttcatgtgactccacggagtaccgggcgccgtccaggcacctcgattagttctcgagcttttggagtacgtcgtctttaggttggggggaggggttttatgcgatggagtttccccacactgagtgggtggagactgaagttaggccagcttggcacttgatgtaattctccttggaatttgccctttttgagtttggatcttggttcattctcaagcctcagacagtggttcaaagtttttttcttccatttcaggtgtcgtgaggatctatttccggtgaattcctcgagactagttctagagcggccgcggatcccgcccctctccctcccccccccctaacgttactggccgaagccgcttggaataaggccggtgtgcgtttgtctatatgttattttccaccatattgccgtcttttggcaatgtgagggcccggaaacctggccctgtcttcttgacgagcattcctaggggtctttcccctctcgccaaaggaatgcaaggtctgttgaatgtcgtgaaggaagcagttcctctggaagcttcttgaagacaaacaacgtctgtagcgaccctttgcaggcagcggaaccccccacctggcgacaggtgcctctgcggccaaaagccacgtgtataagatacacctgcaaaggcggcacaaccccagtgccacgttgtgagttggatagttgtggaaagagtcaaatggctcacctcaagcgtattcaacaaggggctgaaggatgcccagaaggtaccccattgtatgggatctgatctggggcctcggtgcacatgctttacatgtgtttagtcgaggttaaaaaacgtctaggccccccgaaccacggggacgtggttttcctttgaaaaacacgatgataatatggtgagcaagggcgaggaggataacatggccatcatcaaggagttcatgcgcttcaaggtgcacatggagggctccgtgaacggccacgagttcgagatcgagggcgagggcgagggccgcccctacgagggcacccagaccgccaagctgaaggtgaccaagggtggccccctgcccttcgcctgggacatcctgtcccctcagttcatgtacggctccaaggcctacgtgaagcaccccgccgacatccccgactacttgaagctgtccttccccgagggcttcaagtgggagcgcgtgatgaacttcgaggacggcggcgtggtgaccgtgacccaggactcctccctgcaggacggcgagttcatctacaaggtgaagctgcgcggcaccaacttcccctccgacggccccgtaatgcagaagaagaccatgggctgggaggcctcctccgagcggatgtaccccgaggacggcgccctgaagggcgagatcaagcagaggctgaagctgaaggacggcggccactacgacgctgaggtcaagaccacctacaaggccaagaagcccgtgcagctgcccggcgcctacaacgtcaacatcaagttggacatcacctcccacaacgaggactacaccatcgtggaacagtacgaacgcgccgagggccgccactccaccggcggcatggacgagctgtacaagtgaacgcgtctggaacaatcaacctctggattacaaaatttgtgaaagattgactggtattcttaactatgttgctccttttacgctatgtggatacgctgctttaatgcctttgtatcatgctattgcttcccgtatggctttcattttctcctccttgtataaatcctggttgctgtctctttatgaggagttgtggcccgttgtcaggcaacgtggcgtggtgtgcactgtgtttgctgacgcaacccccactggttggggcattgccaccacctgtcagctcctttccgggactttcgctttccccctccctattgccacggcggaactcatcgccgcctgccttgcccgctgctggacaggggctcggctgttgggcactgacaattccgtggtgttgtcggggaagctgacgtcctttccatggctgctcgcctgtgttgccacctggattctgcgcgggacgtccttctgctacgtcccttcggccctcaatccagcggaccttccttcccgcggcctgctgccggctctgcggcctcttccgcgtcttcgccttcgccctcagacgagtcggatctccctttgggccgcctccccgcctggaattaattctgcagtcgagacctagaaaaacatggagcaatcacaagtagcaatacagcagctaccaatgctgattgtgcctggctagaagcacaagaggaggaggaggtgggttttccagtcacacctcaggtacctttaagaccaatgacttacaaggcagctgtagatcttagccactttttaaaagaaaagaggggactggaagggctaattcactcccaacgaagacaagatatccttgatctgtggatctaccacacacaaggctacttccctgattagcagaactacacaccagggccaggggtcagatatccactgacctttggatggtgctacaagctagtaccagttgagccagataaggtagaagaggccaataaaggagagaacaccagcttgttacaccctgtgagcctgcatgggatggatgacccggagagagaagtgttagagtggaggtttgacagccgcctagcatttcatcacgtggcccgagagctgcatccggagtacttcaagaactgctgatatcgagcttgctacaagggactttccgctggggactttccagggaggcgtggcctgggcgggactggggagtggcgagccctcagatcctgcatataagcagctgctttttgcctgtactgggtctctctggttagaccagatctgagcctgggagctctctggctaactagggaacccactgcttaagcctcaataaagcttgccttgagtgcttcaagtagtgtgtgcccgtctgttgtgtgactctggtaactagagatccctcagacccttttagtcagtgtggaaaatctctagcagtagtagttcatgtcatcttattattcagtatttataacttgcaaagaaatgaatatcagagagtgagaggccttgacattgctagcgtttaccgtcgacctctagctagagcttggcgtaatcatggtcatagctgtttcctgtgtgaaattgttatccgctcacaattccacacaacatacgagccggaagcataaagtgtaaagcctggggtgcctaatgagtgagctaactcacattaattgcgttgcgctcactgcccgctttccagtcgggaaacctgtcgtgccagctgcattaatgaatcggccaacgcgcggggagaggcggtttgcgtattgggcgctcttccgcttcctcgctcactgactcgctgcgctcggtcgttcggctgcggcgagcggtatcagctcactcaaaggcggtaatacggttatccacagaatcaggggataacgcaggaaagaacatgtgagcaaaaggccagcaaaaggccaggaaccgtaaaaaggccgcgttgctggcgtttttccataggctccgcccccctgacgagcatcacaaaaatcgacgctcaagtcagaggtggcgaaacccgacaggactataaagataccaggcgtttccccctggaagctccctcgtgcgctctcctgttccgaccctgccgcttaccggatacctgtccgcctttctcccttcgggaagcgtggcgctttctcatagctcacgctgtaggtatctcagttcggtgtaggtcgttcgctccaagctgggctgtgtgcacgaaccccccgttcagcccgaccgctgcgccttatccggtaactatcgtcttgagtccaacccggtaagacacgacttatcgccactggcagcagccactggtaacaggattagcagagcgaggtatgtaggcggtgctacagagttcttgaagtggtggcctaactacggctacactagaagaacagtatttggtatctgcgctctgctgaagccagttaccttcggaaaaagagttggtagctcttgatccggcaaacaaaccaccgctggtagcggtggtttttttgtttgcaagcagcagattacgcgcagaaaaaaaggatctcaagaagatcctttgatcttttctacggggtctgacgctcagtggaacgaaaactcacgttaagggattttggtcatgagattatcaaaaaggatcttcacctagatccttttaaattaaaaatgaagttttaaatcaatctaaagtatatatgagtaaacttggtctgacagttaccaatgcttaatcagtgaggcacctatctcagcgatctgtctatttcgttcatccatagttgcctgactccccgtcgtgtagataactacgatacgggagggcttaccatctggccccagtgctgcaatgataccgcgagacccacgctcaccggctccagatttatcagcaataaaccagccagccggaagggccgagcgcagaagtggtcctgcaactttatccgcctccatccagtctattaattgttgccgggaagctagagtaagtagttcgccagttaatagtttgcgcaacgttgttgccattgctacaggcatcgtggtgtcacgctcgtcgtttggtatggcttcattcagctccggttcccaacgatcaaggcgagttacatgatcccccatgttgtgcaaaaaagcggttagctccttcggtcctccgatcgttgtcagaagtaagttggccgcagtgttatcactcatggttatggcagcactgcataattctcttactgtcatgccatccgtaagatgcttttctgtgactggtgagtactcaaccaagtcattctgagaatagtgtatgcggcgaccgagttgctcttgcccggcgtcaatacgggataataccgcgccacatagcagaactttaaaagtgctcatcattggaaaacgttcttcggggcgaaaactctcaaggatcttaccgctgttgagatccagttcgatgtaacccactcgtgcacccaactgatcttcagcatcttttactttcaccagcgtttctgggtgagcaaaaacaggaaggcaaaatgccgcaaaaaagggaataagggcgacacggaaatgttgaatactcatactcttcctttttcaatattattgaagcatttatcagggttattgtctcatgagcggatacatatttgaatgtatttagaaaaataaacaaataggggttccgcgcacatttccccgaaaagtgccacctgacgtcgacggatcgggagatcaacttgtttattgcagcttataatggttacaaataaagcaatagcatcacaaatttcacaaataaagcatttttttcactgcattctagttgtggtttgtccaaactcatcaatgtatcttatcatgtctggatcaactggataactcaagctaaccaaaatcatcccaaacttcccaccccataccctattaccactgccaattacctgtggtttcatttactctaaacctgtgattcctctgaattattttcattttaaagaaattgtatttgttaaatatgtactacaaacttagtagt

SEQ ID NO: 20 - DNA, 8904 bp, synthetic construct
  misc_feature 1..8904: note = Description of Artificial Sequence: Synthetic polynucleotide
  source 1..8904: mol_type = other DNA
tggaagggctaattcactcccaaagaagacaagatatccttgatctgtggatctaccacacacaaggctacttccctgattagcagaactacacaccagggccaggggtcagatatccactgacctttggatggtgctacaagctagtaccagttgagccagataaggtagaagaggccaataaaggagagaacaccagcttgttacaccctgtgagcctgcatgggatggatgacccggagagagaagtgttagagtggaggtttgacagccgcctagcatttcatcacgtggcccgagagctgcatccggagtacttcaagaactgctgatatcgagcttgctacaagggactttccgctggggactttccagggaggcgtggcctgggcgggactggggagtggcgagccctcagatcctgcatataagcagctgctttttgcctgtactgggtctctctggttagaccagatctgagcctgggagctctctggctaactagggaacccactgcttaagcctcaataaagcttgccttgagtgcttcaagtagtgtgtgcccgtctgttgtgtgactctggtaactagagatccctcagacccttttagtcagtgtggaaaatctctagcagtggcgcccgaacagggacttgaaagcgaaagggaaaccagaggagctctctcgacgcaggactcggcttgctgaagcgcgcacggcaagaggcgaggggcggcgactggtgagtacgccaaaaattttgactagcggaggctagaaggagagagatgggtgcgagagcgtcagtattaagcgggggagaattagatcgcgatgggaaaaaattcggttaaggccagggggaaagaaaaaatataaattaaaacatatagtatgggcaagcagggagctagaacgattcgcagttaatcctggcctgttagaaacatcagaaggctgtagacaaatactgggacagctacaaccatcccttcagacaggatcagaagaacttagatcattatataatacagtagcaaccctctattgtgtgcatcaaaggatagagataaaagacaccaaggaagctttagacaagatagaggaagagcaaaacaaaagtaagaccaccgcacagcaagcggccggccgctgatcttcagacctggaggaggagatatgagggacaattggagaagtgaattatataaatataaagtagtaaaaattgaaccattaggagtagcacccaccaaggcaaagagaagagtggtgcagagagaaaaaagagcagtgggaataggagctttgttccttgggttcttgggagcagcaggaagcactatgggcgcagcgtcaatgacgctgacggtacaggccagacaattattgtctggtatagtgcagcagcagaacaatttgctgagggctattgaggcgcaacagcatctgttgcaactcacagtctggggcatcaagcagctccaggcaagaatcctggctgtggaaagatacctaaaggatcaacagctcctggggatttggggttgctctggaaaactcatttgcaccactgctgtgccttggaatgctagttggagtaataaatctctggaacagatttggaatcacacgacctggatggagtgggacagagaaattaacaattacacaagcttaatacactccttaattgaagaatcgcaaaaccagcaagaaaagaatgaacaagaattattggaattagataaatgggcaagtttgtggaattggtttaacataacaaattggctgtggtatataaaattattcataatgatagtaggaggcttggtaggtttaagaatagtttttgctgtactttctatagtgaatagagttaggcagggatattcaccattatcgtttcagacccacctcccaaccccgaggggacccgacaggcccgaaggaatagaagaagaaggtggagagagagacagagacagatccattcgattagtgaacggatctcgacggtatcgcctttaaaagaaaaggggggattggggggtacagtgcaggggaaagaatagtagacataatagcaacagacatacaaactaaagaattacaaaaacaaattacaaaaattcaaaattttcgggtttattacagggacagcagagatccagtttatcgatgagtaattcatacaaaaggactcgcccctgccttggggaatcccagggaccgtcgttaaactcccactaacgtagaacccagagatcgctgcgttcccgccccctcacccgcccgctctcgtcatcactgaggtggagaagagcaagcgtgaggctccggtgcccgtcagtgggcagagcgcacatcgcccacagtccccgagaagttggggggaggggtcggcaattgatccggagcctagagaaggtggcgcggggtaaactgggaaagtgatgtcgtgtactggctccgcctttttcccgagggtgggggagaaccgtatataagtgcagtagtcgccgtgaacgttctttttcgcaacgggtttgccgccagaacacaggtaagtgccgtgtgtggttcccgcgggcctggcctctttacgggttatggcccttgcgtgccttgaattacttccacgcccctggctgcagtacgtgattcttgatcccgagcttcgggttggaagtgggtgggagagttcgaggccttgcgcttaaggagccccttcgcctcgtgcttgagttgaggcctggcttgggcgctggggccgccgcgtgcgaatctggtggcaccttcgcgcctgtctcgctgctttcgataagtctctagccatttaaaatttttgatgacctgctgcgacgctttttttctggcaagatagtcttgtaaatgcgggccaagatctgcacactggtatttcggtttttggggccgcgggcggcgacggggcccgtgcgtcccagcgcacatgttcggcgaggcggggcctgcgagcgcggccaccgagaatcggacgggggtagtctcaagctggccggcctgctctggtgcctggcctcgcgccgccgtgtatcgccccgccctgggcggcaaggctggcccggtcggcaccagttgcgtgagcggaaagatggccgcttcccggccctgctgcagggagctcaaaatggaggacgcggcgctcgggagagcgggcgggtgagtcacccacacaaaggaaaagggcctttccgtcctcagccgtcgcttcatgtgactccacggagtaccgggcgccgtccaggcacctcgattagttctcgagcttttggagtacgtcgtctttaggttggggggaggggttttatgcgatggagtttccccacactgagtgggtggagactgaagttaggccagcttggcacttgatgtaattctccttggaatttgccctttttgagtttggatcttggttcattctcaagcctcagacagtggttcaaagtttttttcttccatttcaggtgtcgtgaggatctatttccggtgaattcctcgagactagttctagagcggccgcggatcccgcccctctccctcccccccccctaacgttactggccgaagccgcttggaataaggccggtgtgcgtttgtctatatgttattttccaccatattgccgtcttttggcaatgtgagggcccggaaacctggccctgtcttcttgacgagcattcctaggggtctttcccctctcgccaaaggaatgcaaggtctgttgaatgtcgtgaaggaagcagttcctctggaagcttcttgaagacaaacaacgtctgtagcgaccctttgcaggcagcggaaccccccacctggcgacaggtgcctctgcggccaaaagccacgtgtataagatacacctgcaaaggcggcacaaccccagtgccacgttgtgagttggatagttgtggaaagagtcaaatggctcacctcaagcgtattcaacaaggggctgaaggatgcccagaaggtaccccattgtatgggatctgatctggggcctcggtgcacatgctttacatgtgtttagtcgaggttaaaaaacgtctaggccccccgaaccacggggacgtggttttcctttgaaaaacacgatgataatatggtgagcaagggcgaggaggataacatggccatcatcaaggagttcatgcgcttcaaggtgcacatggagggctccgtgaacggccacgagttcgagatcgagggcgagggcgagggccgcccctacgagggcacccagaccgccaagctgaaggtgaccaagggtggccccctgcccttcgcctgggacatcctgtcccctcagttcatgtacggctccaaggcctacgtgaagcaccccgccgacatccccgactacttgaagctgtccttccccgagggcttcaagtgggagcgcgtgatgaacttcgaggacggcggcgtggtgaccgtgacccaggactcctccctgcaggacggcgagttcatctacaaggtgaagctgcgcggcaccaacttcccctccgacggccccgtaatgcagaagaagaccatgggctgggaggcctcctccgagcggatgtaccccgaggacggcgccctgaagggcgagatcaagcagaggctgaagctgaaggacggcggccactacgacgctgaggtcaagaccacctacaaggccaagaagcccgtgcagctgcccggcgcctacaacgtcaacatcaagttggacatcacctcccacaacgaggactacaccatcgtggaacagtacgaacgcgccgagggccgccactccaccggcggcatggacgagctgtacaagtgaacccgtctggaacaatcaacctctggattacaaaatttgtgaaagattgactggtattcttaactatgttgctccttttacgctatgtggatacgctgctttaatgcctttgtatcatgctattgcttcccgtatggctttcattttctcctccttgtataaatcctggttgctgtctctttatgaggagttgtggcccgttgtcaggcaacgtggcgtggtgtgcactgtgtttgctgacgcaacccccactggttggggcattgccaccacctgtcagctcctttccgggactttcgctttccccctccctattgccacggcggaactcatcgccgcctgccttgcccgctgctggacaggggctcggctgttgggcactgacaattccgtggtgttgtcggggaagctgacgtcctttccatggctgctcgcctgtgttgccacctggattctgcgcgggacgtccttctgctacgtcccttcggccctcaatccagcggaccttccttcccgcggcctgctgccggctctgcggcctcttccgcgtcttcgccttcgccctcagacgagtcggatctccctttgggccgcctccccgcctggaattaattctgcagtcgagacctagaaaaacatggagcaatcacaagtagcaatacagcagctaccaatgctgattgtgcctggctagaagcacaagaggaggaggaggtgggttttccagtcacacctcaggtacctttaagaccaatgacttacaaggcagctgtagatcttagccactttttaaaagaaaagaggggactggaagggctaattcactcccaacgaagacaagatatccttgatctgtggatctaccacacacaaggctacttccctgattagcagaactacacaccagggccaggggtcagatatccactgacctttggatggtgctacaagctagtaccagttgagccagataaggtagaagaggccaataaaggagagaacaccagcttgttacaccctgtgagcctgcatgggatggatgacccggagagagaagtgttagagtggaggtttgacagccgcctagcatttcatcacgtggcccgagagctgcatccggagtacttcaagaactgctgatatcgagcttgctacaagggactttccgctggggactttccagggaggcgtggcctgggcgggactggggagtggcgagccctcagatcctgcatataagcagctgctttttgcctgtactgggtctctctggttagaccagatctgagcctgggagctctctggctaactagggaacccactgcttaagcctcaataaagcttgccttgagtgcttcaagtagtgtgtgcccgtctgttgtgtgactctggtaactagagatccctcagacccttttagtcagtgtggaaaatctctagcagtagtagttcatgtcatcttattattcagtatttataacttgcaaagaaatgaatatcagagagtgagaggccttgacattgcttgcgtttaccgtcgacctctagctagagcttggcgtaatcatggtcatagctgtttcctgtgtgaaattgttatccgctcacaattccacacaacatacgagccggaagcataaagtgtaaagcctggggtgcctaatgagtgagctaactcacattaattgcgttgcgctcactgcccgctttccagtcgggaaacctgtcgtgccagctgcattaatgaatcggccaacgcgcggggagaggcggtttgcgtattgggcgctcttccgcttcctcgctcactgactcgctgcgctcggtcgttcggctgcggcgagcggtatcagctcactcaaaggcggtaatacggttatccacagaatcaggggataacgcaggaaagaacatgtgagcaaaaggccagcaaaaggccaggaaccgtaaaaaggccgcgttgctggcgtttttccataggctccgcccccctgacgagcatcacaaaaatcgacgctcaagtcagaggtggcgaaacccgacaggactataaagataccaggcgtttccccctggaagctccctcgtgcgctctcctgttccgaccctgccgcttaccggatacctgtccgcctttctcccttcgggaagcgtggcgctttctcatagctcacgctgtaggtatctcagttcggtgtaggtcgttcgctccaagctgggctgtgtgcacgaaccccccgttcagcccgaccgctgcgccttatccggtaactatcgtcttgagtccaacccggtaagacacgacttatcgccactggcagcagccactggtaacaggattagcagagcgaggtatgtaggcggtgctacagagttcttgaagtggtggcctaactacggctacactagaagaacagtatttggtatctgcgctctgctgaagccagttaccttcggaaaaagagttggtagctcttgatccggcaaacaaaccaccgctggtagcggtggtttttttgtttgcaagcagcagattacgcgcagaaaaaaaggatctcaagaagatcctttgatcttttctacggggtctgacgctcagtggaacgaaaactcacgttaagggattttggtcatgagattatcaaaaaggatcttcacctagatccttttaaattaaaaatgaagttttaaatcaatctaaagtatatatgagtaaacttggtctgacagttaccaatgcttaatcagtgaggcacctatctcagcgatctgtctatttcgttcatccatagttgcctgactccccgtcgtgtagataactacgatacgggagggcttaccatctggccccagtgctgcaatgataccgcgagacccacgctcaccggctccagatttatcagcaataaaccagccagccggaagggccgagcgcagaagtggtcctgcaactttatccgcctccatccagtctattaattgttgccgggaagctagagtaagtagttcgccagttaatagtttgcgcaacgttgttgccattgctacaggcatcgtggtgtcacgctcgtcgtttggtatggcttcattcagctccggttcccaacgatcaaggcgagttacatgatcccccatgttgtgcaaaaaagcggttagctccttcggtcctccgatcgttgtcagaagtaagttggccgcagtgttatcactcatggttatggcagcactgcataattctcttactgtcatgccatccgtaagatgcttttctgtgactggtgagtactcaaccaagtcattctgagaatagtgtatgcggcgaccgagttgctcttgcccggcgtcaatacgggataataccgcgccacatagcagaactttaaaagtgctcatcattggaaaacgttcttcggggcgaaaactctcaaggatcttaccgctgttgagatccagttcgatgtaacccactcgtgcacccaactgatcttcagcatcttttactttcaccagcgtttctgggtgagcaaaaacaggaaggcaaaatgccgcaaaaaagggaataagggcgacacggaaatgttgaatactcatactcttcctttttcaatattattgaagcatttatcagggttattgtctcatgagcggatacatatttgaatgtatttagaaaaataaacaaataggggttccgcgcacatttccccgaaaagtgccacctgacgtcgacggatcgggagatcaacttgtttattgcagcttataatggttacaaataaagcaatagcatcacaaatttcacaaataaagcatttttttcactgcattctagttgtggtttgtccaaactcatcaatgtatcttatcatgtctggatcaactggataactcaagctaaccaaaatcatcccaaacttcccaccccataccctattaccactgccaattacctgtggtttcatttactctaaacctgtgattcctctgaattattttcattttaaagaaattgtatttgttaaatatgtactacaaacttagtagt

SEQ ID NO: 21 - DNA, 12037 bp, synthetic construct
  misc_feature 1..12037: note = Description of Artificial Sequence: Synthetic polynucleotide
  source 1..12037: mol_type = other DNA
tggaagggctaattcactcccaaagaagacaagatatccttgatctgtggatctaccacacacaaggctacttccctgattagcagaactacacaccagggccaggggtcagatatccactgacctttggatggtgctacaagctagtaccagttgagccagataaggtagaagaggccaataaaggagagaacaccagcttgttacaccctgtgagcctgcatgggatggatgacccggagagagaagtgttagagtggaggtttgacagccgcctagcatttcatcacgtggcccgagagctgcatccggagtacttcaagaactgctgatatcgagcttgctacaagggactttccgctggggactttccagggaggcgtggcctgggcgggactggggagtggcgagccctcagatcctgcatataagcagctgctttttgcctgtactgggtctctctggttagaccagatctgagcctgggagctctctggctaactagggaacccactgcttaagcctcaataaagcttgccttgagtgcttcaagtagtgtgtgcccgtctgttgtgtgactctggtaactagagatccctcagacccttttagtcagtgtggaaaatctctagcagtggcgcccgaacagggacttgaaagcgaaagggaaaccagaggagctctctcgacgcaggactcggcttgctgaagcgcgcacggcaagaggcgaggggcggcgactggtgagtacgccaaaaattttgactagcggaggctagaaggagagagatgggtgcgagagcgtcagtattaagcgggggagaattagatcgcgatgggaaaaaattcggttaaggccagggggaaagaaaaaatataaattaaaacatatagtatgggcaagcagggagctagaacgattcgcagttaatcctggcctgttagaaacatcagaaggctgtagacaaatactgggacagctacaaccatcccttcagacaggatcagaagaacttagatcattatataatacagtagcaaccctctattgtgtgcatcaaaggatagagataaaagacaccaaggaagctttagacaagatagaggaagagcaaaacaaaagtaagaccaccgcacagcaagcggccggccgctgatcttcagacctggaggaggagatatgagggacaattggagaagtgaattatataaatataaagtagtaaaaattgaaccattaggagtagcacccaccaaggcaaagagaagagtggtgcagagagaaaaaagagcagtgggaataggagctttgttccttgggttcttgggagcagcaggaagcactatgggcgcagcgtcaatgacgctgacggtacaggccagacaattattgtctggtatagtgcagcagcagaacaatttgctgagggctattgaggcgcaacagcatctgttgcaactcacagtctggggcatcaagcagctccaggcaagaatcctggctgtggaaagatacctaaaggatcaacagctcctggggatttggggttgctctggaaaactcatttgcaccactgctgtgccttggaatgctagttggagtaataaatctctggaacagatttggaatcacacgacctggatggagtgggacagagaaattaacaattacacaagcttaatacactccttaattgaagaatcgcaaaaccagcaagaaaagaatgaacaagaattattggaattagataaatgggcaagtttgtggaattggtttaacataacaaattggctgtggtatataaaattattcataatgatagtaggaggcttggtaggtttaagaatagtttttgctgtactttctatagtgaatagagttaggcagggatattcaccattatcgtttcagacccacctcccaaccccgaggggacccgacaggcccgaaggaatagaagaagaaggtggagagagagacagagacagatccattcgattagtgaacggatctcgacggtatcgcctttaaaagaaaaggggggattggggggtacagtgcaggggaaagaatagtagacataatagcaacagacatacaaactaaagaattacaaaaacaaattacaaaaattcaaaattttcgggtttattacagggacagcagagatccagtttatcgataagcttgggagttccgcgttacataacttacggtaaatggcccgcctggctgaccgcccaacgacccccgcccattgacgtcaataatgacgtatgttcccatagtaacgccaatagggactttccattgacgtcaatgggtggagtatttacggtaaactgcccacttggcagtacatcaagtgtatcatatgccaagtacgccccctattgacgtcaatgacggtaaatggcccgcctggcattatgcccagtacatgaccttatgggactttcctacttggcagtacatctacgtattagtcatcgctattaccatggtgatgcggttttggcagtacatcaatgggcgtggatagcggtttgactcacggggatttccaagtctccaccccattgacgtcaatgggagtttgttttggcaccaaaatcaacgggactttccaaaatgtcgtaacaactccgccccattgacgcaaatgggcggtaggcgtgtacggtgggaggtctatataagcagagctcgtttagtgaaccgtcagatcgcctggagacgccatccacgctgttttgacctccatagaagacaccgactctactagaggatctatttccggtgaattcgccaccatgagcctcgggctcctgtgctgtggggccttttctctcctgtgggcaggaccggtggaagctgacatctaccagaccccaagataccttgttatagggacaggaaagaagatcactctggaatgttctcaaaccatgggccatgacaaaatgtactggtatcaacaagatccaggaatggaactacacctcatccactattcctatggagttaattccacagagaagggagatctttcctctgagtcaacagtctccagaataaggacggagcattttcccctgaccctggagtctgccaggccctcacatacctctcagtacctctgtgccagcagtcggacgcccaacattcagtacttcggcgccgggacccggctctcagtgctggaggacctgaaaaacgtgttcccacccgaactagtcgtgtttgagccatcagaagcagagatctcccacacccaaaaggccacactggtgtgcctggccacaggcttctaccccgaccacgtggagctgagctggtgggtgaatgggaaggaggtgcacagtggggtcagcacagacccgcagcccctcaaggagcagcccgccctcaatgactccagatactgcctgagcagccgcctgagggtctcggccaccttctggcagaacccccgcaaccacttccgctgtcaagtccagttctacgggctctcggagaatgacgagtggacccaggatagggccaaacctgtcacccagatcgtcagcgccgaggcctggggtagagcagactgtggcttcacctccgagtcttaccagcaaggggtcctgtctgccaccatcctctatgagatcttgctagggaaggccaccttgtatgccgtgctggtcagtgccctcgtgctgatggccatggtcaagagaaaggattccagaggcgggagcggagccacgaacttctctctgttaaagcaagcaggagacgtggaagaaaaccccggtcctatgacacgagttagcttgctgtgggcagtcgtggtctccacctgtctcgagtccggcatgggtcaacagctgaatcagagtcctcaatctatgtttatccaggaaggagaagatgtctccatgaactgcacttcttcaagcatatttaacacctggctatggtacaagcaggaacctggggaaggtcctgtcctcttgatagccttatataaggctggtgaattgacctcaaatggaagactgactgctcagtttggtataaccagaaaggacagcttcctgaatatctcagcatccatacctagtgatgtaggcatctacttctgtgctggcacataccagaaagttacctttggaactggaacaaagctccaagtcatcccaaatatccagaaccctgaccctgccgtgtaccagctgagagactctaaatccagtgacaagtctgtctgcctattcaccgattttgattctcaaacaaatgtgtcacaaagtaaggattctgatgtgtatatcacagacaaaactgtgctagacatgaggtctatggacttcaagagcaacagtgctgtggcctggagcaacaaatctgactttgcatgcgcaaacgccttcaacaacagcattattccagaagacaccttcttccccagcccagaaagttcctgtgatgtcaagctggtcgagaaaagctttgaaacagatacgaacctaaactttcaaaacctgtcagtgattgggttccgaatcctcctcctgaaagtggccgggtttaatctgctcatgacgctgcggctgtggtccagctgactcgagggatcccgcccctctccctcccccccccctaacgttactggccgaagccgcttggaataaggccggtgtgcgtttgtctatatgttattttccaccatattgccgtcttttggcaatgtgagggcccggaaacctggccctgtcttcttgacgagcattcctaggggtctttcccctctcgccaaaggaatgcaaggtctgttgaatgtcgtgaaggaagcagttcctctggaagcttcttgaagacaaacaacgtctgtagcgaccctttgcaggcagcggaaccccccacctggcgacaggtgcctctgcggccaaaagccacgtgtataagatacacctgcaaaggcggcacaaccccagtgccacgttgtgagttggatagttgtggaaagagtcaaatggctcacctcaagcgtattcaacaaggggctgaaggatgcccagaaggtaccccattgtatgggatctgatctggggcctcggtgcacatgctttacatgtgtttagtcgaggttaaaaaacgtctaggccccccgaaccacggggacgtggttttcctttgaaaaacacgatgataatatggtgagcaagggcgaggaggataacatggccatcatcaaggagttcatgcgcttcaaggtgcacatggagggctccgtgaacggccacgagttcgagatcgagggcgagggcgagggccgcccctacgagggcacccagaccgccaagctgaaggtgaccaagggtggccccctgcccttcgcctgggacatcctgtcccctcagttcatgtacggctccaaggcctacgtgaagcaccccgccgacatccccgactacttgaagctgtccttccccgagggcttcaagtgggagcgcgtgatgaacttcgaggacggcggcgtggtgaccgtgacccaggactcctccctgcaggacggcgagttcatctacaaggtgaagctgcgcggcaccaacttcccctccgacggccccgtaatgcagaagaagaccatgggctgggaggcctcctccgagcggatgtaccccgaggacggcgccctgaagggcgagatcaagcagaggctgaagctgaaggacggcggccactacgacgctgaggtcaagaccacctacaaggccaagaagcccgtgcagctgcccggcgcctacaacgtcaacatcaagttggacatcacctcccacaacgaggactacaccatcgtggaacagtacgaacgcgccgagggccgccactccaccggcggcatggacgagctgtacaagtgaacgcgtctggaacaagctttttccccgtatccccccaggtgtctgcaggctcaaagagcagcgagaagcgttcagaggaaagcgatcccgtgccaccttccccgtgcccgggctgtccccgcacgctgccggctcggggatgcggggggagcgccggaccggagcggagccccgggcggctcgctgctgccccctagcgggggagggacgtaattacatccctgggggctttgggggggggctgtccccgtgagctcttactccctatcagtgatagagaacgtatgaagagtttactccctatcagtgatagagaacgtatgcagactttactccctatcagtgatagagaacgtataaggagtttactccctatcagtgatagagaacgtatgaccagtttactccctatcagtgatagagaacgtatctacagtttactccctatcagtgatagagaacgtatatccagtttactccctatcagtgatagagaacgtatgtcgaggtaggcgtgtacggtgggcgcctataaaagcagagctcgtttagtgaaccgtcagatcgcctggagcaattccacaacacttttgtcttatacttatgctcgagggagtgcaggtggagactatctccccaggagacgggcgcaccttccccaagcgcggccagacctgcgtggtgcactacaccgggatgcttgaagatggaaagaaagttgattcctcccgggacagaaacaagccctttaagtttatgctaggcaagcaggaggtgatccgaggctgggaagaaggggttgcccagatgagtgtgggtcagagagccaaactgactatatctccagattatgcctatggtgccactgggcacccaggcatcatcccaccacatgccactctcgtcttcgatgtggagcttctaaaactggaatctggcggtggatccggagtcgacggatttggtgatgtcggtgctcttgagagtttgaggggaaatgcagatttggcttacatcctgagcatggagccctgtggccactgcctcattatcaacaatgtgaacttctgccgtgagtccgggctccgcacccgcactggctccaacatcgactgtgagaagttgcggcgtcgcttctcctcgctgcatttcatggtggaggtgaagggcgacctgactgccaagaaaatggtgctggctttgctggagctggcgcggcaggaccacggtgctctggactgctgcgtggtggtcattctctctcacggctgtcaggccagccacctgcagttcccaggggctgtctacggcacagatggatgccctgtgtcggtcgagaagattgtgaacatcttcaatgggaccagctgccccagcctgggagggaagcccaagctctttttcatccaggcctgtggtggggagcagaaagaccatgggtttgaggtggcctccacttcccctgaagacgagtcccctggcagtaaccccgagccagatgccaccccgttccaggaaggtttgaggaccttcgaccagctggacgccatatctagtttgcccacacccagtgacatctttgtgtcctactctactttcccaggttttgtttcctggagggaccccaagagtggctcctggtacgttgagaccctggacgacatctttgagcagtgggctcactctgaagacctgcagtccctcctgcttagggtcgctaatgctgtttcggtgaaagggatttataaacagatgcctggttgctttaatttcctccggaaaaaacttttctttaaaacatcagtcgactatccgtacgacgtaccagactacgcactcgactaaaagctttttccccgtatccccccaggtgtctgcaggctcaaagagcagcgagaagcgttcagaggaaagcgatcccgtgccaccttccccgtgcccgggctgtccccgcacgctgccggctcggggatgcggggggagcgccggaccggagcggagccccgggcggctcgctgctgccccctagcgggggagggacgtaattacatccctgggggctttgggagggggctgtccccgtgagctcaatcaacctctggattacaaaatttgtgaaagattgactggtattcttaactatgttgctccttttacgctatgtggatacgctgctttaatgcctttgtatcatgctattgcttcccgtatggctttcattttctcctccttgtataaatcctggttgctgtctctttatgaggagttgtggcccgttgtcaggcaacgtggcgtggtgtgcactgtgtttgctgacgcaacccccactggttggggcattgccaccacctgtcagctcctttccgggactttcgctttccccctccctattgccacggcggaactcatcgccgcctgccttgcccgctgctggacaggggctcggctgttgggcactgacaattccgtggtgttgtcggggaagctgacgtcctttccatggctgctcgcctgtgttgccacctggattctgcgcgggacgtccttctgctacgtcccttcggccctcaatccagcggaccttccttcccgcggcctgctgccggctctgcggcctcttccgcgtcttcgccttcgccctcagacgagtcggatctccctttgggccgcctccccgcctggaattaattctgcagtcgagacctagaaaaacatggagcaatcacaagtagcaatacagcagctaccaatgctgattgtgcctggctagaagcacaagaggaggaggaggtgggttttccagtcacacctcaggtacctttaagaccaatgacttacaaggcagctgtagatcttagccactttttaaaagaaaagaggggactggaagggctaattcactcccaacgaagacaagatatccttgatctgtggatctaccacacacaaggctacttccctgattagcagaactacacaccagggccaggggtcagatatccactgacctttggatggtgctacaagctagtaccagttgagccagataaggtagaagaggccaataaaggagagaacaccagcttgttacaccctgtgagcctgcatgggatggatgacccggagagagaagtgttagagtggaggtttgacagccgcctagcatttcatcacgtggcccgagagctgcatccggagtacttcaagaactgctgatatcgagcttgctacaagggactttccgctggggactttccagggaggcgtggcctgggcgggactggggagtggcgagccctcagatcctgcatataagcagctgctttttgcctgtactgggtctctctggttagaccagatctgagcctgggagctctctggctaactagggaacccactgcttaagcctcaataaagcttgccttgagtgcttcaagtagtgtgtgcccgtctgttgtgtgactctggtaactagagatccctcagacccttttagtcagtgtggaaaatctctagcagtagtagttcatgtcatcttattattcagtatttataacttgcaaagaaatgaatatcagagagtgagaggccttgacattgctagcgtttaccgtcgacctctagctagagcttggcgtaatcatggtcatagctgtttcctgtgtgaaattgttatccgctcacaattccacacaacatacgagccggaagcataaagtgtaaagcctggggtgcctaatgagtgagctaactcacattaattgcgttgcgctcactgcccgctttccagtcgggaaacctgtcgtgccagctgcattaatgaatcggccaacgcgcggggagaggcggtttgcgtattgggcgctcttccgcttcctcgctcactgactcgctgcgctcggtcgttcggctgcggcgagcggtatcagctcactcaaaggcggtaatacggttatccacagaatcaggggataacgcaggaaagaacatgtgagcaaaaggccagcaaaaggccaggaaccgtaaaaaggccgcgttgctggcgtttttccataggctccgcccccctgacgagcatcacaaaaatcgacgctcaagtcagaggtggcgaaacccgacaggactataaagataccaggcgtttccccctggaagctccctcgtgcgctctcctgttccgaccctgccgcttaccggatacctgtccgcctttctcccttcgggaagcgtggcgctttctcatagctcacgctgtaggtatctcagttcggtgtaggtcgttcgctccaagctgggctgtgtgcacgaaccccccgttcagcccgaccgctgcgccttatccggtaactatcgtcttgagtccaacccggtaagacacgacttatcgccactggcagcagccactggtaacaggattagcagagcgaggtatgtaggcggtgctacagagttcttgaagtggtggcctaactacggctacactagaagaacagtatttggtatctgcgctctgctgaagccagttaccttcggaaaaagagttggtagctcttgatccggcaaacaaaccaccgctggtagcggtggtttttttgtttgcaagcagcagattacgcgcagaaaaaaaggatctcaagaagatcctttgatcttttctacggggtctgacgctcagtggaacgaaaactcacgttaagggattttggtcatgagattatcaaaaaggatcttcacctagatccttttaaattaaaaatgaagttttaaatcaatctaaagtatatatgagtaaacttggtctgacagttaccaatgcttaatcagtgaggcacctatctcagcgatctgtctatttcgttcatccatagttgcctgactccccgtcgtgtagataactacgatacgggagggcttaccatctggccccagtgctgcaatgataccgcgagacccacgctcaccggctccagatttatcagcaataaaccagccagccggaagggccgagcgcagaagtggtcctgcaactttatccgcctccatccagtctattaattgttgccgggaagctagagtaagtagttcgccagttaatagtttgcgcaacgttgttgccattgctacaggcatcgtggtgtcacgctcgtcgtttggtatggcttcattcagctccggttcccaacgatcaaggcgagttacatgatcccccatgttgtgcaaaaaagcggttagctccttcggtcctccgatcgttgtcagaagtaagttggccgcagtgttatcactcatggttatggcagcactgcataattctcttactgtcatgccatccgtaagatgcttttctgtgactggtgagtactcaaccaagtcattctgagaatagtgtatgcggcgaccgagttgctcttgcccggcgtcaatacgggataataccgcgccacatagcagaactttaaaagtgctcatcattggaaaacgttcttcggggcgaaaactctcaaggatcttaccgctgttgagatccagttcgatgtaacccactcgtgcacccaactgatcttcagcatcttttactttcaccagcgtttctgggtgagcaaaaacaggaaggcaaaatgccgcaaaaaagggaataagggcgacacggaaatgttgaatactcatactcttcctttttcaatattattgaagcatttatcagggttattgtctcatgagcggatacatatttgaatgtatttagaaaaataaacaaataggggttccgcgcacatttccccgaaaagtgccacctgacgtcgacggatcgggagatcaacttgtttattgcagcttataatggttacaaataaagcaatagcatcacaaatttcacaaataaagcatttttttcactgcattctagttgtggtttgtccaaactcatcaatgtatcttatcatgtctggatcaactggataactcaagctaaccaaaatcatcccaaacttcccaccccataccctattaccactgccaattacctgtggtttcatttactctaaacctgtgattcctctgaattattttcattttaaagaaattgtatttgttaaatatgtactacaaacttagtagt

SEQ ID NO: 22 - DNA, 12031 bp, synthetic construct
  misc_feature 1..12031: note = Description of Artificial Sequence: Synthetic polynucleotide
  source 1..12031: mol_type = other DNA
tggaagggctaattcactcccaaagaagacaagatatccttgatctgtggatctaccacacacaaggctacttccctgattagcagaactacacaccagggccaggggtcagatatccactgacctttggatggtgctacaagctagtaccagttgagccagataaggtagaagaggccaataaaggagagaacaccagcttgttacaccctgtgagcctgcatgggatggatgacccggagagagaagtgttagagtggaggtttgacagccgcctagcatttcatcacgtggcccgagagctgcatccggagtacttcaagaactgctgatatcgagcttgctacaagggactttccgctggggactttccagggaggcgtggcctgggcgggactggggagtggcgagccctcagatcctgcatataagcagctgctttttgcctgtactgggtctctctggttagaccagatctgagcctgggagctctctggctaactagggaacccactgcttaagcctcaataaagcttgccttgagtgcttcaagtagtgtgtgcccgtctgttgtgtgactctggtaactagagatccctcagacccttttagtcagtgtggaaaatctctagcagtggcgcccgaacagggacttgaaagcgaaagggaaaccagaggagctctctcgacgcaggactcggcttgctgaagcgcgcacggcaagaggcgaggggcggcgactggtgagtacgccaaaaattttgactagcggaggctagaaggagagagatgggtgcgagagcgtcagtattaagcgggggagaattagatcgcgatgggaaaaaattcggttaaggccagggggaaagaaaaaatataaattaaaacatatagtatgggcaagcagggagctagaacgattcgcagttaatcctggcctgttagaaacatcagaaggctgtagacaaatactgggacagctacaaccatcccttcagacaggatcagaagaacttagatcattatataatacagtagcaaccctctattgtgtgcatcaaaggatagagataaaagacaccaaggaagctttagacaagatagaggaagagcaaaacaaaagtaagaccaccgcacagcaagcggccggccgctgatcttcagacctggaggaggagatatgagggacaattggagaagtgaattatataaatataaagtagtaaaaattgaaccattaggagtagcacccaccaaggcaaagagaagagtggtgcagagagaaaaaagagcagtgggaataggagctttgttccttgggttcttgggagcagcaggaagcactatgggcgcagcgtcaatgacgctgacggtacaggccagacaattattgtctggtatagtgcagcagcagaacaatttgctgagggctattgaggcgcaacagcatctgttgcaactcacagtctggggcatcaagcagctccaggcaagaatcctggctgtggaaagatacctaaaggatcaacagctcctggggatttggggttgctctggaaaactcatttgcaccactgctgtgccttggaatgctagttggagtaataaatctctggaacagatttggaatcacacgacctggatggagtgggacagagaaattaacaattacacaagcttaatacactccttaattgaagaatcgcaaaaccagcaagaaaagaatgaacaagaattattggaattagataaatgggcaagtttgtggaattggtttaacataacaaattggctgtggtatataaaattattcataatgatagtaggaggcttggtaggtttaagaatagtttttgctgtactttctatagtgaatagagttaggcagggatattcaccattatcgtttcagacccacctcccaaccccgaggggacccgacaggcccgaaggaatagaagaagaaggtggagagagagacagagacagatccattcgattagtgaacggatctcgacggtatcgcctttaaaagaaaaggggggattggggggtacagtgcaggggaaagaatagtagacataatagcaacagacatacaaactaaagaattacaaaaacaaattacaaaaattcaaaattttcgggtttattacagggacagcagagatccagtttatcgataagcttgggagttccgcgttacataacttacggtaaatggcccgcctggctgaccgcccaacgacccccgcccattgacgtcaataatgacgtatgttcccatagtaacgccaatagggactttccattgacgtcaatgggtggagtatttacggtaaactgcccacttggcagtacatcaagtgtatcatatgccaagtacgccccctattgacgtcaatgacggtaaatggcccgcctggcattatgcccagtacatgaccttatgggactttcctacttggcagtacatctacgtattagtcatcgctattaccatggtgatgcggttttggcagtacatcaatgggcgtggatagcggtttgactcacggggatttccaagtctccaccccattgacgtcaatgggagtttgttttggcaccaaaatcaacgggactttccaaaatgtcgtaacaactccgccccattgacgcaaatgggcggtaggcgtgtacggtgggaggtctatataagcagagctcgtttagtgaaccgtcagatcgcctggagacgccatccacgctgttttgacctccatagaagacaccgactctactagaggatctatttccggtgaattcgccaccatgggacccaggctcctcttctgggcactgctttgtctcctcggaaccggtccggttgaagctgacatctaccagaccccaagataccttgttatagggacaggaaagaagatcactctggaatgttctcaaaccatgggccatgacaaaatgtactggtatcaacaagatccaggaatggaactacacctcatccactattcctatggagttaattccacagagaagggagatctttcctctgagtcaacagtctccagaataaggacggagcattttcccctgaccctggagtctgccaggccctcacatacctctcagtacctctgtgccagcagtcggacgcccaacattcagtacttcggcgccgggacccggctctcagtgctggaggacctgaaaaacgtgttcccacccgaggcggccgcgtttgagccatcagaagcagagatctcccacacccaaaaggccacactggtgtgcctggccacaggcttctaccccgaccacgtggagctgagctggtgggtgaatgggaaggaggtgcacagtggggtcagcacagacccgcagcccctcaaggagcagcccgccctcaatgactccagatactgcctgagcagccgcctgagggtctcggccaccttctggcagaacccccgcaaccacttccgctgtcaagtccagttctacgggctctcggagaatgacgagtggacccaggatagggccaaacctgtcacccagatcgtcagcgccgaggcctggggtagagcagactgtggcttcacctccgagtcttaccagcaaggggtcctgtctgccaccatcctctatgagatcttgctagggaaggccaccttgtatgccgtgctggtcagtgccctcgtgctgatggccatggtcaagagaaaggattccagaggcgggagcggagccacgaacttctctctgttaaagcaagcaggagacgtggaagaaaaccccggtcctatgaactcctctctggactttctaattctgatcttaatgtttggaggaactagtggtcaacagctgaatcagagtcctcaatctatgtttatccaggaaggagaagatgtctccatgaactgcacttcttcaagcatatttaacacctggctatggtacaagcaggaacctggggaaggtcctgtcctcttgatagccttatataaggctggtgaattgacctcaaatggaagactgactgctcagtttggtataaccagaaaggacagcttcctgaatatctcagcatccatacctagtgatgtaggcatctacttctgtgctggcacataccagaaagttacctttggaactggaacaaagctccaagtcatcccaaatatccagaaccctgaccctgccgtgtaccagctgagagactctaaatccagtgacaagtctgcatgcctattcaccgattttgattctcaaacaaatgtgtcacaaagtaaggattctgatgtgtatatcacagacaaaactgtgctagacatgaggtctatggacttcaagagcaacagtgctgtggcctggagcaacaaatctgactttgcatgtgcaaacgccttcaacaacagcattattccagaagacaccttcttccccagcccagaaagttcctgtgatgtcaagctggtcgagaaaagctttgaaacagatacgaacctaaactttcaaaacctgtcagtgattgggttccgaatcctcctcctgaaagtggccgggtttaatctgctcatgacgctgcggctgtggtccagctgactcgagggatcccgcccctctccctcccccccccctaacgttactggccgaagccgcttggaataaggccggtgtgcgtttgtctatatgttattttccaccatattgccgtcttttggcaatgtgagggcccggaaacctggccctgtcttcttgacgagcattcctaggggtctttcccctctcgccaaaggaatgcaaggtctgttgaatgtcgtgaaggaagcagttcctctggaagcttcttgaagacaaacaacgtctgtagcgaccctttgcaggcagcggaaccccccacctggcgacaggtgcctctgcggccaaaagccacgtgtataagatacacctgcaaaggcggcacaaccccagtgccacgttgtgagttggatagttgtggaaagagtcaaatggctcacctcaagcgtattcaacaaggggctgaaggatgcccagaaggtaccccattgtatgggatctgatctggggcctcggtgcacatgctttacatgtgtttagtcgaggttaaaaaacgtctaggccccccgaaccacggggacgtggttttcctttgaaaaacacgatgataatatggtgagcaagggcgaggaggataacatggccatcatcaaggagttcatgcgcttcaaggtgcacatggagggctccgtgaacggccacgagttcgagatcgagggcgagggcgagggccgcccctacgagggcacccagaccgccaagctgaaggtgaccaagggtggccccctgcccttcgcctgggacatcctgtcccctcagttcatgtacggctccaaggcctacgtgaagcaccccgccgacatccccgactacttgaagctgtccttccccgagggcttcaagtgggagcgcgtgatgaacttcgaggacggcggcgtggtgaccgtgacccaggactcctccctgcaggacggcgagttcatctacaaggtgaagctgcgcggcaccaacttcccctccgacggccccgtaatgcagaagaagaccatgggctgggaggcctcctccgagcggatgtaccccgaggacggcgccctgaagggcgagatcaagcagaggctgaagctgaaggacggcggccactacgacgctgaggtcaagaccacctacaaggccaagaagcccgtgcagctgcccggcgcctacaacgtcaacatcaagttggacatcacctcccacaacgaggactacaccatcgtggaacagtacgaacgcgccgagggccgccactccaccggcggcatggacgagctgtacaagtgaacgcgtctggaacaagctttttccccgtatccccccaggtgtctgcaggctcaaagagcagcgagaagcgttcagaggaaagcgatcccgtgccaccttccccgtgcccgggctgtccccgcacgctgccggctcggggatgcggggggagcgccggaccggagcggagccccgggcggctcgctgctgccccctagcgggggagggacgtaattacatccctgggggctttgggggggggctgtccccgtgagctcttactccctatcagtgatagagaacgtatgaagagtttactccctatcagtgatagagaacgtatgcagactttactccctatcagtgatagagaacgtataaggagtttactccctatcagtgatagagaacgtatgaccagtttactccctatcagtgatagagaacgtatctacagtttactccctatcagtgatagagaacgtatatccagtttactccctatcagtgatagagaacgtatgtcgaggtaggcgtgtacggtgggcgcctataaaagcagagctcgtttagtgaaccgtcagatcgcctggagcaattccacaacacttttgtcttatacttatgctcgagggagtgcaggtggagactatctccccaggagacgggcgcaccttccccaagcgcggccagacctgcgtggtgcactacaccgggatgcttgaagatggaaagaaagttgattcctcccgggacagaaacaagccctttaagtttatgctaggcaagcaggaggtgatccgaggctgggaagaaggggttgcccagatgagtgtgggtcagagagccaaactgactatatctccagattatgcctatggtgccactgggcacccaggcatcatcccaccacatgccactctcgtcttcgatgtggagcttctaaaactggaatctggcggtggatccggagtcgacggatttggtgatgtcggtgctcttgagagtttgaggggaaatgcagatttggcttacatcctgagcatggagccctgtggccactgcctcattatcaacaatgtgaacttctgccgtgagtccgggctccgcacccgcactggctccaacatcgactgtgagaagttgcggcgtcgcttctcctcgctgcatttcatggtggaggtgaagggcgacctgactgccaagaaaatggtgctggctttgctggagctggcgcggcaggaccacggtgctctggactgctgcgtggtggtcattctctctcacggctgtcaggccagccacctgcagttcccaggggctgtctacggcacagatggatgccctgtgtcggtcgagaagattgtgaacatcttcaatgggaccagctgccccagcctgggagggaagcccaagctctttttcatccaggcctgtggtggggagcagaaagaccatgggtttgaggtggcctccacttcccctgaagacgagtcccctggcagtaaccccgagccagatgccaccccgttccaggaaggtttgaggaccttcgaccagctggacgccatatctagtttgcccacacccagtgacatctttgtgtcctactctactttcccaggttttgtttcctggagggaccccaagagtggctcctggtacgttgagaccctggacgacatctttgagcagtgggctcactctgaagacctgcagtccctcctgcttagggtcgctaatgctgtttcggtgaaagggatttataaacagatgcctggttgctttaatttcctccggaaaaaacttttctttaaaacatcagtcgactatccgtacgacgtaccagactacgcactcgactaaaagctttttccccgtatccccccaggtgtctgcaggctcaaagagcagcgagaagcgttcagaggaaagcgatcccgtgccaccttccccgtgcccgggctgtccccgcacgctgccggctcggggatgcggggggagcgccggaccggagcggagccccgggcggctcgctgctgccccctagcgggggagggacgtaattacatccctgggggctttgggagggggctgtccccgtgagctcaatcaacctctggattacaaaatttgtgaaagattgactggtattcttaactatgttgctccttttacgctatgtggatacgctgctttaatgcctttgtatcatgctattgcttcccgtatggctttcattttctcctccttgtataaatcctggttgctgtctctttatgaggagttgtggcccgttgtcaggcaacgtggcgtggtgtgcactgtgtttgctgacgcaacccccactggttggggcattgccaccacctgtcagctcctttccgggactttcgctttccccctccctattgccacggcggaactcatcgccgcctgccttgcccgctgctggacaggggctcggctgttgggcactgacaattccgtggtgttgtcggggaagctgacgtcctttccatggctgctcgcctgtgttgccacctggattctgcgcgggacgtccttctgctacgtcccttcggccctcaatccagcggaccttccttcccgcggcctgctgccggctctgcggcctcttccgcgtcttcgccttcgccctcagacgagtcggatctccctttgggccgcctccccgcctggaattaattctgcagtcgagacctagaaaaacatggagcaatcacaagtagcaatacagcagctaccaatgctgattgtgcctggctagaagcacaagaggaggaggaggtgggttttccagtcacacctcaggtacctttaagaccaatgacttacaaggcagctgtagatcttagccactttttaaaagaaaagaggggactggaagggctaattcactcccaacgaagacaagatatccttgatctgtggatctaccacacacaaggctacttccctgattagcagaactacacaccagggccaggggtcagatatccactgacctttggatggtgctacaagctagtaccagttgagccagataaggtagaagaggccaataaaggagagaacaccagcttgttacaccctgtgagcctgcatgggatggatgacccggagagagaagtgttagagtggaggtttgacagccgcctagcatttcatcacgtggcccgagagctgcatccggagtacttcaagaactgctgatatcgagcttgctacaagggactttccgctggggactttccagggaggcgtggcctgggcgggactggggagtggcgagccctcagatcctgcatataagcagctgctttttgcctgtactgggtctctctggttagaccagatctgagcctgggagctctctggctaactagggaacccactgcttaagcctcaataaagcttgccttgagtgcttcaagtagtgtgtgcccgtctgttgtgtgactctggtaactagagatccctcagacccttttagtcagtgtggaaaatctctagcagtagtagttcatgtcatcttattattcagtatttataacttgcaaagaaatgaatatcagagagtgagaggccttgacattgctagcgtttaccgtcgacctctagctagagcttggcgtaatcatggtcatagctgtttcctgtgtgaaattgttatccgctcacaattccacacaacatacgagccggaagcataaagtgtaaagcctggggtgcctaatgagtgagctaactcacattaattgcgttgcgctcactgcccgctttccagtcgggaaacctgtcgtgccagctgcattaatgaatcggccaacgcgcggggagaggcggtttgcgtattgggcgctcttccgcttcctcgctcactgactcgctgcgctcggtcgttcggctgcggcgagcggtatcagctcactcaaaggcggtaatacggttatccacagaatcaggggataacgcaggaaagaacatgtgagcaaaaggccagcaaaaggccaggaaccgtaaaaaggccgcgttgctggcgtttttccataggctccgcccccctgacgagcatcacaaaaatcgacgctcaagtcagaggtggcgaaacccgacaggactataaagataccaggcgtttccccctggaagctccctcgtgcgctctcctgttccgaccctgccgcttaccggatacctgtccgcctttctcccttcgggaagcgtggcgctttctcatagctcacgctgtaggtatctcagttcggtgtaggtcgttcgctccaagctgggctgtgtgcacgaaccccccgttcagcccgaccgctgcgccttatccggtaactatcgtcttgagtccaacccggtaagacacgacttatcgccactggcagcagccactggtaacaggattagcagagcgaggtatgtaggcggtgctacagagttcttgaagtggtggcctaactacggctacactagaagaacagtatttggtatctgcgctctgctgaagccagttaccttcggaaaaagagttggtagctcttgatccggcaaacaaaccaccgctggtagcggtggtttttttgtttgcaagcagcagattacgcgcagaaaaaaaggatctcaagaagatcctttgatcttttctacggggtctgacgctcagtggaacgaaaactcacgttaagggattttggtcatgagattatcaaaaaggatcttcacctagatccttttaaattaaaaatgaagttttaaatcaatctaaagtatatatgagtaaacttggtctgacagttaccaatgcttaatcagtgaggcacctatctcagcgatctgtctatttcgttcatccatagttgcctgactccccgtcgtgtagataactacgatacgggagggcttaccatctggccccagtgctgcaatgataccgcgagacccacgctcaccggctccagatttatcagcaataaaccagccagccggaagggccgagcgcagaagtggtcctgcaactttatccgcctccatccagtctattaattgttgccgggaagctagagtaagtagttcgccagttaatagtttgcgcaacgttgttgccattgctacaggcatcgtggtgtcacgctcgtcgtttggtatggcttcattcagctccggttcccaacgatcaaggcgagttacatgatcccccatgttgtgcaaaaaagcggttagctccttcggtcctccgatcgttgtcagaagtaagttggccgcagtgttatcactcatggttatggcagcactgcataattctcttactgtcatgccatccgtaagatgcttttctgtgactggtgagtactcaaccaagtcattctgagaatagtgtatgcggcgaccgagttgctcttgcccggcgtcaatacgggataataccgcgccacatagcagaactttaaaagtgctcatcattggaaaacgttcttcggggcgaaaactctcaaggatcttaccgctgttgagatccagttcgatgtaacccactcgtgcacccaactgatcttcagcatcttttactttcaccagcgtttctgggtgagcaaaaacaggaaggcaaaatgccgcaaaaaagggaataagggcgacacggaaatgttgaatactcatactcttcctttttcaatattattgaagcatttatcagggttattgtctcatgagcggatacatatttgaatgtatttagaaaaataaacaaataggggttccgcgcacatttccccgaaaagtgccacctgacgtcgacggatcgggagatcaacttgtttattgcagcttataatggttacaaataaagcaatagcatcacaaatttcacaaataaagcatttttttcactgcattctagttgtggtttgtccaaactcatcaatgtatcttatcatgtctggatcaactggataactcaagctaaccaaaatcatcccaaacttcccaccccataccctattaccactgccaattacctgtggtttcatttactctaaacctgtgattcctctgaattattttcattttaaagaaattgtatttgttaaatatgtactacaaacttagtagt

SEQ ID NO: 23 - DNA, 12037 bp, synthetic construct
  misc_feature 1..12037: note = Description of Artificial Sequence: Synthetic polynucleotide
  source 1..12037: mol_type = other DNA
tggaagggctaattcactcccaaagaagacaagatatccttgatctgtggatctaccacacacaaggctacttccctgattagcagaactacacaccagggccaggggtcagatatccactgacctttggatggtgctacaagctagtaccagttgagccagataaggtagaagaggccaataaaggagagaacaccagcttgttacaccctgtgagcctgcatgggatggatgacccggagagagaagtgttagagtggaggtttgacagccgcctagcatttcatcacgtggcccgagagctgcatccggagtacttcaagaactgctgatatcgagcttgctacaagggactttccgctggggactttccagggaggcgtggcctgggcgggactggggagtggcgagccctcagatcctgcatataagcagctgctttttgcctgtactgggtctctctggttagaccagatctgagcctgggagctctctggctaactagggaacccactgcttaagcctcaataaagcttgccttgagtgcttcaagtagtgtgtgcccgtctgttgtgtgactctggtaactagagatccctcagacccttttagtcagtgtggaaaatctctagcagtggcgcccgaacagggacttgaaagcgaaagggaaaccagaggagctctctcgacgcaggactcggcttgctgaagcgcgcacggcaagaggcgaggggcggcgactggtgagtacgccaaaaattttgactagcggaggctagaaggagagagatgggtgcgagagcgtcagtattaagcgggggagaattagatcgcgatgggaaaaaattcggttaaggccagggggaaagaaaaaatataaattaaaacatatagtatgggcaagcagggagctagaacgattcgcagttaatcctggcctgttagaaacatcagaaggctgtagacaaatactgggacagctacaaccatcccttcagacaggatcagaagaacttagatcattatataatacagtagcaaccctctattgtgtgcatcaaaggatagagataaaagacaccaaggaagctttagacaagatagaggaagagcaaaacaaaagtaagaccaccgcacagcaagcggccggccgctgatcttcagacctggaggaggagatatgagggacaattggagaagtgaattatataaatataaagtagtaaaaattgaaccattaggagtagcacccaccaaggcaaagagaagagtggtgcagagagaaaaaagagcagtgggaataggagctttgttccttgggttcttgggagcagcaggaagcactatgggcgcagcgtcaatgacgctgacggtacaggccagacaattattgtctggtatagtgcagcagcagaacaatttgctgagggctattgaggcgcaacagcatctgttgcaactcacagtctggggcatcaagcagctccaggcaagaatcctggctgtggaaagatacctaaaggatcaacagctcctggggatttggggttgctctggaaaactcatttgcaccactgctgtgccttggaatgctagttggagtaataaatctctggaacagatttggaatcacacgacctggatggagtgggacagagaaattaacaattacacaagcttaatacactccttaattgaagaatcgcaaaaccagcaagaaaagaatgaacaagaattattggaattagataaatgggcaagtttgtggaattggtttaacataacaaattggctgtggtatataaaattattcataatgatagtaggaggcttggtaggtttaagaatagtttttgctgtactttctatagtgaatagagttaggcagggatattcaccattatcgtttcagacccacctcccaaccccgaggggacccgacaggcccgaaggaatagaagaagaaggtggagagagagacagagacagatccattcgattagtgaacggatctcgacggtatcgcctttaaaagaaaaggggggattggggggtacagtgcaggggaaagaatagtagacataatagcaacagacatacaaactaaagaattacaaaaacaaattacaaaaattcaaaattttcgggtttattacagggacagcagagatccagtttatcgataagcttgggagttccgcgttacataacttacggtaaatggcccgcctggctgaccgcccaacgacccccgcccattgacgtcaataatgacgtatgttcccatagtaacgccaatagggactttccattgacgtcaatgggtggagtatttacggtaaactgcccacttggcagtacatcaagtgtatcatatgccaagtacgccccctattgacgtcaatgacggtaaatggcccgcctggcattatgcccagtacatgaccttatgggactttcctacttggcagtacatctacgtattagtcatcgctattaccatggtgatgcggttttggcagtacatcaatgggcgtggatagcggtttgactcacggggatttccaagtctccaccccattgacgtcaatgggagtttgttttggcaccaaaatcaacgggactttccaaaatgtcgtaacaactccgccccattgacgcaaatgggcggtaggcgtgtacggtgggaggtctatataagcagagctcgtttagtgaaccgtcagatcgcctggagacgccatccacgctgttttgacctccatagaagacaccgactctactagaggatctatttccggtgaattcgccaccatgggcacaaggttgttcttctatgtggccctttgtctcctgtggaccggtcacatggaagctgacatctaccagaccccaagataccttgttatagggacaggaaagaagatcactctggaatgttctcaaaccatgggccatgacaaaatgtactggtatcaacaagatccaggaatggaactacacctcatccactattcctatggagttaattccacagagaagggagatctttcctctgagtcaacagtctccagaataaggacggagcattttcccctgaccctggagtctgccaggccctcacatacctctcagtacctctgtgccagcagtcggacgcccaacattcagtacttcggcgccgggacccggctctcagtgctggaggacctgaaaaacgtgttcccacccgaggtcgctgtgtttgagccatcagaagcagagatctcccacacccaaaaggccacactagtgtgcctggccacaggcttctaccccgaccacgtggagctgagctggtgggtgaatgggaaggaggtgcacagtggggtcagcacagacccgcagcccctcaaggagcagcccgccctcaatgactccagatactgcctgagcagccgcctgagggtctcggccaccttctggcagaacccccgcaaccacttccgctgtcaagtccagttctacgggctctcggagaatgacgagtggacccaggatagggccaaacctgtcacccagatcgtcagcgccgaggcctggggtagagcagactgtggcttcacctccgagtcttaccagcaaggggtcctgtctgccaccatcctctatgagatcttgctagggaaggccaccttgtatgccgtgctggtcagtgccctcgtgctgatggccatggtcaagagaaaggattccagaggcgggagcggagccacgaacttctctctgttaaagcaagcaggagacgtggaagaaaaccccggtcctatggcaggcattcgagctttatttatgtacttgtggctgcagctggactgggtctcgagaggtcaacagctgaatcagagtcctcaatctatgtttatccaggaaggagaagatgtctccatgaactgcacttcttcaagcatatttaacacctggctatggtacaagcaggaacctggggaaggtcctgtcctcttgatagccttatataaggctggtgaattgacctcaaatggaagactgactgctcagtttggtataaccagaaaggacagcttcctgaatatctcagcatccatacctagtgatgtaggcatctacttctgtgctggcacataccagaaagttacctttggaactggaacaaagctccaagtcatcccaaatatccagaaccctgaccctgccgtgtaccagctgagagactctaaatccagtgacaagtctgtctgcctattcaccgattttgattctcaaacaaatgtgtcacaaagtaaggattctgatgtgtatatcacagacaaaactgtgctagacatgaggtctatggacttcaagagcaacagtgcggccgcctggagcaacaaatctgactttgcatgtgcaaacgccttcaacaacagcattattccagaagacaccttcttccccagcccagaaagttcctgtgatgtcaagctggtcgagaaaagctttgaaacagatacgaacctaaactttcaaaacctgtcagtgattgggttccgaatcctcctcctgaaagtggccgggtttaatctgctcatgacgctgcggctgtggtccagctgactcgagggatcccgcccctctccctcccccccccctaacgttactggccgaagccgcttggaataaggccggtgtgcgtttgtctatatgttattttccaccatattgccgtcttttggcaatgtgagggcccggaaacctggccctgtcttcttgacgagcattcctaggggtctttcccctctcgccaaaggaatgcaaggtctgttgaatgtcgtgaaggaagcagttcctctggaagcttcttgaagacaaacaacgtctgtagcgaccctttgcaggcagcggaaccccccacctggcgacaggtgcctctgcggccaaaagccacgtgtataagatacacctgcaaaggcggcacaaccccagtgccacgttgtgagttggatagttgtggaaagagtcaaatggctcacctcaagcgtattcaacaaggggctgaaggatgcccagaaggtaccccattgtatgggatctgatctggggcctcggtgcacatgctttacatgtgtttagtcgaggttaaaaaacgtctaggccccccgaaccacggggacgtggttttcctttgaaaaacacgatgataatatggtgagcaagggcgaggaggataacatggccatcatcaaggagttcatgcgcttcaaggtgcacatggagggctccgtgaacggccacgagttcgagatcgagggcgagggcgagggccgcccctacgagggcacccagaccgccaagctgaaggtgaccaagggtggccccctgcccttcgcctgggacatcctgtcccctcagttcatgtacggctccaaggcctacgtgaagcaccccgccgacatccccgactacttgaagctgtccttccccgagggcttcaagtgggagcgcgtgatgaacttcgaggacggcggcgtggtgaccgtgacccaggactcctccctgcaggacggcgagttcatctacaaggtgaagctgcgcggcaccaacttcccctccgacggccccgtaatgcagaagaagaccatgggctgggaggcctcctccgagcggatgtaccccgaggacggcgccctgaagggcgagatcaagcagaggctgaagctgaaggacggcggccactacgacgctgaggtcaagaccacctacaaggccaagaagcccgtgcagctgcccggcgcctacaacgtcaacatcaagttggacatcacctcccacaacgaggactacaccatcgtggaacagtacgaacgcgccgagggccgccactccaccggcggcatggacgagctgtacaagtgaacgcgtctggaacaagctttttccccgtatccccccaggtgtctgcaggctcaaagagcagcgagaagcgttcagaggaaagcgatcccgtgccaccttccccgtgcccgggctgtccccgcacgctgccggctcggggatgcggggggagcgccggaccggagcggagccccgggcggctcgctgctgccccctagcgggggagggacgtaattacatccctgggggctttgggggggggctgtccccgtgagctcttactccctatcagtgatagagaacgtatgaagagtttactccctatcagtgatagagaacgtatgcagactttactccctatcagtgatagagaacgtataaggagtttactccctatcagtgatagagaacgtatgaccagtttactccctatcagtgatagagaacgtatctacagtttactccctatcagtgatagagaacgtatatccagtttactccctatcagtgatagagaacgtatgtcgaggtaggcgtgtacggtgggcgcctataaaagcagagctcgtttagtgaaccgtcagatcgcctggagcaattccacaacacttttgtcttatacttatgctcgagggagtgcaggtggagactatctccccaggagacgggcgcaccttccccaagcgcggccagacctgcgtggtgcactacaccgggatgcttgaagatggaaagaaagttgattcctcccgggacagaaacaagccctttaagtttatgctaggcaagcaggaggtgatccgaggctgggaagaaggggttgcccagatgagtgtgggtcagagagccaaactgactatatctccagattatgcctatggtgccactgggcacccaggcatcatcccaccacatgccactctcgtcttcgatgtggagcttctaaaactggaatctggcggtggatccggagtcgacggatttggtgatgtcggtgctcttgagagtttgaggggaaatgcagatttggcttacatcctgagcatggagccctgtggccactgcctcattatcaacaatgtgaacttctgccgtgagtccgggctccgcacccgcactggctccaacatcgactgtgagaagttgcggcgtcgcttctcctcgctgcatttcatggtggaggtgaagggcgacctgactgccaagaaaatggtgctggctttgctggagctggcgcggcaggaccacggtgctctggactgctgcgtggtggtcattctctctcacggctgtcaggccagccacctgcagttcccaggggctgtctacggcacagatggatgccctgtgtcggtcgagaagattgtgaacatcttcaatgggaccagctgccccagcctgggagggaagcccaagctctttttcatccaggcctgtggtggggagcagaaagaccatgggtttgaggtggcctccacttcccctgaagacgagtcccctggcagtaaccccgagccagatgccaccccgttccaggaaggtttgaggaccttcgaccagctggacgccatatctagtttgcccacacccagtgacatctttgtgtcctactctactttcccaggttttgtttcctggagggaccccaagagtggctcctggtacgttgagaccctggacgacatctttgagcagtgggctcactctgaagacctgcagtccctcctgcttagggtcgctaatgctgtttcggtgaaagggatttataaacagatgcctggttgctttaatttcctccggaaaaaacttttctttaaaacatcagtcgactatccgtacgacgtaccagactacgcactcgactaaaagctttttccccgtatccccccaggtgtctgcaggctcaaagagcagcgagaagcgttcagaggaaagcgatcccgtgccaccttccccgtgcccgggctgtccccgcacgctgccggctcggggatgcggggggagcgccggaccggagcggagccccgggcggctcgctgctgccccctagcgggggagggacgtaattacatccctgggggctttgggagggggctgtccccgtgagctcaatcaacctctggattacaaaatttgtgaaagattgactggtattcttaactatgttgctccttttacgctatgtggatacgctgctttaatgcctttgtatcatgctattgcttcccgtatggctttcattttctcctccttgtataaatcctggttgctgtctctttatgaggagttgtggcccgttgtcaggcaacgtggcgtggtgtgcactgtgtttgctgacgcaacccccactggttggggcattgccaccacctgtcagctcctttccgggactttcgctttccccctccctattgccacggcggaactcatcgccgcctgccttgcccgctgctggacaggggctcggctgttgggcactgacaattccgtggtgttgtcggggaagctgacgtcctttccatggctgctcgcctgtgttgccacctggattctgcgcgggacgtccttctgctacgtcccttcggccctcaatccagcggaccttccttcccgcggcctgctgccggctctgcggcctcttccgcgtcttcgccttcgccctcagacgagtcggatctccctttgggccgcctccccgcctggaattaattctgcagtcgagacctagaaaaacatggagcaatcacaagtagcaatacagcagctaccaatgctgattgtgcctggctagaagcacaagaggaggaggaggtgggttttccagtcacacctcaggtacctttaagaccaatgacttacaaggcagctgtagatcttagccactttttaaaagaaaagaggggactggaagggctaattcactcccaacgaagacaagatatccttgatctgtggatctaccacacacaaggctacttccctgattagcagaactacacaccagggccaggggtcagatatccactgacctttggatggtgctacaagctagtaccagttgagccagataaggtagaagaggccaataaaggagagaacaccagcttgttacaccctgtgagcctgcatgggatggatgacccggagagagaagtgttagagtggaggtttgacagccgcctagcatttcatcacgtggcccgagagctgcatccggagtacttcaagaactgctgatatcgagcttgctacaagggactttccgctggggactttccagggaggcgtggcctgggcgggactggggagtggcgagccctcagatcctgcatataagcagctgctttttgcctgtactgggtctctctggttagaccagatctgagcctgggagctctctggctaactagggaacccactgcttaagcctcaataaagcttgccttgagtgcttcaagtagtgtgtgcccgtctgttgtgtgactctggtaactagagatccctcagacccttttagtcagtgtggaaaatctctagcagtagtagttcatgtcatcttattattcagtatttataacttgcaaagaaatgaatatcagagagtgagaggccttgacattgctagcgtttaccgtcgacctctagctagagcttggcgtaatcatggtcatagctgtttcctgtgtgaaattgttatccgctcacaattccacacaacatacgagccggaagcataaagtgtaaagcctggggtgcctaatgagtgagctaactcacattaattgcgttgcgctcactgcccgctttccagtcgggaaacctgtcgtgccagctgcattaatgaatcggccaacgcgcggggagaggcggtttgcgtattgggcgctcttccgcttcctcgctcactgactcgctgcgctcggtcgttcggctgcggcgagcggtatcagctcactcaaaggcggtaatacggttatccacagaatcaggggataacgcaggaaagaacatgtgagcaaaaggccagcaaaaggccaggaaccgtaaaaaggccgcgttgctggcgtttttccataggctccgcccccctgacgagcatcacaaaaatcgacgctcaagtcagaggtggcgaaacccgacaggactataaagataccaggcgtttccccctggaagctccctcgtgcgctctcctgttccgaccctgccgcttaccggatacctgtccgcctttctcccttcgggaagcgtggcgctttctcatagctcacgctgtaggtatctcagttcggtgtaggtcgttcgctccaagctgggctgtgtgcacgaaccccccgttcagcccgaccgctgcgccttatccggtaactatcgtcttgagtccaacccggtaagacacgacttatcgccactggcagcagccactggtaacaggattagcagagcgaggtatgtaggcggtgctacagagttcttgaagtggtggcctaactacggctacactagaagaacagtatttggtatctgcgctctgctgaagccagttaccttcggaaaaagagttggtagctcttgatccggcaaacaaaccaccgctggtagcggtggtttttttgtttgcaagcagcagattacgcgcagaaaaaaaggatctcaagaagatcctttgatcttttctacggggtctgacgctcagtggaacgaaaactcacgttaagggattttggtcatgagattatcaaaaaggatcttcacctagatccttttaaattaaaaatgaagttttaaatcaatctaaagtatatatgagtaaacttggtctgacagttaccaatgcttaatcagtgaggcacctatctcagcgatctgtctatttcgttcatccatagttgcctgactccccgtcgtgtagataactacgatacgggagggcttaccatctggccccagtgctgcaatgataccgcgagacccacgctcaccggctccagatttatcagcaataaaccagccagccggaagggccgagcgcagaagtggtcctgcaactttatccgcctccatccagtctattaattgttgccgggaagctagagtaagtagttcgccagttaatagtttgcgcaacgttgttgccattgctacaggcatcgtggtgtcacgctcgtcgtttggtatggcttcattcagctccggttcccaacgatcaaggcgagttacatgatcccccatgttgtgcaaaaaagcggttagctccttcggtcctccgatcgttgtcagaagtaagttggccgcagtgttatcactcatggttatggcagcactgcataattctcttactgtcatgccatccgtaagatgcttttctgtgactggtgagtactcaaccaagtcattctgagaatagtgtatgcggcgaccgagttgctcttgcccggcgtcaatacgggataataccgcgccacatagcagaactttaaaagtgctcatcattggaaaacgttcttcggggcgaaaactctcaaggatcttaccgctgttgagatccagttcgatgtaacccactcgtgcacccaactgatcttcagcatcttttactttcaccagcgtttctgggtgagcaaaaacaggaaggcaaaatgccgcaaaaaagggaataagggcgacacggaaatgttgaatactcatactcttcctttttcaatattattgaagcatttatcagggttattgtctcatgagcggatacatatttgaatgtatttagaaaaataaacaaataggggttccgcgcacatttccccgaaaagtgccacctgacgtcgacggatcgggagatcaacttgtttattgcagcttataatggttacaaataaagcaatagcatcacaaatttcacaaataaagcatttttttcactgcattctagttgtggtttgtccaaactcatcaatgtatcttatcatgtctggatcaactggataactcaagctaaccaaaatcatcccaaacttcccaccccataccctattaccactgccaattacctgtggtttcatttactctaaacctgtgattcctctgaattattttcattttaaagaaattgtatttgttaaatatgtactacaaacttagtagt

SEQ ID NO: 24 - DNA, 12037 bp, synthetic construct
  misc_feature 1..12037: note = Description of Artificial Sequence: Synthetic polynucleotide
  source 1..12037: mol_type = other DNA
tggaagggctaattcactcccaaagaagacaagatatccttgatctgtggatctaccacacacaaggctacttccctgattagcagaactacacaccagggccaggggtcagatatccactgacctttggatggtgctacaagctagtaccagttgagccagataaggtagaagaggccaataaaggagagaacaccagcttgttacaccctgtgagcctgcatgggatggatgacccggagagagaagtgttagagtggaggtttgacagccgcctagcatttcatcacgtggcccgagagctgcatccggagtacttcaagaactgctgatatcgagcttgctacaagggactttccgctggggactttccagggaggcgtggcctgggcgggactggggagtggcgagccctcagatcctgcatataagcagctgctttttgcctgtactgggtctctctggttagaccagatctgagcctgggagctctctggctaactagggaacccactgcttaagcctcaataaagcttgccttgagtgcttcaagtagtgtgtgcccgtctgttgtgtgactctggtaactagagatccctcagacccttttagtcagtgtggaaaatctctagcagtggcgcccgaacagggacttgaaagcgaaagggaaaccagaggagctctctcgacgcaggactcggcttgctgaagcgcgcacggcaagaggcgaggggcggcgactggtgagtacgccaaaaattttgactagcggaggctagaaggagagagatgggtgcgagagcgtcagtattaagcgggggagaattagatcgcgatgggaaaaaattcggttaaggccagggggaaagaaaaaatataaattaaaacatatagtatgggcaagcagggagctagaacgattcgcagttaatcctggcctgttagaaacatcagaaggctgtagacaaatactgggacagctacaaccatcccttcagacaggatcagaagaacttagatcattatataatacagtagcaaccctctattgtgtgcatcaaaggatagagataaaagacaccaaggaagctttagacaagatagaggaagagcaaaacaaaagtaagaccaccgcacagcaagcggccggccgctgatcttcagacctggaggaggagatatgagggacaattggagaagtgaattatataaatataaagtagtaaaaattgaaccattaggagtagcacccaccaaggcaaagagaagagtggtgcagagagaaaaaagagcagtgggaataggagctttgttccttgggttcttgggagcagcaggaagcactatgggcgcagcgtcaatgacgctgacggtacaggccagacaattattgtctggtatagtgcagcagcagaacaatttgctgagggctattgaggcgcaacagcatctgttgcaactcacagtctggggcatcaagcagctccaggcaagaatcctggctgtggaaagatacctaaaggatcaacagctcctggggatttggggttgctctggaaaactcatttgcaccactgctgtgccttggaatgctagttggagtaataaatctctggaacagatttggaatcacacgacctggatggagtgggacagagaaattaacaattacacaagcttaatacactccttaattgaagaatcgcaaaaccagcaagaaaagaatgaacaagaattattggaattagataaatgggcaagtttgtggaattggtttaacataacaaattggctgtggtatataaaattattcataatgatagtaggaggcttggtaggtttaagaatagtttttgctgtactttctatagtgaatagagttaggcagggatattcaccattatcgtttcagacccacctcccaaccccgaggggacccgacaggcccgaaggaatagaagaagaaggtggagagagagacagagacagatccattcgattagtgaacggatctcgacggtatcgcctttaaaagaaaaggggggattggggggtacagtgcaggggaaagaatagtagacataatagcaacagacatacaaactaaagaattacaaaaacaaattacaaaaattcaaaattttcgggtttattacagggacagcagagatccagtttatcgataagcttgggagttccgcgttacataacttacggtaaatggcccgcctggctgaccgcccaacgacccccgcccattgacgtcaataatgacgtatgttcccatagtaacgccaatagggactttccattgacgtcaatgggtggagtatttacggtaaactgcccacttggcagtacatcaagtgtatcatatgccaagtacgccccctattgacgtcaatgacggtaaatggcccgcctggcattatgcccagtacatgaccttatgggactttcctacttggcagtacatctacgtattagtcatcgctattaccatggtgatgcggttttggcagtacatcaatgggcgtggatagcggtttgactcacggggatttccaagtctccaccccattgacgtcaatgggagtttgttttggcaccaaaatcaacgggactttccaaaatgtcgtaacaactccgccccattgacgcaaatgggcggtaggcgtgtacggtgggaggtctatataagcagagctcgtttagtgaaccgtcagatcgcctggagacgccatccacgctgttttgacctccatagaagacaccgactctactagaggatctatttccggtgaattcgccaccatgggaatcaggctcctgtgtcgtgtggccttttgtttcctggctgtaggactagtagaagctgacatctaccagaccccaagataccttgttatagggacaggaaagaagatcactctggaatgttctcaaaccatgggccatgacaaaatgtactggtatcaacaagatccaggaatggaactacacctcatccactattcctatggagttaattccacagagaagggagatctttcctctgagtcaacagtctccagaataaggacggagcattttcccctgaccctggagtctgccaggccctcacatacctctcagtacctctgtgccagcagtcggacgcccaacattcagtacttcggcgccgggacccggctctcagtgctggaggacctgaaaaacgtgttcccacccgaggtcgctgtgtttgagccatcagaagcagagatctcccacacccaaaaggccacactggcatgcctggccacaggcttctaccccgaccacgtggagctgagctggtgggtgaatgggaaggaggtgcacagtggggtcagcacagacccgcagcccctcaaggagcagcccgccctcaatgactccagatactgcctgagcagccgcctgagggtctcggccaccttctggcagaacccccgcaaccacttccgctgtcaagtccagttctacgggctctcggagaatgacgagtggacccaggatagggccaaacctgtcacccagatcgtcagcgccgaggcctggggtagagcagactgtggcttcacctccgagtcttaccagcaaggggtcctgtctgccaccatcctctatgagatcttgctagggaaggccaccttgtatgccgtgctggtcagtgccctcgtgctgatggccatggtcaagagaaaggattccagaggcgggagcggagccacgaacttctctctgttaaagcaagcaggagacgtggaagaaaaccccggtcctatgacacgagttagcttgctgtgggcagtcgtggtctccacctgtctcgagtccggcatgggtcaacagctgaatcagagtcctcaatctatgtttatccaggaaggagaagatgtctccatgaactgcacttcttcaagcatatttaacacctggctatggtacaagcaggaacctggggaaggtcctgtcctcttgatagccttatataaggctggtgaattgacctcaaatggaagactgactgctcagtttggtataaccagaaaggacagcttcctgaatatctcagcatccatacctagtgatgtaggcatctacttctgtgctggcacataccagaaagttacctttggaactggaacaaagctccaagtcatcccaaatatccagaaccctgaccctgccgtgtaccagctgagagactctaaatccagtgacaagtctgtctgcctattcaccgattttgattctcaaacaaatgtgtcacaaagtaaggattctgatgtgtatatcacagacaaaactgtgctagacatgaggtctatggacttcaagagcaacagtgcggccgcctggagcaacaaatctgactttgcatgtgcaaacgccttcaacaacagcattattccagaagacaccttcttccccagcccagaaagttcctgtgatgtcaagctggtcgagaaaagctttgaaacagatacgaacctaaactttcaaaacctgtcagtgattgggttccgaatcctcctcctgaaagtggccgggtttaatctgctcatgacgctgcggctgtggtccagctgactcgagggatcccgcccctctccctcccccccccctaacgttactggccgaagccgcttggaataaggccggtgtgcgtttgtctatatgttattttccaccatattgccgtcttttggcaatgtgagggcccggaaacctggccctgtcttcttgacgagcattcctaggggtctttcccctctcgccaaaggaatgcaaggtctgttgaatgtcgtgaaggaagcagttcctctggaagcttcttgaagacaaacaacgtctgtagcgaccctttgcaggcagcggaaccccccacctggcgacaggtgcctctgcggccaaaagccacgtgtataagatacacctgcaaaggcggcacaaccccagtgccacgttgtgagttggatagttgtggaaagagtcaaatggctcacctcaagcgtattcaacaaggggctgaaggatgcccagaaggtaccccattgtatgggatctgatctggggcctcggtgcacatgctttacatgtgtttagtcgaggttaaaaaacgtctaggccccccgaaccacggggacgtggttttcctttgaaaaacacgatgataatatggtgagcaagggcgaggaggataacatggccatcatcaaggagttcatgcgcttcaaggtgcacatggagggctccgtgaacggccacgagttcgagatcgagggcgagggcgagggccgcccctacgagggcacccagaccgccaagctgaaggtgaccaagggtggccccctgcccttcgcctgggacatcctgtcccctcagttcatgtacggctccaaggcctacgtgaagcaccccgccgacatccccgactacttgaagctgtccttccccgagggcttcaagtgggagcgcgtgatgaacttcgaggacggcggcgtggtgaccgtgacccaggactcctccctgcaggacggcgagttcatctacaaggtgaagctgcgcggcaccaacttcccctccgacggccccgtaatgcagaagaagaccatgggctgggaggcctcctccgagcggatgtaccccgaggacggcgccctgaagggcgagatcaagcagaggctgaagctgaaggacggcggccactacgacgctgaggtcaagaccacctacaaggccaagaagcccgtgcagctgcccggcgcctacaacgtcaacatcaagttggacatcacctcccacaacgaggactacaccatcgtggaacagtacgaacgcgccgagggccgccactccaccggcggcatggacgagctgtacaagtgaacgcgtctggaacaagctttttccccgtatccccccaggtgtctgcaggctcaaagagcagcgagaagcgttcagaggaaagcgatcccgtgccaccttccccgtgcccgggctgtccccgcacgctgccggctcggggatgcggggggagcgccggaccggagcggagccccgggcggctcgctgctgccccctagcgggggagggacgtaattacatccctgggggctttgggggggggctgtccccgtgagctcttactccctatcagtgatagagaacgtatgaagagtttactccctatcagtgatagagaacgtatgcagactttactccctatcagtgatagagaacgtataaggagtttactccctatcagtgatagagaacgtatgaccagtttactccctatcagtgatagagaacgtatctacagtttactccctatcagtgatagagaacgtatatccagtttactccctatcagtgatagagaacgtatgtcgaggtaggcgtgtacggtgggcgcctataaaagcagagctcgtttagtgaaccgtcagatcgcctggagcaattccacaacacttttgtcttatacttatgctcgagggagtgcaggtggagactatctccccaggagacgggcgcaccttccccaagcgcggccagacctgcgtggtgcactacaccgggatgcttgaagatggaaagaaagttgattcctcccgggacagaaacaagccctttaagtttatgctaggcaagcaggaggtgatccgaggctgggaagaaggggttgcccagatgagtgtgggtcagagagccaaactgactatatctccagattatgcctatggtgccactgggcacccaggcatcatcccaccacatgccactctcgtcttcgatgtggagcttctaaaactggaatctggcggtggatccggagtcgacggatttggtgatgtcggtgctcttgagagtttgaggggaaatgcagatttggcttacatcctgagcatggagccctgtggccactgcctcattatcaacaatgtgaacttctgccgtgagtccgggctccgcacccgcactggctccaacatcgactgtgagaagttgcggcgtcgcttctcctcgctgcatttcatggtggaggtgaagggcgacctgactgccaagaaaatggtgctggctttgctggagctggcgcggcaggaccacggtgctctggactgctgcgtggtggtcattctctctcacggctgtcaggccagccacctgcagttcccaggggctgtctacggcacagatggatgccctgtgtcggtcgagaagattgtgaacatcttcaatgggaccagctgccccagcctgggagggaagcccaagctctttttcatccaggcctgtggtggggagcagaaagaccatgggtttgaggtggcctccacttcccctgaagacgagtcccctggcagtaaccccgagccagatgccaccccgttccaggaaggtttgaggaccttcgaccagctggacgccatatctagtttgcccacacccagtgacatctttgtgtcctactctactttcccaggttttgtttcctggagggaccccaagagtggctcctggtacgttgagaccctggacgacatctttgagcagtgggctcactctgaagacctgcagtccctcctgcttagggtcgctaatgctgtttcggtgaaagggatttataaacagatgcctggttgctttaatttcctccggaaaaaacttttctttaaaacatcagtcgactatccgtacgacgtaccagactacgcactcgactaaaagctttttccccgtatccccccaggtgtctgcaggctcaaagagcagcgagaagcgttcagaggaaagcgatcccgtgccaccttccccgtgcccgggctgtccccgcacgctgccggctcggggatgcggggggagcgccggaccggagcggagccccgggcggctcgctgctgccccctagcgggggagggacgtaattacatccctgggggctttgggagggggctgtccccgtgagctcaatcaacctctggattacaaaatttgtgaaagattgactggtattcttaactatgttgctccttttacgctatgtggatacgctgctttaatgcctttgtatcatgctattgcttcccgtatggctttcattttctcctccttgtataaatcctggttgctgtctctttatgaggagttgtggcccgttgtcaggcaacgtggcgtggtgtgcactgtgtttgctgacgcaacccccactggttggggcattgccaccacctgtcagctcctttccgggactttcgctttccccctccctattgccacggcggaactcatcgccgcctgccttgcccgctgctggacaggggctcggctgttgggcactgacaattccgtggtgttgtcggggaagctgacgtcctttccatggctgctcgcctgtgttgccacctggattctgcgcgggacgtccttctgctacgtcccttcggccctcaatccagcggaccttccttcccgcggcctgctgccggctctgcggcctcttccgcgtcttcgccttcgccctcagacgagtcggatctccctttgggccgcctccccgcctggaattaattctgcagtcgagacctagaaaaacatggagcaatcacaagtagcaatacagcagctaccaatgctgattgtgcctggctagaagcacaagaggaggaggaggtgggttttccagtcacacctcaggtacctttaagaccaatgacttacaaggcagctgtagatcttagccactttttaaaagaaaagaggggactggaagggctaattcactcccaacgaagacaagatatccttgatctgtggatctaccacacacaaggctacttccctgattagcagaactacacaccagggccaggggtcagatatccactgacctttggatggtgctacaagctagtaccagttgagccagataaggtagaagaggccaataaaggagagaacaccagcttgttacaccctgtgagcctgcatgggatggatgacccggagagagaagtgttagagtggaggtttgacagccgcctagcatttcatcacgtggcccgagagctgcatccggagtacttcaagaactgctgatatcgagcttgctacaagggactttccgctggggactttccagggaggcgtggcctgggcgggactggggagtggcgagccctcagatcctgcatataagcagctgctttttgcctgtactgggtctctctggttagaccagatctgagcctgggagctctctggctaactagggaacccactgcttaagcctcaataaagcttgccttgagtgcttcaagtagtgtgtgcccgtctgttgtgtgactctggtaactagagatccctcagacccttttagtcagtgtggaaaatctctagcagtagtagttcatgtcatcttattattcagtatttataacttgcaaagaaatgaatatcagagagtgagaggccttgacattgctagcgtttaccgtcgacctctagctagagcttggcgtaatcatggtcatagctgtttcctgtgtgaaattgttatccgctcacaattccacacaacatacgagccggaagcataaagtgtaaagcctggggtgcctaatgagtgagctaactcacattaattgcgttgcgctcactgcccgctttccagtcgggaaacctgtcgtgccagctgcattaatgaatcggccaacgcgcggggagaggcggtttgcgtattgggcgctcttccgcttcctcgctcactgactcgctgcgctcggtcgttcggctgcggcgagcggtatcagctcactcaaaggcggtaatacggttatccacagaatcaggggataacgcaggaaagaacatgtgagcaaaaggccagcaaaaggccaggaaccgtaaaaaggccgcgttgctggcgtttttccataggctccgcccccctgacgagcatcacaaaaatcgacgctcaagtcagaggtggcgaaacccgacaggactataaagataccaggcgtttccccctggaagctccctcgtgcgctctcctgttccgaccctgccgcttaccggatacctgtccgcctttctcccttcgggaagcgtggcgctttctcatagctcacgctgtaggtatctcagttcggtgtaggtcgttcgctccaagctgggctgtgtgcacgaaccccccgttcagcccgaccgctgcgccttatccggtaactatcgtcttgagtccaacccggtaagacacgacttatcgccactggcagcagccactggtaacaggattagcagagcgaggtatgtaggcggtgctacagagttcttgaagtggtggcctaactacggctacactagaagaacagtatttggtatctgcgctctgctgaagccagttaccttcggaaaaagagttggtagctcttgatccggcaaacaaaccaccgctggtagcggtggtttttttgtttgcaagcagcagattacgcgcagaaaaaaaggatctcaagaagatcctttgatcttttctacggggtctgacgctcagtggaacgaaaactcacgttaagggattttggtcatgagattatcaaaaaggatcttcacctagatccttttaaattaaaaatgaagttttaaatcaatctaaagtatatatgagtaaacttggtctgacagttaccaatgcttaatcagtgaggcacctatctcagcgatctgtctatttcgttcatccatagttgcctgactccccgtcgtgtagataactacgatacgggagggcttaccatctggccccagtgctgcaatgataccgcgagacccacgctcaccggctccagatttatcagcaataaaccagccagccggaagggccgagcgcagaagtggtcctgcaactttatccgcctccatccagtctattaattgttgccgggaagctagagtaagtagttcgccagttaatagtttgcgcaacgttgttgccattgctacaggcatcgtggtgtcacgctcgtcgtttggtatggcttcattcagctccggttcccaacgatcaaggcgagttacatgatcccccatgttgtgcaaaaaagcggttagctccttcggtcctccgatcgttgtcagaagtaagttggccgcagtgttatcactcatggttatggcagcactgcataattctcttactgtcatgccatccgtaagatgcttttctgtgactggtgagtactcaaccaagtcattctgagaatagtgtatgcggcgaccgagttgctcttgcccggcgtcaatacgggataataccgcgccacatagcagaactttaaaagtgctcatcattggaaaacgttcttcggggcgaaaactctcaaggatcttaccgctgttgagatccagttcgatgtaacccactcgtgcacccaactgatcttcagcatcttttactttcaccagcgtttctgggtgagcaaaaacaggaaggcaaaatgccgcaaaaaagggaataagggcgacacggaaatgttgaatactcatactcttcctttttcaatattattgaagcatttatcagggttattgtctcatgagcggatacatatttgaatgtatttagaaaaataaacaaataggggttccgcgcacatttccccgaaaagtgccacctgacgtcgacggatcgggagatcaacttgtttattgcagcttataatggttacaaataaagcaatagcatcacaaatttcacaaataaagcatttttttcactgcattctagttgtggtttgtccaaactcatcaatgtatcttatcatgtctggatcaactggataactcaagctaaccaaaatcatcccaaacttcccaccccataccctattaccactgccaattacctgtggtttcatttactctaaacctgtgattcctctgaattattttcattttaaagaaattgtatttgttaaatatgtactacaaacttagtagt

SEQ ID NO: 25 - DNA, 12031 bp, synthetic construct
  misc_feature 1..12031: note = Description of Artificial Sequence: Synthetic polynucleotide
  source 1..12031: mol_type = other DNA
tggaagggctaattcactcccaaagaagacaagatatccttgatctgtggatctaccacacacaaggctacttccctgattagcagaactacacaccagggccaggggtcagatatccactgacctttggatggtgctacaagctagtaccagttgagccagataaggtagaagaggccaataaaggagagaacaccagcttgttacaccctgtgagcctgcatgggatggatgacccggagagagaagtgttagagtggaggtttgacagccgcctagcatttcatcacgtggcccgagagctgcatccggagtacttcaagaactgctgatatcgagcttgctacaagggactttccgctggggactttccagggaggcgtggcctgggcgggactggggagtggcgagccctcagatcctgcatataagcagctgctttttgcctgtactgggtctctctggttagaccagatctgagcctgggagctctctggctaactagggaacccactgcttaagcctcaataaagcttgccttgagtgcttcaagtagtgtgtgcccgtctgttgtgtgactctggtaactagagatccctcagacccttttagtcagtgtggaaaatctctagcagtggcgcccgaacagggacttgaaagcgaaagggaaaccagaggagctctctcgacgcaggactcggcttgctgaagcgcgcacggcaagaggcgaggggcggcgactggtgagtacgccaaaaattttgactagcggaggctagaaggagagagatgggtgcgagagcgtcagtattaagcgggggagaattagatcgcgatgggaaaaaattcggttaaggccagggggaaagaaaaaatataaattaaaacatatagtatgggcaagcagggagctagaacgattcgcagttaatcctggcctgttagaaacatcagaaggctgtagacaaatactgggacagctacaaccatcccttcagacaggatcagaagaacttagatcattatataatacagtagcaaccctctattgtgtgcatcaaaggatagagataaaagacaccaaggaagctttagacaagatagaggaagagcaaaacaaaagtaagaccaccgcacagcaagcggccggccgctgatcttcagacctggaggaggagatatgagggacaattggagaagtgaattatataaatataaagtagtaaaaattgaaccattaggagtagcacccaccaaggcaaagagaagagtggtgcagagagaaaaaagagcagtgggaataggagctttgttccttgggttcttgggagcagcaggaagcactatgggcgcagcgtcaatgacgctgacggtacaggccagacaattattgtctggtatagtgcagcagcagaacaatttgctgagggctattgaggcgcaacagcatctgttgcaactcacagtctggggcatcaagcagctccaggcaagaatcctggctgtggaaagatacctaaaggatcaacagctcctggggatttggggttgctctggaaaactcatttgcaccactgctgtgccttggaatgctagttggagtaataaatctctggaacagatttggaatcacacgacctggatggagtgggacagagaaattaacaattacacaagcttaatacactccttaattgaagaatcgcaaaaccagcaagaaaagaatgaacaagaattattggaattagataaatgggcaagtttgtggaattggtttaacataacaaattggctgtggtatataaaattattcataatgatagtaggaggcttggtaggtttaagaatagtttttgctgtactttctatagtgaatagagttaggcagggatattcaccattatcgtttcagacccacctcccaaccccgaggggacccgacaggcccgaaggaatagaagaagaaggtggagagagagacagagacagatccattcgattagtgaacggatctcgacggtatcgcctttaaaagaaaaggggggattggggggtacagtgcaggggaaagaatagtagacataatagcaacagacatacaaactaaagaattacaaaaacaaattacaaaaattcaaaattttcgggtttattacagggacagcagagatccagtttatcgataagcttgggagttccgcgttacataacttacggtaaatggcccgcctggctgaccgcccaacgacccccgcccattgacgtcaataatgacgtatgttcccatagtaacgccaatagggactttccattgacgtcaatgggtggagtatttacggtaaactgcccacttggcagtacatcaagtgtatcatatgccaagtacgccccctattgacgtcaatgacggtaaatggcccgcctggcattatgcccagtacatgaccttatgggactttcctacttggcagtacatctacgtattagtcatcgctattaccatggtgatgcggttttggcagtacatcaatgggcgtggatagcggtttgactcacggggatttccaagtctccaccccattgacgtcaatgggagtttgttttggcaccaaaatcaacgggactttccaaaatgtcgtaacaactccgccccattgacgcaaatgggcggtaggcgtgtacggtgggaggtctatataagcagagctcgtttagtgaaccgtcagatcgcctggagacgccatccacgctgttttgacctccatagaagacaccgactctactagaggatctatttccggtgaattcgccaccatggcctccctgctcttcttctgtggggccttttatctcctgggaaccggttccatggaagctgacatctaccagaccccaagataccttgttatagggacaggaaagaagatcactctggaatgttctcaaaccatgggccatgacaaaatgtactggtatcaacaagatccaggaatggaactacacctcatccactattcctatggagttaattccacagagaagggagatctttcctctgagtcaacagtctccagaataaggacggagcattttcccctgaccctggagtctgccaggccctcacatacctctcagtacctctgtgccagcagtcggacgcccaacattcagtacttcggcgccgggacccggctctcagtgctggaggacctgaaaaacgtgttcccacccgaggtcgctgtgtttgagccatcagaagcagagatctcccacacccaaaaggccacactagtgtgcctggccacaggcttctaccccgaccacgtggagctgagctggtgggtgaatgggaaggaggtgcacagtggggtcagcacagacccgcagcccctcaaggagcagcccgccctcaatgactccagatactgcctgagcagccgcctgagggtctcggccaccttctggcagaacccccgcaaccacttccgctgtcaagtccagttctacgggctctcggagaatgacgagtggacccaggatagggccaaacctgtcacccagatcgtcagcgccgaggcctggggtagagcagactgtggcttcacctccgagtcttaccagcaaggggtcctgtctgccaccatcctctatgagatcttgctagggaaggccaccttgtatgccgtgctggtcagtgccctcgtgctgatggccatggtcaagagaaaggattccagaggcgggagcggagccacgaacttctctctgttaaagcaagcaggagacgtggaagaaaaccccggtcctatgaactcctctctggactttctaattctgatcttaatgtttggaggaactagtggtcaacagctgaatcagagtcctcaatctatgtttatccaggaaggagaagatgtctccatgaactgcacttcttcaagcatatttaacacctggctatggtacaagcaggaacctggggaaggtcctgtcctcttgatagccttatataaggctggtgaattgacctcaaatggaagactgactgctcagtttggtataaccagaaaggacagcttcctgaatatctcagcatccatacctagtgatgtaggcatctacttctgtgctggcacataccagaaagttacctttggaactggaacaaagctccaagtcatcccaaatatccagaaccctgaccctgccgtgtaccagctgagagactctaaatccagtgacaagtctgcatgcctattcaccgattttgattctcaaacaaatgtgtcacaaagtaaggattctgatgtgtatatcacagacaaaactgtgctagacatgaggtctatggacttcaagagcaacagtgctgtggcctggagcaacaaatctgactttgcatgtgcaaacgccttcaacaacagcattattccagaagacaccttcttccccagcccagaaagttcctgtgatgtcaagctggtcgagaaaagctttgaaacagatacgaacctaaactttcaaaacctgtcagtgattgggttccgaatcctcctcctgaaagtggccgggtttaatctgctcatgacgctgcggctgtggtccagctgactcgagggatcccgcccctctccctcccccccccctaacgttactggccgaagccgcttggaataaggccggtgtgcgtttgtctatatgttattttccaccatattgccgtcttttggcaatgtgagggcccggaaacctggccctgtcttcttgacgagcattcctaggggtctttcccctctcgccaaaggaatgcaaggtctgttgaatgtcgtgaaggaagcagttcctctggaagcttcttgaagacaaacaacgtctgtagcgaccctttgcaggcagcggaaccccccacctggcgacaggtgcctctgcggccaaaagccacgtgtataagatacacctgcaaaggcggcacaaccccagtgccacgttgtgagttggatagttgtggaaagagtcaaatggctcacctcaagcgtattcaacaaggggctgaaggatgcccagaaggtaccccattgtatgggatctgatctggggcctcggtgcacatgctttacatgtgtttagtcgaggttaaaaaacgtctaggccccccgaaccacggggacgtggttttcctttgaaaaacacgatgataatatggtgagcaagggcgaggaggataacatggccatcatcaaggagttcatgcgcttcaaggtgcacatggagggctccgtgaacggccacgagttcgagatcgagggcgagggcgagggccgcccctacgagggcacccagaccgccaagctgaaggtgaccaagggtggccccctgcccttcgcctgggacatcctgtcccctcagttcatgtacggctccaaggcctacgtgaagcaccccgccgacatccccgactacttgaagctgtccttccccgagggcttcaagtgggagcgcgtgatgaacttcgaggacggcggcgtggtgaccgtgacccaggactcctccctgcaggacggcgagttcatctacaaggtgaagctgcgcggcaccaacttcccctccgacggccccgtaatgcagaagaagaccatgggctgggaggcctcctccgagcggatgtaccccgaggacggcgccctgaagggcgagatcaagcagaggctgaagctgaaggacggcggccactacgacgctgaggtcaagaccacctacaaggccaagaagcccgtgcagctgcccggcgcctacaacgtcaacatcaagttggacatcacctcccacaacgaggactacaccatcgtggaacagtacgaacgcgccgagggccgccactccaccggcggcatggacgagctgtacaagtgaacgcgtctggaacaagctttttccccgtatccccccaggtgtctgcaggctcaaagagcagcgagaagcgttcagaggaaagcgatcccgtgccaccttccccgtgcccgggctgtccccgcacgctgccggctcggggatgcggggggagcgccggaccggagcggagccccgggcggctcgctgctgccccctagcgggggagggacgtaattacatccctgggggctttgggggggggctgtccccgtgagctcttactccctatcagtgatagagaacgtatgaagagtttactccctatcagtgatagagaacgtatgcagactttactccctatcagtgatagagaacgtataaggagtttactccctatcagtgatagagaacgtatgaccagtttactccctatcagtgatagagaacgtatctacagtttactccctatcagtgatagagaacgtatatccagtttactccctatcagtgatagagaacgtatgtcgaggtaggcgtgtacggtgggcgcctataaaagcagagctcgtttagtgaaccgtcagatcgcctggagcaattccacaacacttttgtcttatacttatgctcgagggagtgcaggtggagactatctccccaggagacgggcgcaccttccccaagcgcggccagacctgcgtggtgcactacaccgggatgcttgaagatggaaagaaagttgattcctcccgggacagaaacaagccctttaagtttatgctaggcaagcaggaggtgatccgaggctgggaagaaggggttgcccagatgagtgtgggtcagagagccaaactgactatatctccagattatgcctatggtgccactgggcacccaggcatcatcccaccacatgccactctcgtcttcgatgtggagcttctaaaactggaatctggcggtggatccggagtcgacggatttggtgatgtcggtgctcttgagagtttgaggggaaatgcagatttggcttacatcctgagcatggagccctgtggccactgcctcattatcaacaatgtgaacttctgccgtgagtccgggctccgcacccgcactggctccaacatcgactgtgagaagttgcggcgtcgcttctcctcgctgcatttcatggtggaggtgaagggcgacctgactgccaagaaaatggtgctggctttgctggagctggcgcggcaggaccacggtgctctggactgctgcgtggtggtcattctctctcacggctgtcaggccagccacctgcagttcccaggggctgtctacggcacagatggatgccctgtgtcggtcgagaagattgtgaacatcttcaatgggaccagctgccccagcctgggagggaagcccaagctctttttcatccaggcctgtggtggggagcagaaagaccatgggtttgaggtggcctccacttcccctgaagacgagtcccctggcagtaaccccgagccagatgccaccccgttccaggaaggtttgaggaccttcgaccagctggacgccatatctagtttgcccacacccagtgacatctttgtgtcctactctactttcccaggttttgtttcctggagggaccccaagagtggctcctggtacgttgagaccctggacgacatctttgagcagtgggctcactctgaagacctgcagtccctcctgcttagggtcgctaatgctgtttcggtgaaagggatttataaacagatgcctggttgctttaatttcctccggaaaaaacttttctttaaaacatcagtcgactatccgtacgacgtaccagactacgcactcgactaaaagctttttccccgtatccccccaggtgtctgcaggctcaaagagcagcgagaagcgttcagaggaaagcgatcccgtgccaccttccccgtgcccgggctgtccccgcacgctgccggctcggggatgcggggggagcgccggaccggagcggagccccgggcggctcgctgctgccccctagcgggggagggacgtaattacatccctgggggctttgggagggggctgtccccgtgagctcaatcaacctctggattacaaaatttgtgaaagattgactggtattcttaactatgttgctccttttacgctatgtggatacgctgctttaatgcctttgtatcatgctattgcttcccgtatggctttcattttctcctccttgtataaatcctggttgctgtctctttatgaggagttgtggcccgttgtcaggcaacgtggcgtggtgtgcactgtgtttgctgacgcaacccccactggttggggcattgccaccacctgtcagctcctttccgggactttcgctttccccctccctattgccacggcggaactcatcgccgcctgccttgcccgctgctggacaggggctcggctgttgggcactgacaattccgtggtgttgtcggggaagctgacgtcctttccatggctgctcgcctgtgttgccacctggattctgcgcgggacgtccttctgctacgtcccttcggccctcaatccagcggaccttccttcccgcggcctgctgccggctctgcggcctcttccgcgtcttcgccttcgccctcagacgagtcggatctccctttgggccgcctccccgcctggaattaattctgcagtcgagacctagaaaaacatggagcaatcacaagtagcaatacagcagctaccaatgctgattgtgcctggctagaagcacaagaggaggaggaggtgggttttccagtcacacctcaggtacctttaagaccaatgacttacaaggcagctgtagatcttagccactttttaaaagaaaagaggggactggaagggctaattcactcccaacgaagacaagatatccttgatctgtggatctaccacacacaaggctacttccctgattagcagaactacacaccagggccaggggtcagatatccactgacctttggatggtgctacaagctagtaccagttgagccagataaggtagaagaggccaataaaggagagaacaccagcttgttacaccctgtgagcctgcatgggatggatgacccggagagagaagtgttagagtggaggtttgacagccgcctagcatttcatcacgtggcccgagagctgcatccggagtacttcaagaactgctgatatcgagcttgctacaagggactttccgctggggactttccagggaggcgtggcctgggcgggactggggagtggcgagccctcagatcctgcatataagcagctgctttttgcctgtactgggtctctctggttagaccagatctgagcctgggagctctctggctaactagggaacccactgcttaagcctcaataaagcttgccttgagtgcttcaagtagtgtgtgcccgtctgttgtgtgactctggtaactagagatccctcagacccttttagtcagtgtggaaaatctctagcagtagtagttcatgtcatcttattattcagtatttataacttgcaaagaaatgaatatcagagagtgagaggccttgacattgctagcgtttaccgtcgacctctagctagagcttggcgtaatcatggtcatagctgtttcctgtgtgaaattgttatccgctcacaattccacacaacatacgagccggaagcataaagtgtaaagcctggggtgcctaatgagtgagctaactcacattaattgcgttgcgctcactgcccgctttccagtcgggaaacctgtcgtgccagctgcattaatgaatcggccaacgcgcggggagaggcggtttgcgtattgggcgctcttccgcttcctcgctcactgactcgctgcgctcggtcgttcggctgcggcgagcggtatcagctcactcaaaggcggtaatacggttatccacagaatcaggggataacgcaggaaagaacatgtgagcaaaaggccagcaaaaggccaggaaccgtaaaaaggccgcgttgctggcgtttttccataggctccgcccccctgacgagcatcacaaaaatcgacgctcaagtcagaggtggcgaaacccgacaggactataaagataccaggcgtttccccctggaagctccctcgtgcgctctcctgttccgaccctgccgcttaccggatacctgtccgcctttctcccttcgggaagcgtggcgctttctcatagctcacgctgtaggtatctcagttcggtgtaggtcgttcgctccaagctgggctgtgtgcacgaaccccccgttcagcccgaccgctgcgccttatccggtaactatcgtcttgagtccaacccggtaagacacgacttatcgccactggcagcagccactggtaacaggattagcagagcgaggtatgtaggcggtgctacagagttcttgaagtggtggcctaactacggctacactagaagaacagtatttggtatctgcgctctgctgaagccagttaccttcggaaaaagagttggtagctcttgatccggcaaacaaaccaccgctggtagcggtggtttttttgtttgcaagcagcagattacgcgcagaaaaaaaggatctcaagaagatcctttgatcttttctacggggtctgacgctcagtggaacgaaaactcacgttaagggattttggtcatgagattatcaaaaaggatcttcacctagatccttttaaattaaaaatgaagttttaaatcaatctaaagtatatatgagtaaacttggtctgacagttaccaatgcttaatcagtgaggcacctatctcagcgatctgtctatttcgttcatccatagttgcctgactccccgtcgtgtagataactacgatacgggagggcttaccatctggccccagtgctgcaatgataccgcgagacccacgctcaccggctccagatttatcagcaataaaccagccagccggaagggccgagcgcagaagtggtcctgcaactttatccgcctccatccagtctattaattgttgccgggaagctagagtaagtagttcgccagttaatagtttgcgcaacgttgttgccattgctacaggcatcgtggtgtcacgctcgtcgtttggtatggcttcattcagctccggttcccaacgatcaaggcgagttacatgatcccccatgttgtgcaaaaaagcggttagctccttcggtcctccgatcgttgtcagaagtaagttggccgcagtgttatcactcatggttatggcagcactgcataattctcttactgtcatgccatccgtaagatgcttttctgtgactggtgagtactcaaccaagtcattctgagaatagtgtatgcggcgaccgagttgctcttgcccggcgtcaatacgggataataccgcgccacatagcagaactttaaaagtgctcatcattggaaaacgttcttcggggcgaaaactctcaaggatcttaccgctgttgagatccagttcgatgtaacccactcgtgcacccaactgatcttcagcatcttttactttcaccagcgtttctgggtgagcaaaaacaggaaggcaaaatgccgcaaaaaagggaataagggcgacacggaaatgttgaatactcatactcttcctttttcaatattattgaagcatttatcagggttattgtctcatgagcggatacatatttgaatgtatttagaaaaataaacaaataggggttccgcgcacatttccccgaaaagtgccacctgacgtcgacggatcgggagatcaacttgtttattgcagcttataatggttacaaataaagcaatagcatcacaaatttcacaaataaagcatttttttcactgcattctagttgtggtttgtccaaactcatcaatgtatcttatcatgtctggatcaactggataactcaagctaaccaaaatcatcccaaacttcccaccccataccctattaccactgccaattacctgtggtttcatttactctaaacctgtgattcctctgaattattttcattttaaagaaattgtatttgttaaatatgtactacaaacttagtagt

SEQ ID NO: 26 - DNA, 9961 bp, synthetic construct
  misc_feature 1..9961: note = Description of Artificial Sequence: Synthetic polynucleotide
  source 1..9961: mol_type = other DNA
tggaagggctaattcactcccaaagaagacaagatatccttgatctgtggatctaccacacacaaggctacttccctgattagcagaactacacaccagggccaggggtcagatatccactgacctttggatggtgctacaagctagtaccagttgagccagataaggtagaagaggccaataaaggagagaacaccagcttgttacaccctgtgagcctgcatgggatggatgacccggagagagaagtgttagagtggaggtttgacagccgcctagcatttcatcacgtggcccgagagctgcatccggagtacttcaagaactgctgatatcgagcttgctacaagggactttccgctggggactttccagggaggcgtggcctgggcgggactggggagtggcgagccctcagatcctgcatataagcagctgctttttgcctgtactgggtctctctggttagaccagatctgagcctgggagctctctggctaactagggaacccactgcttaagcctcaataaagcttgccttgagtgcttcaagtagtgtgtgcccgtctgttgtgtgactctggtaactagagatccctcagacccttttagtcagtgtggaaaatctctagcagtggcgcccgaacagggacttgaaagcgaaagggaaaccagaggagctctctcgacgcaggactcggcttgctgaagcgcgcacggcaagaggcgaggggcggcgactggtgagtacgccaaaaattttgactagcggaggctagaaggagagagatgggtgcgagagcgtcagtattaagcgggggagaattagatcgcgatgggaaaaaattcggttaaggccagggggaaagaaaaaatataaattaaaacatatagtatgggcaagcagggagctagaacgattcgcagttaatcctggcctgttagaaacatcagaaggctgtagacaaatactgggacagctacaaccatcccttcagacaggatcagaagaacttagatcattatataatacagtagcaaccctctattgtgtgcatcaaaggatagagataaaagacaccaaggaagctttagacaagatagaggaagagcaaaacaaaagtaagaccaccgcacagcaagcggccggccgctgatcttcagacctggaggaggagatatgagggacaattggagaagtgaattatataaatataaagtagtaaaaattgaaccattaggagtagcacccaccaaggcaaagagaagagtggtgcagagagaaaaaagagcagtgggaataggagctttgttccttgggttcttgggagcagcaggaagcactatgggcgcagcgtcaatgacgctgacggtacaggccagacaattattgtctggtatagtgcagcagcagaacaatttgctgagggctattgaggcgcaacagcatctgttgcaactcacagtctggggcatcaagcagctccaggcaagaatcctggctgtggaaagatacctaaaggatcaacagctcctggggatttggggttgctctggaaaactcatttgcaccactgctgtgccttggaatgctagttggagtaataaatctctggaacagatttggaatcacacgacctggatggagtgggacagagaaattaacaattacacaagcttaatacactccttaattgaagaatcgcaaaaccagcaagaaaagaatgaacaagaattattggaattagataaatgggcaagtttgtggaattggtttaacataacaaattggctgtggtatataaaattattcataatgatagtaggaggcttggtaggtttaagaatagtttttgctgtactttctatagtgaatagagttaggcagggatattcaccattatcgtttcagacccacctcccaaccccgaggggacccgacaggcccgaaggaatagaagaagaaggtggagagagagacagagacagatccattcgattagtgaacggatctcgacggtatcgcctttaaaagaaaaggggggattggggggtacagtgcaggggaaagaatagtagacataatagcaacagacatacaaactaaagaattacaaaaacaaattacaaaaattcaaaattttcgggtttattacagggacagcagagatccagtttatcgataagcttgggagttccgcgttacataacttacggtaaatggcccgcctggctgaccgcccaacgacccccgcccattgacgtcaataatgacgtatgttcccatagtaacgccaatagggactttccattgacgtcaatgggtggagtatttacggtaaactgcccacttggcagtacatcaagtgtatcatatgccaagtacgccccctattgacgtcaatgacggtaaatggcccgcctggcattatgcccagtacatgaccttatgggactttcctacttggcagtacatctacgtattagtcatcgctattaccatggtgatgcggttttggcagtacatcaatgggcgtggatagcggtttgactcacggggatttccaagtctccaccccattgacgtcaatgggagtttgttttggcaccaaaatcaacgggactttccaaaatgtcgtaacaactccgccccattgacgcaaatgggcggtaggcgtgtacggtgggaggtctatataagcagagctcgtttagtgaaccgtcagatcgcctggagacgccatccacgctgttttgacctccatagaagacaccgactctactagaggatctatttccggtgaattcgccaccatgagcctcgggctcctgtgctgtggggccttttctctcctgtgggcaggaccggtggaagctgacatctaccagaccccaagataccttgttatagggacaggaaagaagatcactctggaatgttctcaaaccatgggccatgacaaaatgtactggtatcaacaagatccaggaatggaactacacctcatccactattcctatggagttaattccacagagaagggagatctttcctctgagtcaacagtctccagaataaggacggagcattttcccctgaccctggagtctgccaggccctcacatacctctcagtacctctgtgccagcagtcggacgcccaacattcagtacttcggcgccgggacccggctctcagtgctggaggacctgaaaaacgtgttcccacccgaactagtcgtgtttgagccatcagaagcagagatctcccacacccaaaaggccacactggtgtgcctggccacaggcttctaccccgaccacgtggagctgagctggtgggtgaatgggaaggaggtgcacagtggggtcagcacagacccgcagcccctcaaggagcagcccgccctcaatgactccagatactgcctgagcagccgcctgagggtctcggccaccttctggcagaacccccgcaaccacttccgctgtcaagtccagttctacgggctctcggagaatgacgagtggacccaggatagggccaaacctgtcacccagatcgtcagcgccgaggcctggggtagagcagactgtggcttcacctccgagtcttaccagcaaggggtcctgtctgccaccatcctctatgagatcttgctagggaaggccaccttgtatgccgtgctggtcagtgccctcgtgctgatggccatggtcaagagaaaggattccagaggcgggagcggagccacgaacttctctctgttaaagcaagcaggagacgtggaagaaaaccccggtcctatgacacgagttagcttgctgtgggcagtcgtggtctccacctgtctcgagtccggcatgggtcaacagctgaatcagagtcctcaatctatgtttatccaggaaggagaagatgtctccatgaactgcacttcttcaagcatatttaacacctggctatggtacaagcaggaacctggggaaggtcctgtcctcttgatagccttatataaggctggtgaattgacctcaaatggaagactgactgctcagtttggtataaccagaaaggacagcttcctgaatatctcagcatccatacctagtgatgtaggcatctacttctgtgctggcacataccagaaagttacctttggaactggaacaaagctccaagtcatcccaaatatccagaaccctgaccctgccgtgtaccagctgagagactctaaatccagtgacaagtctgtctgcctattcaccgattttgattctcaaacaaatgtgtcacaaagtaaggattctgatgtgtatatcacagacaaaactgtgctagacatgaggtctatggacttcaagagcaacagtgctgtggcctggagcaacaaatctgactttgcatgcgcaaacgccttcaacaacagcattattccagaagacaccttcttccccagcccagaaagttcctgtgatgtcaagctggtcgagaaaagctttgaaacagatacgaacctaaactttcaaaacctgtcagtgattgggttccgaatcctcctcctgaaagtggccgggtttaatctgctcatgacgctgcggctgtggtccagctgactcgagggatcccgcccctctccctcccccccccctaacgttactggccgaagccgcttggaataaggccggtgtgcgtttgtctatatgttattttccaccatattgccgtcttttggcaatgtgagggcccggaaacctggccctgtcttcttgacgagcattcctaggggtctttcccctctcgccaaaggaatgcaaggtctgttgaatgtcgtgaaggaagcagttcctctggaagcttcttgaagacaaacaacgtctgtagcgaccctttgcaggcagcggaaccccccacctggcgacaggtgcctctgcggccaaaagccacgtgtataagatacacctgcaaaggcggcacaaccccagtgccacgttgtgagttggatagttgtggaaagagtcaaatggctcacctcaagcgtattcaacaaggggctgaaggatgcccagaaggtaccccattgtatgggatctgatctggggcctcggtgcacatgctttacatgtgtttagtcgaggttaaaaaacgtctaggccccccgaaccacggggacgtggttttcctttgaaaaacacgatgataatatggtgagcaagggcgaggaggataacatggccatcatcaaggagttcatgcgcttcaaggtgcacatggagggctccgtgaacggccacgagttcgagatcgagggcgagggcgagggccgcccctacgagggcacccagaccgccaagctgaaggtgaccaagggtggccccctgcccttcgcctgggacatcctgtcccctcagttcatgtacggctccaaggcctacgtgaagcaccccgccgacatccccgactacttgaagctgtccttccccgagggcttcaagtgggagcgcgtgatgaacttcgaggacggcggcgtggtgaccgtgacccaggactcctccctgcaggacggcgagttcatctacaaggtgaagctgcgcggcaccaacttcccctccgacggccccgtaatgcagaagaagaccatgggctgggaggcctcctccgagcggatgtaccccgaggacggcgccctgaagggcgagatcaagcagaggctgaagctgaaggacggcggccactacgacgctgaggtcaagaccacctacaaggccaagaagcccgtgcagctgcccggcgcctacaacgtcaacatcaagttggacatcacctcccacaacgaggactacaccatcgtggaacagtacgaacgcgccgagggccgccactccaccggcggcatggacgagctgtacaagtgaacgcgtctggaacaatcaacctctggattacaaaatttgtgaaagattgactggtattcttaactatgttgctccttttacgctatgtggatacgctgctttaatgcctttgtatcatgctattgcttcccgtatggctttcattttctcctccttgtataaatcctggttgctgtctctttatgaggagttgtggcccgttgtcaggcaacgtggcgtggtgtgcactgtgtttgctgacgcaacccccactggttggggcattgccaccacctgtcagctcctttccgggactttcgctttccccctccctattgccacggcggaactcatcgccgcctgccttgcccgctgctggacaggggctcggctgttgggcactgacaattccgtggtgttgtcggggaagctgacgtcctttccatggctgctcgcctgtgttgccacctggattctgcgcgggacgtccttctgctacgtcccttcggccctcaatccagcggaccttccttcccgcggcctgctgccggctctgcggcctcttccgcgtcttcgccttcgccctcagacgagtcggatctccctttgggccgcctccccgcctggaattaattctgcagtcgagacctagaaaaacatggagcaatcacaagtagcaatacagcagctaccaatgctgattgtgcctggctagaagcacaagaggaggaggaggtgggttttccagtcacacctcaggtacctttaagaccaatgacttacaaggcagctgtagatcttagccactttttaaaagaaaagaggggactggaagggctaattcactcccaacgaagacaagatatccttgatctgtggatctaccacacacaaggctacttccctgattagcagaactacacaccagggccaggggtcagatatccactgacctttggatggtgctacaagctagtaccagttgagccagataaggtagaagaggccaataaaggagagaacaccagcttgttacaccctgtgagcctgcatgggatggatgacccggagagagaagtgttagagtggaggtttgacagccgcctagcatttcatcacgtggcccgagagctgcatccggagtacttcaagaactgctgatatcgagcttgctacaagggactttccgctggggactttccagggaggcgtggcctgggcgggactggggagtggcgagccctcagatcctgcatataagcagctgctttttgcctgtactgggtctctctggttagaccagatctgagcctgggagctctctggctaactagggaacccactgcttaagcctcaataaagcttgccttgagtgcttcaagtagtgtgtgcccgtctgttgtgtgactctggtaactagagatccctcagacccttttagtcagtgtggaaaatctctagcagtagtagttcatgtcatcttattattcagtatttataacttgcaaagaaatgaatatcagagagtgagaggccttgacattgctagcgtttaccgtcgacctctagctagagcttggcgtaatcatggtcatagctgtttcctgtgtgaaattgttatccgctcacaattccacacaacatacgagccggaagcataaagtgtaaagcctggggtgcctaatgagtgagctaactcacattaattgcgttgcgctcactgcccgctttccagtcgggaaacctgtcgtgccagctgcattaatgaatcggccaacgcgcggggagaggcggtttgcgtattgggcgctcttccgcttcctcgctcactgactcgctgcgctcggtcgttcggctgcggcgagcggtatcagctcactcaaaggcggtaatacggttatccacagaatcaggggataacgcaggaaagaacatgtgagcaaaaggccagcaaaaggccaggaaccgtaaaaaggccgcgttgctggcgtttttccataggctccgcccccctgacgagcatcacaaaaatcgacgctcaagtcagaggtggcgaaacccgacaggactataaagataccaggcgtttccccctggaagctccctcgtgcgctctcctgttccgaccctgccgcttaccggatacctgtccgcctttctcccttcgggaagcgtggcgctttctcatagctcacgctgtaggtatctcagttcggtgtaggtcgttcgctccaagctgggctgtgtgcacgaaccccccgttcagcccgaccgctgcgccttatccggtaactatcgtcttgagtccaacccggtaagacacgacttatcgccactggcagcagccactggtaacaggattagcagagcgaggtatgtaggcggtgctacagagttcttgaagtggtggcctaactacggctacactagaagaacagtatttggtatctgcgctctgctgaagccagttaccttcggaaaaagagttggtagctcttgatccggcaaacaaaccaccgctggtagcggtggtttttttgtttgcaagcagcagattacgcgcagaaaaaaaggatctcaagaagatcctttgatcttttctacggggtctgacgctcagtggaacgaaaactcacgttaagggattttggtcatgagattatcaaaaaggatcttcacctagatccttttaaattaaaaatgaagttttaaatcaatctaaagtatatatgagtaaacttggtctgacagttaccaatgcttaatcagtgaggcacctatctcagcgatctgtctatttcgttcatccatagttgcctgactccccgtcgtgtagataactacgatacgggagggcttaccatctggccccagtgctgcaatgataccgcgagacccacgctcaccggctccagatttatcagcaataaaccagccagccggaagggccgagcgcagaagtggtcctgcaactttatccgcctccatccagtctattaattgttgccgggaagctagagtaagtagttcgccagttaatagtttgcgcaacgttgttgccattgctacaggcatcgtggtgtcacgctcgtcgtttggtatggcttcattcagctccggttcccaacgatcaaggcgagttacatgatcccccatgttgtgcaaaaaagcggttagctccttcggtcctccgatcgttgtcagaagtaagttggccgcagtgttatcactcatggttatggcagcactgcataattctcttactgtcatgccatccgtaagatgcttttctgtgactggtgagtactcaaccaagtcattctgagaatagtgtatgcggcgaccgagttgctcttgcccggcgtcaatacgggataataccgcgccacatagcagaactttaaaagtgctcatcattggaaaacgttcttcggggcgaaaactctcaaggatcttaccgctgttgagatccagttcgatgtaacccactcgtgcacccaactgatcttcagcatcttttactttcaccagcgtttctgggtgagcaaaaacaggaaggcaaaatgccgcaaaaaagggaataagggcgacacggaaatgttgaatactcatactcttcctttttcaatattattgaagcatttatcagggttattgtctcatgagcggatacatatttgaatgtatttagaaaaataaacaaataggggttccgcgcacatttccccgaaaagtgccacctgacgtcgacggatcgggagatcaacttgtttattgcagcttataatggttacaaataaagcaatagcatcacaaatttcacaaataaagcatttttttcactgcattctagttgtggtttgtccaaactcatcaatgtatcttatcatgtctggatcaactggataactcaagctaaccaaaatcatcccaaacttcccaccccataccctattaccactgccaattacctgtggtttcatttactctaaacctgtgattcctctgaattattttcattttaaagaaattgtatttgttaaatatgtactacaaacttagtagt

SEQ ID NO: 27 - DNA, 9955 bp, synthetic construct
  misc_feature 1..9955: note = Description of Artificial Sequence: Synthetic polynucleotide
  source 1..9955: mol_type = other DNA
tggaagggctaattcactcccaaagaagacaagatatccttgatctgtggatctaccacacacaaggctacttccctgattagcagaactacacaccagggccaggggtcagatatccactgacctttggatggtgctacaagctagtaccagttgagccagataaggtagaagaggccaataaaggagagaacaccagcttgttacaccctgtgagcctgcatgggatggatgacccggagagagaagtgttagagtggaggtttgacagccgcctagcatttcatcacgtggcccgagagctgcatccggagtacttcaagaactgctgatatcgagcttgctacaagggactttccgctggggactttccagggaggcgtggcctgggcgggactggggagtggcgagccctcagatcctgcatataagcagctgctttttgcctgtactgggtctctctggttagaccagatctgagcctgggagctctctggctaactagggaacccactgcttaagcctcaataaagcttgccttgagtgcttcaagtagtgtgtgcccgtctgttgtgtgactctggtaactagagatccctcagacccttttagtcagtgtggaaaatctctagcagtggcgcccgaacagggacttgaaagcgaaagggaaaccagaggagctctctcgacgcaggactcggcttgctgaagcgcgcacggcaagaggcgaggggcggcgactggtgagtacgccaaaaattttgactagcggaggctagaaggagagagatgggtgcgagagcgtcagtattaagcgggggagaattagatcgcgatgggaaaaaattcggttaaggccagggggaaagaaaaaatataaattaaaacatatagtatgggcaagcagggagctagaacgattcgcagttaatcctggcctgttagaaacatcagaaggctgtagacaaatactgggacagctacaaccatcccttcagacaggatcagaagaacttagatcattatataatacagtagcaaccctctattgtgtgcatcaaaggatagagataaaagacaccaaggaagctttagacaagatagaggaagagcaaaacaaaagtaagaccaccgcacagcaagcggccggccgctgatcttcagacctggaggaggagatatgagggacaattggagaagtgaattatataaatataaagtagtaaaaattgaaccattaggagtagcacccaccaaggcaaagagaagagtggtgcagagagaaaaaagagcagtgggaataggagctttgttccttgggttcttgggagcagcaggaagcactatgggcgcagcgtcaatgacgctgacggtacaggccagacaattattgtctggtatagtgcagcagcagaacaatttgctgagggctattgaggcgcaacagcatctgttgcaactcacagtctggggcatcaagcagctccaggcaagaatcctggctgtggaaagatacctaaaggatcaacagctcctggggatttggggttgctctggaaaactcatttgcaccactgctgtgccttggaatgctagttggagtaataaatctctggaacagatttggaatcacacgacctggatggagtgggacagagaaattaacaattacacaagcttaatacactccttaattgaagaatcgcaaaaccagcaagaaaagaatgaacaagaattattggaattagataaatgggcaagtttgtggaattggtttaacataacaaattggctgtggtatataaaattattcataatgatagtaggaggcttggtaggtttaagaatagtttttgctgtactttctatagtgaatagagttaggcagggatattcaccattatcgtttcagacccacctcccaaccccgaggggacccgacaggcccgaaggaatagaagaagaaggtggagagagagacagagacagatccattcgattagtgaacggatctcgacggtatcgcctttaaaagaaaaggggggattggggggtacagtgcaggggaaagaatagtagacataatagcaacagacatacaaactaaagaattacaaaaacaaattacaaaaattcaaaattttcgggtttattacagggacagcagagatccagtttatcgataagcttgggagttccgcgttacataacttacggtaaatggcccgcctggctgaccgcccaacgacccccgcccattgacgtcaataatgacgtatgttcccatagtaacgccaatagggactttccattgacgtcaatgggtggagtatttacggtaaactgcccacttggcagtacatcaagtgtatcatatgccaagtacgccccctattgacgtcaatgacggtaaatggcccgcctggcattatgcccagtacatgaccttatgggactttcctacttggcagtacatctacgtattagtcatcgctattaccatggtgatgcggttttggcagtacatcaatgggcgtggatagcggtttgactcacggggatttccaagtctccaccccattgacgtcaatgggagtttgttttggcaccaaaatcaacgggactttccaaaatgtcgtaacaactccgccccattgacgcaaatgggcggtaggcgtgtacggtgggaggtctatataagcagagctcgtttagtgaaccgtcagatcgcctggagacgccatccacgctgttttgacctccatagaagacaccgactctactagaggatctatttccggtgaattcgccaccatgggacccaggctcctcttctgggcactgctttgtctcctcggaaccggtccggttgaagctgacatctaccagaccccaagataccttgttatagggacaggaaagaagatcactctggaatgttctcaaaccatgggccatgacaaaatgtactggtatcaacaagatccaggaatggaactacacctcatccactattcctatggagttaattccacagagaagggagatctttcctctgagtcaacagtctccagaataaggacggagcattttcccctgaccctggagtctgccaggccctcacatacctctcagtacctctgtgccagcagtcggacgcccaacattcagtacttcggcgccgggacccggctctcagtgctggaggacctgaaaaacgtgttcccacccgaggcggccgcgtttgagccatcagaagcagagatctcccacacccaaaaggccacactggtgtgcctggccacaggcttctaccccgaccacgtggagctgagctggtgggtgaatgggaaggaggtgcacagtggggtcagcacagacccgcagcccctcaaggagcagcccgccctcaatgactccagatactgcctgagcagccgcctgagggtctcggccaccttctggcagaacccccgcaaccacttccgctgtcaagtccagttctacgggctctcggagaatgacgagtggacccaggatagggccaaacctgtcacccagatcgtcagcgccgaggcctggggtagagcagactgtggcttcacctccgagtcttaccagcaaggggtcctgtctgccaccatcctctatgagatcttgctagggaaggccaccttgtatgccgtgctggtcagtgccctcgtgctgatggccatggtcaagagaaaggattccagaggcgggagcggagccacgaacttctctctgttaaagcaagcaggagacgtggaagaaaaccccggtcctatgaactcctctctggactttctaattctgatcttaatgtttggaggaactagtggtcaacagctgaatcagagtcctcaatctatgtttatccaggaaggagaagatgtctccatgaactgcacttcttcaagcatatttaacacctggctatggtacaagcaggaacctggggaaggtcctgtcctcttgatagccttatataaggctggtgaattgacctcaaatggaagactgactgctcagtttggtataaccagaaaggacagcttcctgaatatctcagcatccatacctagtgatgtaggcatctacttctgtgctggcacataccagaaagttacctttggaactggaacaaagctccaagtcatcccaaatatccagaaccctgaccctgccgtgtaccagctgagagactctaaatccagtgacaagtctgcatgcctattcaccgattttgattctcaaacaaatgtgtcacaaagtaaggattctgatgtgtatatcacagacaaaactgtgctagacatgaggtctatggacttcaagagcaacagtgctgtggcctggagcaacaaatctgactttgcatgtgcaaacgccttcaacaacagcattattccagaagacaccttcttccccagcccagaaagttcctgtgatgtcaagctggtcgagaaaagctttgaaacagatacgaacctaaactttcaaaacctgtcagtgattgggttccgaatcctcctcctgaaagtggccgggtttaatctgctcatgacgctgcggctgtggtccagctgactcgagggatcccgcccctctccctcccccccccctaacgttactggccgaagccgcttggaataaggccggtgtgcgtttgtctatatgttattttccaccatattgccgtcttttggcaatgtgagggcccggaaacctggccctgtcttcttgacgagcattcctaggggtctttcccctctcgccaaaggaatgcaaggtctgttgaatgtcgtgaaggaagcagttcctctggaagcttcttgaagacaaacaacgtctgtagcgaccctttgcaggcagcggaaccccccacctggcgacaggtgcctctgcggccaaaagccacgtgtataagatacacctgcaaaggcggcacaaccccagtgccacgttgtgagttggatagttgtggaaagagtcaaatggctcacctcaagcgtattcaacaaggggctgaaggatgcccagaaggtaccccattgtatgggatctgatctggggcctcggtgcacatgctttacatgtgtttagtcgaggttaaaaaacgtctaggccccccgaaccacggggacgtggttttcctttgaaaaacacgatgataatatggtgagcaagggcgaggaggataacatggccatcatcaaggagttcatgcgcttcaaggtgcacatggagggctccgtgaacggccacgagttcgagatcgagggcgagggcgagggccgcccctacgagggcacccagaccgccaagctgaaggtgaccaagggtggccccctgcccttcgcctgggacatcctgtcccctcagttcatgtacggctccaaggcctacgtgaagcaccccgccgacatccccgactacttgaagctgtccttccccgagggcttcaagtgggagcgcgtgatgaacttcgaggacggcggcgtggtgaccgtgacccaggactcctccctgcaggacggcgagttcatctacaaggtgaagctgcgcggcaccaacttcccctccgacggccccgtaatgcagaagaagaccatgggctgggaggcctcctccgagcggatgtaccccgaggacggcgccctgaagggcgagatcaagcagaggctgaagctgaaggacggcggccactacgacgctgaggtcaagaccacctacaaggccaagaagcccgtgcagctgcccggcgcctacaacgtcaacatcaagttggacatcacctcccacaacgaggactacaccatcgtggaacagtacgaacgcgccgagggccgccactccaccggcggcatggacgagctgtacaagtgaacgcgtctggaacaatcaacctctggattacaaaatttgtgaaagattgactggtattcttaactatgttgctccttttacgctatgtggatacgctgctttaatgcctttgtatcatgctattgcttcccgtatggctttcattttctcctccttgtataaatcctggttgctgtctctttatgaggagttgtggcccgttgtcaggcaacgtggcgtggtgtgcactgtgtttgctgacgcaacccccactggttggggcattgccaccacctgtcagctcctttccgggactttcgctttccccctccctattgccacggcggaactcatcgccgcctgccttgcccgctgctggacaggggctcggctgttgggcactgacaattccgtggtgttgtcggggaagctgacgtcctttccatggctgctcgcctgtgttgccacctggattctgcgcgggacgtccttctgctacgtcccttcggccctcaatccagcggaccttccttcccgcggcctgctgccggctctgcggcctcttccgcgtcttcgccttcgccctcagacgagtcggatctccctttgggccgcctccccgcctggaattaattctgcagtcgagacctagaaaaacatggagcaatcacaagtagcaatacagcagctaccaatgctgattgtgcctggctagaagcacaagaggaggaggaggtgggttttccagtcacacctcaggtacctttaagaccaatgacttacaaggcagctgtagatcttagccactttttaaaagaaaagaggggactggaagggctaattcactcccaacgaagacaagatatccttgatctgtggatctaccacacacaaggctacttccctgattagcagaactacacaccagggccaggggtcagatatccactgacctttggatggtgctacaagctagtaccagttgagccagataaggtagaagaggccaataaaggagagaacaccagcttgttacaccctgtgagcctgcatgggatggatgacccggagagagaagtgttagagtggaggtttgacagccgcctagcatttcatcacgtggcccgagagctgcatccggagtacttcaagaactgctgatatcgagcttgctacaagggactttccgctggggactttccagggaggcgtggcctgggcgggactggggagtggcgagccctcagatcctgcatataagcagctgctttttgcctgtactgggtctctctggttagaccagatctgagcctgggagctctctggctaactagggaacccactgcttaagcctcaataaagcttgccttgagtgcttcaagtagtgtgtgcccgtctgttgtgtgactctggtaactagagatccctcagacccttttagtcagtgtggaaaatctctagcagtagtagttcatgtcatcttattattcagtatttataacttgcaaagaaatgaatatcagagagtgagaggccttgacattgctagcgtttaccgtcgacctctagctagagcttggcgtaatcatggtcatagctgtttcctgtgtgaaattgttatccgctcacaattccacacaacatacgagccggaagcataaagtgtaaagcctggggtgcctaatgagtgagctaactcacattaattgcgttgcgctcactgcccgctttccagtcgggaaacctgtcgtgccagctgcattaatgaatcggccaacgcgcggggagaggcggtttgcgtattgggcgctcttccgcttcctcgctcactgactcgctgcgctcggtcgttcggctgcggcgagcggtatcagctcactcaaaggcggtaatacggttatccacagaatcaggggataacgcaggaaagaacatgtgagcaaaaggccagcaaaaggccaggaaccgtaaaaaggccgcgttgctggcgtttttccataggctccgcccccctgacgagcatcacaaaaatcgacgctcaagtcagaggtggcgaaacccgacaggactataaagataccaggcgtttccccctggaagctccctcgtgcgctctcctgttccgaccctgccgcttaccggatacctgtccgcctttctcccttcgggaagcgtggcgctttctcatagctcacgctgtaggtatctcagttcggtgtaggtcgttcgctccaagctgggctgtgtgcacgaaccccccgttcagcccgaccgctgcgccttatccggtaactatcgtcttgagtccaacccggtaagacacgacttatcgccactggcagcagccactggtaacaggattagcagagcgaggtatgtaggcggtgctacagagttcttgaagtggtggcctaactacggctacactagaagaacagtatttggtatctgcgctctgctgaagccagttaccttcggaaaaagagttggtagctcttgatccggcaaacaaaccaccgctggtagcggtggtttttttgtttgcaagcagcagattacgcgcagaaaaaaaggatctcaagaagatcctttgatcttttctacggggtctgacgctcagtggaacgaaaactcacgttaagggattttggtcatgagattatcaaaaaggatcttcacctagatccttttaaattaaaaatgaagttttaaatcaatctaaagtatatatgagtaaacttggtctgacagttaccaatgcttaatcagtgaggcacctatctcagcgatctgtctatttcgttcatccatagttgcctgactccccgtcgtgtagataactacgatacgggagggcttaccatctggccccagtgctgcaatgataccgcgagacccacgctcaccggctccagatttatcagcaataaaccagccagccggaagggccgagcgcagaagtggtcctgcaactttatccgcctccatccagtctattaattgttgccgggaagctagagtaagtagttcgccagttaatagtttgcgcaacgttgttgccattgctacaggcatcgtggtgtcacgctcgtcgtttggtatggcttcattcagctccggttcccaacgatcaaggcgagttacatgatcccccatgttgtgcaaaaaagcggttagctccttcggtcctccgatcgttgtcagaagtaagttggccgcagtgttatcactcatggttatggcagcactgcataattctcttactgtcatgccatccgtaagatgcttttctgtgactggtgagtactcaaccaagtcattctgagaatagtgtatgcggcgaccgagttgctcttgcccggcgtcaatacgggataataccgcgccacatagcagaactttaaaagtgctcatcattggaaaacgttcttcggggcgaaaactctcaaggatcttaccgctgttgagatccagttcgatgtaacccactcgtgcacccaactgatcttcagcatcttttactttcaccagcgtttctgggtgagcaaaaacaggaaggcaaaatgccgcaaaaaagggaataagggcgacacggaaatgttgaatactcatactcttcctttttcaatattattgaagcatttatcagggttattgtctcatgagcggatacatatttgaatgtatttagaaaaataaacaaataggggttccgcgcacatttccccgaaaagtgccacctgacgtcgacggatcgggagatcaacttgtttattgcagcttataatggttacaaataaagcaatagcatcacaaatttcacaaataaagcatttttttcactgcattctagttgtggtttgtccaaactcatcaatgtatcttatcatgtctggatcaactggataactcaagctaaccaaaatcatcccaaacttcccaccccataccctattaccactgccaattacctgtggtttcatttactctaaacctgtgattcctctgaattattttcattttaaagaaattgtatttgttaaatatgtactacaaacttagtagt

SEQ ID NO: 28 - DNA, 9961 bp, synthetic construct
  misc_feature 1..9961: note = Description of Artificial Sequence: Synthetic polynucleotide
  source 1..9961: mol_type = other DNA
tggaagggctaattcactcccaaagaagacaagatatccttgatctgtggatctaccacacacaaggctacttccctgattagcagaactacacaccagggccaggggtcagatatccactgacctttggatggtgctacaagctagtaccagttgagccagataaggtagaagaggccaataaaggagagaacaccagcttgttacaccctgtgagcctgcatgggatggatgacccggagagagaagtgttagagtggaggtttgacagccgcctagcatttcatcacgtggcccgagagctgcatccggagtacttcaagaactgctgatatcgagcttgctacaagggactttccgctggggactttccagggaggcgtggcctgggcgggactggggagtggcgagccctcagatcctgcatataagcagctgctttttgcctgtactgggtctctctggttagaccagatctgagcctgggagctctctggctaactagggaacccactgcttaagcctcaataaagcttgccttgagtgcttcaagtagtgtgtgcccgtctgttgtgtgactctggtaactagagatccctcagacccttttagtcagtgtggaaaatctctagcagtggcgcccgaacagggacttgaaagcgaaagggaaaccagaggagctctctcgacgcaggactcggcttgctgaagcgcgcacggcaagaggcgaggggcggcgactggtgagtacgccaaaaattttgactagcggaggctagaaggagagagatgggtgcgagagcgtcagtattaagcgggggagaattagatcgcgatgggaaaaaattcggttaaggccagggggaaagaaaaaatataaattaaaacatatagtatgggcaagcagggagctagaacgattcgcagttaatcctggcctgttagaaacatcagaaggctgtagacaaatactgggacagctacaaccatcccttcagacaggatcagaagaacttagatcattatataatacagtagcaaccctctattgtgtgcatcaaaggatagagataaaagacaccaaggaagctttagacaagatagaggaagagcaaaacaaaagtaagaccaccgcacagcaagcggccggccgctgatcttcagacctggaggaggagatatgagggacaattggagaagtgaattatataaatataaagtagtaaaaattgaaccattaggagtagcacccaccaaggcaaagagaagagtggtgcagagagaaaaaagagcagtgggaataggagctttgttccttgggttcttgggagcagcaggaagcactatgggcgcagcgtcaatgacgctgacggtacaggccagacaattattgtctggtatagtgcagcagcagaacaatttgctgagggctattgaggcgcaacagcatctgttgcaactcacagtctggggcatcaagcagctccaggcaagaatcctggctgtggaaagatacctaaaggatcaacagctcctggggatttggggttgctctggaaaactcatttgcaccactgctgtgccttggaatgctagttggagtaataaatctctggaacagatttggaatcacacgacctggatggagtgggacagagaaattaacaattacacaagcttaatacactccttaattgaagaatcgcaaaaccagcaagaaaagaatgaacaagaattattggaattagataaatgggcaagtttgtggaattggtttaacataacaaattggctgtggtatataaaattattcataatgatagtaggaggcttggtaggtttaagaatagtttttgctgtactttctatagtgaatagagttaggcagggatattcaccattatcgtttcagacccacctcccaaccccgaggggacccgacaggcccgaaggaatagaagaagaaggtggagagagagacagagacagatccattcgattagtgaacggatctcgacggtatcgcctttaaaagaaaaggggggattggggggtacagtgcaggggaaagaatagtagacataatagcaacagacatacaaactaaagaattacaaaaacaaattacaaaaattcaaaattttcgggtttattacagggacagcagagatccagtttatcgataagcttgggagttccgcgttacataacttacggtaaatggcccgcctggctgaccgcccaacgacccccgcccattgacgtcaataatgacgtatgttcccatagtaacgccaatagggactttccattgacgtcaatgggtggagtatttacggtaaactgcccacttggcagtacatcaagtgtatcatatgccaagtacgccccctattgacgtcaatgacggtaaatggcccgcctggcattatgcccagtacatgaccttatgggactttcctacttggcagtacatctacgtattagtcatcgctattaccatggtgatgcggttttggcagtacatcaatgggcgtggatagcggtttgactcacggggatttccaagtctccaccccattgacgtcaatgggagtttgttttggcaccaaaatcaacgggactttccaaaatgtcgtaacaactccgccccattgacgcaaatgggcggtaggcgtgtacggtgggaggtctatataagcagagctcgtttagtgaaccgtcagatcgcctggagacgccatccacgctgttttgacctccatagaagacaccgactctactagaggatctatttccggtgaattcgccaccatgggcacaaggttgttcttctatgtggccctttgtctcctgtggaccggtcacatggaagctgacatctaccagaccccaagataccttgttatagggacaggaaagaagatcactctggaatgttctcaaaccatgggccatgacaaaatgtactggtatcaacaagatccaggaatggaactacacctcatccactattcctatggagttaattccacagagaagggagatctttcctctgagtcaacagtctccagaataaggacggagcattttcccctgaccctggagtctgccaggccctcacatacctctcagtacctctgtgccagcagtcggacgcccaacattcagtacttcggcgccgggacccggctctcagtgctggaggacctgaaaaacgtgttcccacccgaggtcgctgtgtttgagccatcagaagcagagatctcccacacccaaaaggccacactagtgtgcctggccacaggcttctaccccgaccacgtggagctgagctggtgggtgaatgggaaggaggtgcacagtggggtcagcacagacccgcagcccctcaaggagcagcccgccctcaatgactccagatactgcctgagcagccgcctgagggtctcggccaccttctggcagaacccccgcaaccacttccgctgtcaagtccagttctacgggctctcggagaatgacgagtggacccaggatagggccaaacctgtcacccagatcgtcagcgccgaggcctggggtagagcagactgtggcttcacctccgagtcttaccagcaaggggtcctgtctgccaccatcctctatgagatcttgctagggaaggccaccttgtatgccgtgctggtcagtgccctcgtgctgatggccatggtcaagagaaaggattccagaggcgggagcggagccacgaacttctctctgttaaagcaagcaggagacgtggaagaaaaccccggtcctatggcaggcattcgagctttatttatgtacttgtggctgcagctggactgggtctcgagaggtcaacagctgaatcagagtcctcaatctatgtttatccaggaaggagaagatgtctccatgaactgcacttcttcaagcatatttaacacctggctatggtacaagcaggaacctggggaaggtcctgtcctcttgatagccttatataaggctggtgaattgacctcaaatggaagactgactgctcagtttggtataaccagaaaggacagcttcctgaatatctcagcatccatacctagtgatgtaggcatctacttctgtgctggcacataccagaaagttacctttggaactggaacaaagctccaagtcatcccaaatatccagaaccctgaccctgccgtgtaccagctgagagactctaaatccagtgacaagtctgtctgcctattcaccgattttgattctcaaacaaatgtgtcacaaagtaaggattctgatgtgtatatcacagacaaaactgtgctagacatgaggtctatggacttcaagagcaacagtgcggccgcctggagcaacaaatctgactttgcatgtgcaaacgccttcaacaacagcattattccagaagacaccttcttccccagcccagaaagttcctgtgatgtcaagctggtcgagaaaagctttgaaacagatacgaacctaaactttcaaaacctgtcagtgattgggttccgaatcctcctcctgaaagtggccgggtttaatctgctcatgacgctgcggctgtggtccagctgactcgagggatcccgcccctctccctcccccccccctaacgttactggccgaagccgcttggaataaggccggtgtgcgtttgtctatatgttattttccaccatattgccgtcttttggcaatgtgagggcccggaaacctggccctgtcttcttgacgagcattcctaggggtctttcccctctcgccaaaggaatgcaaggtctgttgaatgtcgtgaaggaagcagttcctctggaagcttcttgaagacaaacaacgtctgtagcgaccctttgcaggcagcggaaccccccacctggcgacaggtgcctctgcggccaaaagccacgtgtataagatacacctgcaaaggcggcacaaccccagtgccacgttgtgagttggatagttgtggaaagagtcaaatggctcacctcaagcgtattcaacaaggggctgaaggatgcccagaaggtaccccattgtatgggatctgatctggggcctcggtgcacatgctttacatgtgtttagtcgaggttaaaaaacgtctaggccccccgaaccacggggacgtggttttcctttgaaaaacacgatgataatatggtgagcaagggcgaggaggataacatggccatcatcaaggagttcatgcgcttcaaggtgcacatggagggctccgtgaacggccacgagttcgagatcgagggcgagggcgagggccgcccctacgagggcacccagaccgccaagctgaaggtgaccaagggtggccccctgcccttcgcctgggacatcctgtcccctcagttcatgtacggctccaaggcctacgtgaagcaccccgccgacatccccgactacttgaagctgtccttccccgagggcttcaagtgggagcgcgtgatgaacttcgaggacggcggcgtggtgaccgtgacccaggactcctccctgcaggacggcgagttcatctacaaggtgaagctgcgcggcaccaacttcccctccgacggccccgtaatgcagaagaagaccatgggctgggaggcctcctccgagcggatgtaccccgaggacggcgccctgaagggcgagatcaagcagaggctgaagctgaaggacggcggccactacgacgctgaggtcaagaccacctacaaggccaagaagcccgtgcagctgcccggcgcctacaacgtcaacatcaagttggacatcacctcccacaacgaggactacaccatcgtggaacagtacgaacgcgccgagggccgccactccaccggcggcatggacgagctgtacaagtgaacgcgtctggaacaatcaacctctggattacaaaatttgtgaaagattgactggtattcttaactatgttgctccttttacgctatgtggatacgctgctttaatgcctttgtatcatgctattgcttcccgtatggctttcattttctcctccttgtataaatcctggttgctgtctctttatgaggagttgtggcccgttgtcaggcaacgtggcgtggtgtgcactgtgtttgctgacgcaacccccactggttggggcattgccaccacctgtcagctcctttccgggactttcgctttccccctccctattgccacggcggaactcatcgccgcctgccttgcccgctgctggacaggggctcggctgttgggcactgacaattccgtggtgttgtcggggaagctgacgtcctttccatggctgctcgcctgtgttgccacctggattctgcgcgggacgtccttctgctacgtcccttcggccctcaatccagcggaccttccttcccgcggcctgctgccggctctgcggcctcttccgcgtcttcgccttcgccctcagacgagtcggatctccctttgggccgcctccccgcctggaattaattctgcagtcgagacctagaaaaacatggagcaatcacaagtagcaatacagcagctaccaatgctgattgtgcctggctagaagcacaagaggaggaggaggtgggttttccagtcacacctcaggtacctttaagaccaatgacttacaaggcagctgtagatcttagccactttttaaaagaaaagaggggactggaagggctaattcactcccaacgaagacaagatatccttgatctgtggatctaccacacacaaggctacttccctgattagcagaactacacaccagggccaggggtcagatatccactgacctttggatggtgctacaagctagtaccagttgagccagataaggtagaagaggccaataaaggagagaacaccagcttgttacaccctgtgagcctgcatgggatggatgacccggagagagaagtgttagagtggaggtttgacagccgcctagcatttcatcacgtggcccgagagctgcatccggagtacttcaagaactgctgatatcgagcttgctacaagggactttccgctggggactttccagggaggcgtggcctgggcgggactggggagtggcgagccctcagatcctgcatataagcagctgctttttgcctgtactgggtctctctggttagaccagatctgagcctgggagctctctggctaactagggaacccactgcttaagcctcaataaagcttgccttgagtgcttcaagtagtgtgtgcccgtctgttgtgtgactctggtaactagagatccctcagacccttttagtcagtgtggaaaatctctagcagtagtagttcatgtcatcttattattcagtatttataacttgcaaagaaatgaatatcagagagtgagaggccttgacattgctagcgtttaccgtcgacctctagctagagcttggcgtaatcatggtcatagctgtttcctgtgtgaaattgttatccgctcacaattccacacaacatacgagccggaagcataaagtgtaaagcctggggtgcctaatgagtgagctaactcacattaattgcgttgcgctcactgcccgctttccagtcgggaaacctgtcgtgccagctgcattaatgaatcggccaacgcgcggggagaggcggtttgcgtattgggcgctcttccgcttcctcgctcactgactcgctgcgctcggtcgttcggctgcggcgagcggtatcagctcactcaaaggcggtaatacggttatccacagaatcaggggataacgcaggaaagaacatgtgagcaaaaggccagcaaaaggccaggaaccgtaaaaaggccgcgttgctggcgtttttccataggctccgcccccctgacgagcatcacaaaaatcgacgctcaagtcagaggtggcgaaacccgacaggactataaagataccaggcgtttccccctggaagctccctcgtgcgctctcctgttccgaccctgccgcttaccggatacctgtccgcctttctcccttcgggaagcgtggcgctttctcatagctcacgctgtaggtatctcagttcggtgtaggtcgttcgctccaagctgggctgtgtgcacgaaccccccgttcagcccgaccgctgcgccttatccggtaactatcgtcttgagtccaacccggtaagacacgacttatcgccactggcagcagccactggtaacaggattagcagagcgaggtatgtaggcggtgctacagagttcttgaagtggtggcctaactacggctacactagaagaacagtatttggtatctgcgctctgctgaagccagttaccttcggaaaaagagttggtagctcttgatccggcaaacaaaccaccgctggtagcggtggtttttttgtttgcaagcagcagattacgcgcagaaaaaaaggatctcaagaagatcctttgatcttttctacggggtctgacgctcagtggaacgaaaactcacgttaagggattttggtcatgagattatcaaaaaggatcttcacctagatccttttaaattaaaaatgaagttttaaatcaatctaaagtatatatgagtaaacttggtctgacagttaccaatgcttaatcagtgaggcacctatctcagcgatctgtctatttcgttcatccatagttgcctgactccccgtcgtgtagataactacgatacgggagggcttaccatctggccccagtgctgcaatgataccgcgagacccacgctcaccggctccagatttatcagcaataaaccagccagccggaagggccgagcgcagaagtggtcctgcaactttatccgcctccatccagtctattaattgttgccgggaagctagagtaagtagttcgccagttaatagtttgcgcaacgttgttgccattgctacaggcatcgtggtgtcacgctcgtcgtttggtatggcttcattcagctccggttcccaacgatcaaggcgagttacatgatcccccatgttgtgcaaaaaagcggttagctccttcggtcctccgatcgttgtcagaagtaagttggccgcagtgttatcactcatggttatggcagcactgcataattctcttactgtcatgccatccgtaagatgcttttctgtgactggtgagtactcaaccaagtcattctgagaatagtgtatgcggcgaccgagttgctcttgcccggcgtcaatacgggataataccgcgccacatagcagaactttaaaagtgctcatcattggaaaacgttcttcggggcgaaaactctcaaggatcttaccgctgttgagatccagttcgatgtaacccactcgtgcacccaactgatcttcagcatcttttactttcaccagcgtttctgggtgagcaaaaacaggaaggcaaaatgccgcaaaaaagggaataagggcgacacggaaatgttgaatactcatactcttcctttttcaatattattgaagcatttatcagggttattgtctcatgagcggatacatatttgaatgtatttagaaaaataaacaaataggggttccgcgcacatttccccgaaaagtgccacctgacgtcgacggatcgggagatcaacttgtttattgcagcttataatggttacaaataaagcaatagcatcacaaatttcacaaataaagcatttttttcactgcattctagttgtggtttgtccaaactcatcaatgtatcttatcatgtctggatcaactggataactcaagctaaccaaaatcatcccaaacttcccaccccataccctattaccactgccaattacctgtggtttcatttactctaaacctgtgattcctctgaattattttcattttaaagaaattgtatttgttaaatatgtactacaaacttagtagt

SEQ ID NO: 29 - DNA, 9961 bp, synthetic construct
  misc_feature 1..9961: note = Description of Artificial Sequence: Synthetic polynucleotide
  source 1..9961: mol_type = other DNA
tggaagggctaattcactcccaaagaagacaagatatccttgatctgtggatctaccacacacaaggctacttccctgattagcagaactacacaccagggccaggggtcagatatccactgacctttggatggtgctacaagctagtaccagttgagccagataaggtagaagaggccaataaaggagagaacaccagcttgttacaccctgtgagcctgcatgggatggatgacccggagagagaagtgttagagtggaggtttgacagccgcctagcatttcatcacgtggcccgagagctgcatccggagtacttcaagaactgctgatatcgagcttgctacaagggactttccgctggggactttccagggaggcgtggcctgggcgggactggggagtggcgagccctcagatcctgcatataagcagctgctttttgcctgtactgggtctctctggttagaccagatctgagcctgggagctctctggctaactagggaacccactgcttaagcctcaataaagcttgccttgagtgcttcaagtagtgtgtgcccgtctgttgtgtgactctggtaactagagatccctcagacccttttagtcagtgtggaaaatctctagcagtggcgcccgaacagggacttgaaagcgaaagggaaaccagaggagctctctcgacgcaggactcggcttgctgaagcgcgcacggcaagaggcgaggggcggcgactggtgagtacgccaaaaattttgactagcggaggctagaaggagagagatgggtgcgagagcgtcagtattaagcgggggagaattagatcgcgatgggaaaaaattcggttaaggccagggggaaagaaaaaatataaattaaaacatatagtatgggcaagcagggagctagaacgattcgcagttaatcctggcctgttagaaacatcagaaggctgtagacaaatactgggacagctacaaccatcccttcagacaggatcagaagaacttagatcattatataatacagtagcaaccctctattgtgtgcatcaaaggatagagataaaagacaccaaggaagctttagacaagatagaggaagagcaaaacaaaagtaagaccaccgcacagcaagcggccggccgctgatcttcagacctggaggaggagatatgagggacaattggagaagtgaattatataaatataaagtagtaaaaattgaaccattaggagtagcacccaccaaggcaaagagaagagtggtgcagagagaaaaaagagcagtgggaataggagctttgttccttgggttcttgggagcagcaggaagcactatgggcgcagcgtcaatgacgctgacggtacaggccagacaattattgtctggtatagtgcagcagcagaacaatttgctgagggctattgaggcgcaacagcatctgttgcaactcacagtctggggcatcaagcagctccaggcaagaatcctggctgtggaaagatacctaaaggatcaacagctcctggggatttggggttgctctggaaaactcatttgcaccactgctgtgccttggaatgctagttggagtaataaatctctggaacagatttggaatcacacgacctggatggagtgggacagagaaattaacaattacacaagcttaatacactccttaattgaagaatcgcaaaaccagcaagaaaagaatgaacaagaattattggaattagataaatgggcaagtttgtggaattggtttaacataacaaattggctgtggtatataaaattattcataatgatagtaggaggcttggtaggtttaagaatagtttttgctgtactttctatagtgaatagagttaggcagggatattcaccattatcgtttcagacccacctcccaaccccgaggggacccgacaggcccgaaggaatagaagaagaaggtggagagagagacagagacagatccattcgattagtgaacggatctcgacggtatcgcctttaaaagaaaaggggggattggggggtacagtgcaggggaaagaatagtagacataatagcaacagacatacaaactaaagaattacaaaaacaaattacaaaaattcaaaattttcgggtttattacagggacagcagagatccagtttatcgataagcttgggagttccgcgttacataacttacggtaaatggcccgcctggctgaccgcccaacgacccccgcccattgacgtcaataatgacgtatgttcccatagtaacgccaatagggactttccattgacgtcaatgggtggagtatttacggtaaactgcccacttggcagtacatcaagtgtatcatatgccaagtacgccccctattgacgtcaatgacggtaaatggcccgcctggcattatgcccagtacatgaccttatgggactttcctacttggcagtacatctacgtattagtcatcgctattaccatggtgatgcggttttggcagtacatcaatgggcgtggatagcggtttgactcacggggatttccaagtctccaccccattgacgtcaatgggagtttgttttggcaccaaaatcaacgggactttccaaaatgtcgtaacaactccgccccattgacgcaaatgggcggtaggcgtgtacggtgggaggtctatataagcagagctcgtttagtgaaccgtcagatcgcctggagacgccatccacgctgttttgacctccatagaagacaccgactctactagaggatctatttccggtgaattcgccaccatgggaatcaggctcctgtgtcgtgtggccttttgtttcctggctgtaggactagtagaagctgacatctaccagaccccaagataccttgttatagggacaggaaagaagatcactctggaatgttctcaaaccatgggccatgacaaaatgtactggtatcaacaagatccaggaatggaactacacctcatccactattcctatggagttaattccacagagaagggagatctttcctctgagtcaacagtctccagaataaggacggagcattttcccctgaccctggagtctgccaggccctcacatacctctcagtacctctgtgccagcagtcggacgcccaacattcagtacttcggcgccgggacccggctctcagtgctggaggacctgaaaaacgtgttcccacccgaggtcgctgtgtttgagccatcagaagcagagatctcccacacccaaaaggccacactggcatgcctggccacaggcttctaccccgaccacgtggagctgagctggtgggtgaatgggaaggaggtgcacagtggggtcagcacagacccgcagcccctcaaggagcagcccgccctcaatgactccagatactgcctgagcagccgcctgagggtctcggccaccttctggcagaacccccgcaaccacttccgctgtcaagtccagttctacgggctctcggagaatgacgagtggacccaggatagggccaaacctgtcacccagatcgtcagcgccgaggcctggggtagagcagactgtggcttcacctccgagtcttaccagcaaggggtcctgtctgccaccatcctctatgagatcttgctagggaaggccaccttgtatgccgtgctggtcagtgccctcgtgctgatggccatggtcaagagaaaggattccagaggcgggagcggagccacgaacttctctctgttaaagcaagcaggagacgtggaagaaaaccccggtcctatgacacgagttagcttgctgtgggcagtcgtggtctccacctgtctcgagtccggcatgggtcaacagctgaatcagagtcctcaatctatgtttatccaggaaggagaagatgtctccatgaactgcacttcttcaagcatatttaacacctggctatggtacaagcaggaacctggggaaggtcctgtcctcttgatagccttatataaggctggtgaattgacctcaaatggaagactgactgctcagtttggtataaccagaaaggacagcttcctgaatatctcagcatccatacctagtgatgtaggcatctacttctgtgctggcacataccagaaagttacctttggaactggaacaaagctccaagtcatcccaaatatccagaaccctgaccctgccgtgtaccagctgagagactctaaatccagtgacaagtctgtctgcctattcaccgattttgattctcaaacaaatgtgtcacaaagtaaggattctgatgtgtatatcacagacaaaactgtgctagacatgaggtctatggacttcaagagcaacagtgcggccgcctggagcaacaaatctgactttgcatgtgcaaacgccttcaacaacagcattattccagaagacaccttcttccccagcccagaaagttcctgtgatgtcaagctggtcgagaaaagctttgaaacagatacgaacctaaactttcaaaacctgtcagtgattgggttccgaatcctcctcctgaaagtggccgggtttaatctgctcatgacgctgcggctgtggtccagctgactcgagggatcccgcccctctccctcccccccccctaacgttactggccgaagccgcttggaataaggccggtgtgcgtttgtctatatgttattttccaccatattgccgtcttttggcaatgtgagggcccggaaacctggccctgtcttcttgacgagcattcctaggggtctttcccctctcgccaaaggaatgcaaggtctgttgaatgtcgtgaaggaagcagttcctctggaagcttcttgaagacaaacaacgtctgtagcgaccctttgcaggcagcggaaccccccacctggcgacaggtgcctctgcggccaaaagccacgtgtataagatacacctgcaaaggcggcacaaccccagtgccacgttgtgagttggatagttgtggaaagagtcaaatggctcacctcaagcgtattcaacaaggggctgaaggatgcccagaaggtaccccattgtatgggatctgatctggggcctcggtgcacatgctttacatgtgtttagtcgaggttaaaaaacgtctaggccccccgaaccacggggacgtggttttcctttgaaaaacacgatgataatatggtgagcaagggcgaggaggataacatggccatcatcaaggagttcatgcgcttcaaggtgcacatggagggctccgtgaacggccacgagttcgagatcgagggcgagggcgagggccgcccctacgagggcacccagaccgccaagctgaaggtgaccaagggtggccccctgcccttcgcctgggacatcctgtcccctcagttcatgtacggctccaaggcctacgtgaagcaccccgccgacatccccgactacttgaagctgtccttccccgagggcttcaagtgggagcgcgtgatgaacttcgaggacggcggcgtggtgaccgtgacccaggactcctccctgcaggacggcgagttcatctacaaggtgaagctgcgcggcaccaacttcccctccgacggccccgtaatgcagaagaagaccatgggctgggaggcctcctccgagcggatgtaccccgaggacggcgccctgaagggcgagatcaagcagaggctgaagctgaaggacggcggccactacgacgctgaggtcaagaccacctacaaggccaagaagcccgtgcagctgcccggcgcctacaacgtcaacatcaagttggacatcacctcccacaacgaggactacaccatcgtggaacagtacgaacgcgccgagggccgccactccaccggcggcatggacgagctgtacaagtgaacgcgtctggaacaatcaacctctggattacaaaatttgtgaaagattgactggtattcttaactatgttgctccttttacgctatgtggatacgctgctttaatgcctttgtatcatgctattgcttcccgtatggctttcattttctcctccttgtataaatcctggttgctgtctctttatgaggagttgtggcccgttgtcaggcaacgtggcgtggtgtgcactgtgtttgctgacgcaacccccactggttggggcattgccaccacctgtcagctcctttccgggactttcgctttccccctccctattgccacggcggaactcatcgccgcctgccttgcccgctgctggacaggggctcggctgttgggcactgacaattccgtggtgttgtcggggaagctgacgtcctttccatggctgctcgcctgtgttgccacctggattctgcgcgggacgtccttctgctacgtcccttcggccctcaatccagcggaccttccttcccgcggcctgctgccggctctgcggcctcttccgcgtcttcgccttcgccctcagacgagtcggatctccctttgggccgcctccccgcctggaattaattctgcagtcgagacctagaaaaacatggagcaatcacaagtagcaatacagcagctaccaatgctgattgtgcctggctagaagcacaagaggaggaggaggtgggttttccagtcacacctcaggtacctttaagaccaatgacttacaaggcagctgtagatcttagccactttttaaaagaaaagaggggactggaagggctaattcactcccaacgaagacaagatatccttgatctgtggatctaccacacacaaggctacttccctgattagcagaactacacaccagggccaggggtcagatatccactgacctttggatggtgctacaagctagtaccagttgagccagataaggtagaagaggccaataaaggagagaacaccagcttgttacaccctgtgagcctgcatgggatggatgacccggagagagaagtgttagagtggaggtttgacagccgcctagcatttcatcacgtggcccgagagctgcatccggagtacttcaagaactgctgatatcgagcttgctacaagggactttccgctggggactttccagggaggcgtggcctgggcgggactggggagtggcgagccctcagatcctgcatataagcagctgctttttgcctgtactgggtctctctggttagaccagatctgagcctgggagctctctggctaactagggaacccactgcttaagcctcaataaagcttgccttgagtgcttcaagtagtgtgtgcccgtctgttgtgtgactctggtaactagagatccctcagacccttttagtcagtgtggaaaatctctagcagtagtagttcatgtcatcttattattcagtatttataacttgcaaagaaatgaatatcagagagtgagaggccttgacattgctagcgtttaccgtcgacctctagctagagcttggcgtaatcatggtcatagctgtttcctgtgtgaaattgttatccgctcacaattccacacaacatacgagccggaagcataaagtgtaaagcctggggtgcctaatgagtgagctaactcacattaattgcgttgcgctcactgcccgctttccagtcgggaaacctgtcgtgccagctgcattaatgaatcggccaacgcgcggggagaggcggtttgcgtattgggcgctcttccgcttcctcgctcactgactcgctgcgctcggtcgttcggctgcggcgagcggtatcagctcactcaaaggcggtaatacggttatccacagaatcaggggataacgcaggaaagaacatgtgagcaaaaggccagcaaaaggccaggaaccgtaaaaaggccgcgttgctggcgtttttccataggctccgcccccctgacgagcatcacaaaaatcgacgctcaagtcagaggtggcgaaacccgacaggactataaagataccaggcgtttccccctggaagctccctcgtgcgctctcctgttccgaccctgccgcttaccggatacctgtccgcctttctcccttcgggaagcgtggcgctttctcatagctcacgctgtaggtatctcagttcggtgtaggtcgttcgctccaagctgggctgtgtgcacgaaccccccgttcagcccgaccgctgcgccttatccggtaactatcgtcttgagtccaacccggtaagacacgacttatcgccactggcagcagccactggtaacaggattagcagagcgaggtatgtaggcggtgctacagagttcttgaagtggtggcctaactacggctacactagaagaacagtatttggtatctgcgctctgctgaagccagttaccttcggaaaaagagttggtagctcttgatccggcaaacaaaccaccgctggtagcggtggtttttttgtttgcaagcagcagattacgcgcagaaaaaaaggatctcaagaagatcctttgatcttttctacggggtctgacgctcagtggaacgaaaactcacgttaagggattttggtcatgagattatcaaaaaggatcttcacctagatccttttaaattaaaaatgaagttttaaatcaatctaaagtatatatgagtaaacttggtctgacagttaccaatgcttaatcagtgaggcacctatctcagcgatctgtctatttcgttcatccatagttgcctgactccccgtcgtgtagataactacgatacgggagggcttaccatctggccccagtgctgcaatgataccgcgagacccacgctcaccggctccagatttatcagcaataaaccagccagccggaagggccgagcgcagaagtggtcctgcaactttatccgcctccatccagtctattaattgttgccgggaagctagagtaagtagttcgccagttaatagtttgcgcaacgttgttgccattgctacaggcatcgtggtgtcacgctcgtcgtttggtatggcttcattcagctccggttcccaacgatcaaggcgagttacatgatcccccatgttgtgcaaaaaagcggttagctccttcggtcctccgatcgttgtcagaagtaagttggccgcagtgttatcactcatggttatggcagcactgcataattctcttactgtcatgccatccgtaagatgcttttctgtgactggtgagtactcaaccaagtcattctgagaatagtgtatgcggcgaccgagttgctcttgcccggcgtcaatacgggataataccgcgccacatagcagaactttaaaagtgctcatcattggaaaacgttcttcggggcgaaaactctcaaggatcttaccgctgttgagatccagttcgatgtaacccactcgtgcacccaactgatcttcagcatcttttactttcaccagcgtttctgggtgagcaaaaacaggaaggcaaaatgccgcaaaaaagggaataagggcgacacggaaatgttgaatactcatactcttcctttttcaatattattgaagcatttatcagggttattgtctcatgagcggatacatatttgaatgtatttagaaaaataaacaaataggggttccgcgcacatttccccgaaaagtgccacctgacgtcgacggatcgggagatcaacttgtttattgcagcttataatggttacaaataaagcaatagcatcacaaatttcacaaataaagcatttttttcactgcattctagttgtggtttgtccaaactcatcaatgtatcttatcatgtctggatcaactggataactcaagctaaccaaaatcatcccaaacttcccaccccataccctattaccactgccaattacctgtggtttcatttactctaaacctgtgattcctctgaattattttcattttaaagaaattgtatttgttaaatatgtactacaaacttagtagt

SEQ ID NO: 30 - DNA, 9955 bp, synthetic construct
  misc_feature 1..9955: note = Description of Artificial Sequence: Synthetic polynucleotide
  source 1..9955: mol_type = other DNA
tggaagggctaattcactcccaaagaagacaagatatccttgatctgtggatctaccacacacaaggctacttccctgattagcagaactacacaccagggccaggggtcagatatccactgacctttggatggtgctacaagctagtaccagttgagccagataaggtagaagaggccaataaaggagagaacaccagcttgttacaccctgtgagcctgcatgggatggatgacccggagagagaagtgttagagtggaggtttgacagccgcctagcatttcatcacgtggcccgagagctgcatccggagtacttcaagaactgctgatatcgagcttgctacaagggactttccgctggggactttccagggaggcgtggcctgggcgggactggggagtggcgagccctcagatcctgcatataagcagctgctttttgcctgtactgggtctctctggttagaccagatctgagcctgggagctctctggctaactagggaacccactgcttaagcctcaataaagcttgccttgagtgcttcaagtagtgtgtgcccgtctgttgtgtgactctggtaactagagatccctcagacccttttagtcagtgtggaaaatctctagcagtggcgcccgaacagggacttgaaagcgaaagggaaaccagaggagctctctcgacgcaggactcggcttgctgaagcgcgcacggcaagaggcgaggggcggcgactggtgagtacgccaaaaattttgactagcggaggctagaaggagagagatgggtgcgagagcgtcagtattaagcgggggagaattagatcgcgatgggaaaaaattcggttaaggccagggggaaagaaaaaatataaattaaaacatatagtatgggcaagcagggagctagaacgattcgcagttaatcctggcctgttagaaacatcagaaggctgtagacaaatactgggacagctacaaccatcccttcagacaggatcagaagaacttagatcattatataatacagtagcaaccctctattgtgtgcatcaaaggatagagataaaagacaccaaggaagctttagacaagatagaggaagagcaaaacaaaagtaagaccaccgcacagcaagcggccggccgctgatcttcagacctggaggaggagatatgagggacaattggagaagtgaattatataaatataaagtagtaaaaattgaaccattaggagtagcacccaccaaggcaaagagaagagtggtgcagagagaaaaaagagcagtgggaataggagctttgttccttgggttcttgggagcagcaggaagcactatgggcgcagcgtcaatgacgctgacggtacaggccagacaattattgtctggtatagtgcagcagcagaacaatttgctgagggctattgaggcgcaacagcatctgttgcaactcacagtctggggcatcaagcagctccaggcaagaatcctggctgtggaaagatacctaaaggatcaacagctcctggggatttggggttgctctggaaaactcatttgcaccactgctgtgccttggaatgctagttggagtaataaatctctggaacagatttggaatcacacgacctggatggagtgggacagagaaattaacaattacacaagcttaatacactccttaattgaagaatcgcaaaaccagcaagaaaagaatgaacaagaattattggaattagataaatgggcaagtttgtggaattggtttaacataacaaattggctgtggtatataaaattattcataatgatagtaggaggcttggtaggtttaagaatagtttttgctgtactttctatagtgaatagagttaggcagggatattcaccattatcgtttcagacccacctcccaaccccgaggggacccgacaggcccgaaggaatagaagaagaaggtggagagagagacagagacagatccattcgattagtgaacggatctcgacggtatcgcctttaaaagaaaaggggggattggggggtacagtgcaggggaaagaatagtagacataatagcaacagacatacaaactaaagaattacaaaaacaaattacaaaaattcaaaattttcgggtttattacagggacagcagagatccagtttatcgataagcttgggagttccgcgttacataacttacggtaaatggcccgcctggctgaccgcccaacgacccccgcccattgacgtcaataatgacgtatgttcccatagtaacgccaatagggactttccattgacgtcaatgggtggagtatttacggtaaactgcccacttggcagtacatcaagtgtatcatatgccaagtacgccccctattgacgtcaatgacggtaaatggcccgcctggcattatgcccagtacatgaccttatgggactttcctacttggcagtacatctacgtattagtcatcgctattaccatggtgatgcggttttggcagtacatcaatgggcgtggatagcggtttgactcacggggatttccaagtctccaccccattgacgtcaatgggagtttgttttggcaccaaaatcaacgggactttccaaaatgtcgtaacaactccgccccattgacgcaaatgggcggtaggcgtgtacggtgggaggtctatataagcagagctcgtttagtgaaccgtcagatcgcctggagacgccatccacgctgttttgacctccatagaagacaccgactctactagaggatctatttccggtgaattcgccaccatggcctccctgctcttcttctgtggggccttttatctcctgggaaccggttccatggaagctgacatctaccagaccccaagataccttgttatagggacaggaaagaagatcactctggaatgttctcaaaccatgggccatgacaaaatgtactggtatcaacaagatccaggaatggaactacacctcatccactattcctatggagttaattccacagagaagggagatctttcctctgagtcaacagtctccagaataaggacggagcattttcccctgaccctggagtctgccaggccctcacatacctctcagtacctctgtgccagcagtcggacgcccaacattcagtacttcggcgccgggacccggctctcagtgctggaggacctgaaaaacgtgttcccacccgaggtcgctgtgtttgagccatcagaagcagagatctcccacacccaaaaggccacactagtgtgcctggccacaggcttctaccccgaccacgtggagctgagctggtgggtgaatgggaaggaggtgcacagtggggtcagcacagacccgcagcccctcaaggagcagcccgccctcaatgactccagatactgcctgagcagccgcctgagggtctcggccaccttctggcagaacccccgcaaccacttccgctgtcaagtccagttctacgggctctcggagaatgacgagtggacccaggatagggccaaacctgtcacccagatcgtcagcgccgaggcctggggtagagcagactgtggcttcacctccgagtcttaccagcaaggggtcctgtctgccaccatcctctatgagatcttgctagggaaggccaccttgtatgccgtgctggtcagtgccctcgtgctgatggccatggtcaagagaaaggattccagaggcgggagcggagccacgaacttctctctgttaaagcaagcaggagacgtggaagaaaaccccggtcctatgaactcctctctggactttctaattctgatcttaatgtttggaggaactagtggtcaacagctgaatcagagtcctcaatctatgtttatccaggaaggagaagatgtctccatgaactgcacttcttcaagcatatttaacacctggctatggtacaagcaggaacctggggaaggtcctgtcctcttgatagccttatataaggctggtgaattgacctcaaatggaagactgactgctcagtttggtataaccagaaaggacagcttcctgaatatctcagcatccatacctagtgatgtaggcatctacttctgtgctggcacataccagaaagttacctttggaactggaacaaagctccaagtcatcccaaatatccagaaccctgaccctgccgtgtaccagctgagagactctaaatccagtgacaagtctgcatgcctattcaccgattttgattctcaaacaaatgtgtcacaaagtaaggattctgatgtgtatatcacagacaaaactgtgctagacatgaggtctatggacttcaagagcaacagtgctgtggcctggagcaacaaatctgactttgcatgtgcaaacgccttcaacaacagcattattccagaagacaccttcttccccagcccagaaagttcctgtgatgtcaagctggtcgagaaaagctttgaaacagatacgaacctaaactttcaaaacctgtcagtgattgggttccgaatcctcctcctgaaagtggccgggtttaatctgctcatgacgctgcggctgtggtccagctgactcgagggatcccgcccctctccctcccccccccctaacgttactggccgaagccgcttggaataaggccggtgtgcgtttgtctatatgttattttccaccatattgccgtcttttggcaatgtgagggcccggaaacctggccctgtcttcttgacgagcattcctaggggtctttcccctctcgccaaaggaatgcaaggtctgttgaatgtcgtgaaggaagcagttcctctggaagcttcttgaagacaaacaacgtctgtagcgaccctttgcaggcagcggaaccccccacctggcgacaggtgcctctgcggccaaaagccacgtgtataagatacacctgcaaaggcggcacaaccccagtgccacgttgtgagttggatagttgtggaaagagtcaaatggctcacctcaagcgtattcaacaaggggctgaaggatgcccagaaggtaccccattgtatgggatctgatctggggcctcggtgcacatgctttacatgtgtttagtcgaggttaaaaaacgtctaggccccccgaaccacggggacgtggttttcctttgaaaaacacgatgataatatggtgagcaagggcgaggaggataacatggccatcatcaaggagttcatgcgcttcaaggtgcacatggagggctccgtgaacggccacgagttcgagatcgagggcgagggcgagggccgcccctacgagggcacccagaccgccaagctgaaggtgaccaagggtggccccctgcccttcgcctgggacatcctgtcccctcagttcatgtacggctccaaggcctacgtgaagcaccccgccgacatccccgactacttgaagctgtccttccccgagggcttcaagtgggagcgcgtgatgaacttcgaggacggcggcgtggtgaccgtgacccaggactcctccctgcaggacggcgagttcatctacaaggtgaagctgcgcggcaccaacttcccctccgacggccccgtaatgcagaagaagaccatgggctgggaggcctcctccgagcggatgtaccccgaggacggcgccctgaagggcgagatcaagcagaggctgaagctgaaggacggcggccactacgacgctgaggtcaagaccacctacaaggccaagaagcccgtgcagctgcccggcgcctacaacgtcaacatcaagttggacatcacctcccacaacgaggactacaccatcgtggaacagtacgaacgcgccgagggccgccactccaccggcggcatggacgagctgtacaagtgaacgcgtctggaacaatcaacctctggattacaaaatttgtgaaagattgactggtattcttaactatgttgctccttttacgctatgtggatacgctgctttaatgcctttgtatcatgctattgcttcccgtatggctttcattttctcctccttgtataaatcctggttgctgtctctttatgaggagttgtggcccgttgtcaggcaacgtggcgtggtgtgcactgtgtttgctgacgcaacccccactggttggggcattgccaccacctgtcagctcctttccgggactttcgctttccccctccctattgccacggcggaactcatcgccgcctgccttgcccgctgctggacaggggctcggctgttgggcactgacaattccgtggtgttgtcggggaagctgacgtcctttccatggctgctcgcctgtgttgccacctggattctgcgcgggacgtccttctgctacgtcccttcggccctcaatccagcggaccttccttcccgcggcctgctgccggctctgcggcctcttccgcgtcttcgccttcgccctcagacgagtcggatctccctttgggccgcctccccgcctggaattaattctgcagtcgagacctagaaaaacatggagcaatcacaagtagcaatacagcagctaccaatgctgattgtgcctggctagaagcacaagaggaggaggaggtgggttttccagtcacacctcaggtacctttaagaccaatgacttacaaggcagctgtagatcttagccactttttaaaagaaaagaggggactggaagggctaattcactcccaacgaagacaagatatccttgatctgtggatctaccacacacaaggctacttccctgattagcagaactacacaccagggccaggggtcagatatccactgacctttggatggtgctacaagctagtaccagttgagccagataaggtagaagaggccaataaaggagagaacaccagcttgttacaccctgtgagcctgcatgggatggatgacccggagagagaagtgttagagtggaggtttgacagccgcctagcatttcatcacgtggcccgagagctgcatccggagtacttcaagaactgctgatatcgagcttgctacaagggactttccgctggggactttccagggaggcgtggcctgggcgggactggggagtggcgagccctcagatcctgcatataagcagctgctttttgcctgtactgggtctctctggttagaccagatctgagcctgggagctctctggctaactagggaacccactgcttaagcctcaataaagcttgccttgagtgcttcaagtagtgtgtgcccgtctgttgtgtgactctggtaactagagatccctcagacccttttagtcagtgtggaaaatctctagcagtagtagttcatgtcatcttattattcagtatttataacttgcaaagaaatgaatatcagagagtgagaggccttgacattgctagcgtttaccgtcgacctctagctagagcttggcgtaatcatggtcatagctgtttcctgtgtgaaattgttatccgctcacaattccacacaacatacgagccggaagcataaagtgtaaagcctggggtgcctaatgagtgagctaactcacattaattgcgttgcgctcactgcccgctttccagtcgggaaacctgtcgtgccagctgcattaatgaatcggccaacgcgcggggagaggcggtttgcgtattgggcgctcttccgcttcctcgctcactgactcgctgcgctcggtcgttcggctgcggcgagcggtatcagctcactcaaaggcggtaatacggttatccacagaatcaggggataacgcaggaaagaacatgtgagcaaaaggccagcaaaaggccaggaaccgtaaaaaggccgcgttgctggcgtttttccataggctccgcccccctgacgagcatcacaaaaatcgacgctcaagtcagaggtggcgaaacccgacaggactataaagataccaggcgtttccccctggaagctccctcgtgcgctctcctgttccgaccctgccgcttaccggatacctgtccgcctttctcccttcgggaagcgtggcgctttctcatagctcacgctgtaggtatctcagttcggtgtaggtcgttcgctccaagctgggctgtgtgcacgaaccccccgttcagcccgaccgctgcgccttatccggtaactatcgtcttgagtccaacccggtaagacacgacttatcgccactggcagcagccactggtaacaggattagcagagcgaggtatgtaggcggtgctacagagttcttgaagtggtggcctaactacggctacactagaagaacagtatttggtatctgcgctctgctgaagccagttaccttcggaaaaagagttggtagctcttgatccggcaaacaaaccaccgctggtagcggtggtttttttgtttgcaagcagcagattacgcgcagaaaaaaaggatctcaagaagatcctttgatcttttctacggggtctgacgctcagtggaacgaaaactcacgttaagggattttggtcatgagattatcaaaaaggatcttcacctagatccttttaaattaaaaatgaagttttaaatcaatctaaagtatatatgagtaaacttggtctgacagttaccaatgcttaatcagtgaggcacctatctcagcgatctgtctatttcgttcatccatagttgcctgactccccgtcgtgtagataactacgatacgggagggcttaccatctggccccagtgctgcaatgataccgcgagacccacgctcaccggctccagatttatcagcaataaaccagccagccggaagggccgagcgcagaagtggtcctgcaactttatccgcctccatccagtctattaattgttgccgggaagctagagtaagtagttcgccagttaatagtttgcgcaacgttgttgccattgctacaggcatcgtggtgtcacgctcgtcgtttggtatggcttcattcagctccggttcccaacgatcaaggcgagttacatgatcccccatgttgtgcaaaaaagcggttagctccttcggtcctccgatcgttgtcagaagtaagttggccgcagtgttatcactcatggttatggcagcactgcataattctcttactgtcatgccatccgtaagatgcttttctgtgactggtgagtactcaaccaagtcattctgagaatagtgtatgcggcgaccgagttgctcttgcccggcgtcaatacgggataataccgcgccacatagcagaactttaaaagtgctcatcattggaaaacgttcttcggggcgaaaactctcaaggatcttaccgctgttgagatccagttcgatgtaacccactcgtgcacccaactgatcttcagcatcttttactttcaccagcgtttctgggtgagcaaaaacaggaaggcaaaatgccgcaaaaaagggaataagggcgacacggaaatgttgaatactcatactcttcctttttcaatattattgaagcatttatcagggttattgtctcatgagcggatacatatttgaatgtatttagaaaaataaacaaataggggttccgcgcacatttccccgaaaagtgccacctgacgtcgacggatcgggagatcaacttgtttattgcagcttataatggttacaaataaagcaatagcatcacaaatttcacaaataaagcatttttttcactgcattctagttgtggtttgtccaaactcatcaatgtatcttatcatgtctggatcaactggataactcaagctaaccaaaatcatcccaaacttcccaccccataccctattaccactgccaattacctgtggtttcatttactctaaacctgtgattcctctgaattattttcattttaaagaaattgtatttgttaaatatgtactacaaacttagtagt

SEQ ID NO: 31 - protein, 431 aa, Homo sapiens
MPNPRPGKPSAPSLALGPSPGASPSWRAAPKASDLLGARGPGGTFQGRDLRGGAHASSSSLNPMPPSQLQLPTLPLVMVAPSGARLGPLPHLQALLQDRPHFMHQLSTVDAHARTPVLQVHPLESPAMISLTPPTTATGVFSLKARPGLPPGINVASLEWVSREPALLCTFPNPSAPRKDSTLSAVPQSSYPLLANGVCKWPGCEKVFEEPEDFLKHCQADHLLDEKGRAQCLLQREMVQSLEQQLVLEKEKLSAMQAHLAGKMALTKASSVASSDKGSCCIVAAGSQGPVVPAWSGPREAPDSLFAVRRHLWGSHGNSTFPEFLHNMDYFKFHNMRPPFTYATLIRWAILEAPEKQRTLNEIYHWFTRMFAFFRNHPATWKNAIRHNLSLHKCFVRVESEKGAVWTVDELEFRKKRSQRPSRCSNPTPGP

SEQ ID NO: 32 - protein, 825 aa, Homo sapiens
MLDICLEKRVGTTLAAPKCNSSTVRFQGLAEGTKGTMKMDMEDADMTLWTEAEFEEKCTYIVNDHPWDSGADGGTSVQAEASLPRNLLFKYATNSEEVIGVMSKEYIPKGTRFGPLIGEIYTNDTVPKNANRKYFWRIYSRGELHHFIDGFNEEKSNWMRYVNPAHSPREQNLAACQNGMNIYFYTIKPIPANQELLVWYCRDFAERLHYPYPGELTMMNLTQTQSSLKQPSTEKNELCPKNVPKREYSVKEILKLDSNPSKGKDLYRSNISPLTSEKDLDDFRRRGSPEMPFYPRVVYPIRAPLPEDFLKASLAYGIERPTYITRSPIPSSTTPSPSARSSPDQSLKSSSPHSSPGNTVSPVGPGSQEHRDSYAYLNASYGTEGLGSYPGYAPLPHLPPAFIPSYNAHYPKFLLPPYGMNCNGLSAVSSMNGINNFGLFPRLCPVYSNLLGGGSLPHPMLNPTSLPSSLPSDGARRLLQPEHPREVLVPAPHSAFSFTGAAASMKDKACSPTSGSPTAGTAATAEHVVQPKATSAAMAAPSSDEAMNLIKNKRNMTGYKTLPYPLKKQNGKIKYECNVCAKTFGQLSNLKVHLRVHSGERPFKCQTCNKGFTQLAHLQKHYLVHTGEKPHECQVCHKRFSSTSNLKTHLRLHSGEKPYQCKVCPAKFTQFVHLKLHKRLHTRERPHKCSQCHKNYIHLCSLKVHLKGNCAAAPAPGLPLEDLTRINEEIEKFDISDNADRLEDVEDDISVISVVEKEILAVVRKEKEETGLKVSLQRNMGNGLLSSGCSLYESSDLPLMKLPPSNPLPLVPVKVKQETVEPMDP

SEQ ID NO: 33 - protein, 390 aa, Homo sapiens
MPPSGLRLLLLLLPLLWLLVLTPGRPAAGLSTCKTIDMELVKRKRIEAIRGQILSKLRLASPPSQGEVPPGPLPEAVLALYNSTRDRVAGESAEPEPEPEADYYAKEVTRVLMVETHNEIYDKFKQSTHSIYMFFNTSELREAVPEPVLLSRAELRLLRLKLKVEQHVELYQKYSNNSWRYLSNRLLAPSDSPEWLSFDVTGVVRQWLSRGGEIEGFRLSAHCSCDSRDNTLQVDINGFTTGRRGDLATIHGMNRPFLLLMATPLERAQHLQSSRHRRALDTNYCFSSTEKNCCVRQLYIDFRKDLGWKWIHEPKGYHANFCLGPCPYIWSLDTQYSKVLALYNQHNPGASAAPCCVPQALEPLPIVYYVGRKPKVEQLSNMIVRSCKCS

SEQ ID NO: 34 - DNA, 42 bp, synthetic construct
  misc_feature 1..42: note = Description of Artificial Sequence: Synthetic primer
  source 1..42: mol_type = other DNA
cgcagtagcggtaaacggcgatgctgaagtcrcmcagactcc

SEQ ID NO: 35 - DNA, 39 bp, synthetic construct
  misc_feature 1..39: note = Description of Artificial Sequence: Synthetic primer
  source 1..39: mol_type = other DNA
cgcagtagcggtaaacggcgatgcwgmtgttwcccagac

SEQ ID NO: 36 - DNA, 42 bp, synthetic construct
  misc_feature 1..42: note = Description of Artificial Sequence: Synthetic primer
  source 1..42: mol_type = other DNA
cgcagtagcggtaaacggcgacactgragtyacscagacacc

SEQ ID NO: 37 - DNA, 39 bp, synthetic construct
  misc_feature 1..39: note = Description of Artificial Sequence: Synthetic primer
  source 1..39: mol_type = other DNA
cgcagtagcggtaaacggcgaggctggagtcachcaaas

SEQ ID NO: 38 - DNA, 39 bp, synthetic construct
  misc_feature 1..39: note = Description of Artificial Sequence: Synthetic primer
  source 1..39: mol_type = other DNA
cgcagtagcggtaaacggcgagcctggwgtcasycagac

SEQ ID NO: 39 - DNA, 38 bp, synthetic construct
  misc_feature 1..38: note = Description of Artificial Sequence: Synthetic primer
  source 1..38: mol_type = other DNA
cgcagtagcggtaaacggcggtgctggagtykcccagw

SEQ ID NO: 40 - DNA, 38 bp, synthetic construct
  misc_feature 1..38: note = Description of Artificial Sequence: Synthetic primer
  source 1..38: mol_type = other DNA
cgcagtagcggtaaacggcgatgctgrratcacccagr

SEQ ID NO: 41 - DNA, 39 bp, synthetic construct
  misc_feature 1..39: note = Description of Artificial Sequence: Synthetic primer
  source 1..39: mol_type = other DNA
cgcagtagcggtaaacggcgaagctgaagttgcccagtc

SEQ ID NO: 42 - DNA, 39 bp, synthetic construct
  misc_feature 1..39: note = Description of Artificial Sequence: Synthetic primer
  source 1..39: mol_type = other DNA
cgcagtagcggtaaacggcgatgctggagtyatccagtc

SEQ ID NO: 43 - DNA, 38 bp, synthetic construct
  misc_feature 1..38: note = Description of Artificial Sequence: Synthetic primer
  source 1..38: mol_type = other DNA
cgcagtagcggtaaacggcgaagctggagtkrytcagt

SEQ ID NO: 44 - DNA, 39 bp, synthetic construct
  misc_feature 1..39: note = Description of Artificial Sequence: Synthetic primer
  source 1..39: mol_type = other DNA
cgcagtagcggtaaacggcgatgccatggtcatccagaa

SEQ ID NO: 45 - DNA, 39 bp, synthetic construct
  misc_feature 1..39: note = Description of Artificial Sequence: Synthetic primer
  source 1..39: mol_type = other DNA
cgcagtagcggtaaacggcaatgccggcgtcatgcagaa

SEQ ID NO: 46 - DNA, 39 bp, synthetic construct
  misc_feature 1..39: note = Description of Artificial Sequence: Synthetic primer
  source 1..39: mol_type = other DNA
cgcagtagcggtaaacggcgatggtggaatcactcagtc

SEQ ID NO: 47 - DNA, 39 bp, synthetic construct
  misc_feature 1..39: note = Description of Artificial Sequence: Synthetic primer
  source 1..39: mol_type = other DNA
cgcagtagcggtaaacggcagtgctgtcrtctctcaama

SEQ ID NO: 48 - DNA, 39 bp, synthetic construct
  misc_feature 1..39: note = Description of Artificial Sequence: Synthetic primer
  source 1..39: mol_type = other DNA
cgcagtagcggtaaacggcgaagctgacatctaccagac

SEQ ID NO: 49 - DNA, 42 bp, synthetic construct
  misc_feature 1..42: note = Description of Artificial Sequence: Synthetic primer
  source 1..42: mol_type = other DNA
cgcagtagcggtaaacggcgatgtgaaagtracccagarcyc

SEQ ID NO: 50 - DNA, 39 bp, synthetic construct
  misc_feature 1..39: note = Description of Artificial Sequence: Synthetic primer
  source 1..39: mol_type = other DNA
cgcagtagcggtaaacggcacactccaggcacagagata

SEQ ID NO: 51 - DNA, 55 bp, synthetic construct
  misc_feature 1..55: note = Description of Artificial Sequence: Synthetic primer
  source 1..55: mol_type = other DNA
tgctaaaacgctagctgctggttcgtcgaccaaggcagtatctggagtcattgag

SEQ ID NO: 52 - DNA, 19 bp, synthetic construct
  misc_feature 1..19: note = Description of Artificial Sequence: Synthetic primer
  source 1..19: mol_type = other DNA
cgcagtagcggtaaacggc

SEQ ID NO: 53 - DNA, 41 bp, synthetic construct
  misc_feature 1..41: note = Description of Artificial Sequence: Synthetic primer
  source 1..41: mol_type = other DNA
ccagcagctagcgttttagcaggacaaarcmttgascagcc

SEQ ID NO: 54 - DNA, 41 bp, synthetic construct
  misc_feature 1..41: note = Description of Artificial Sequence: Synthetic primer
  source 1..41: mol_type = other DNA
ccagcagctagcgttttagcaaaggaccaagtgtttcagcc

SEQ ID NO: 55 - DNA, 41 bp, synthetic construct
  misc_feature 1..41: note = Description of Artificial Sequence: Synthetic primer
  source 1..41: mol_type = other DNA
ccagcagctagcgttttagcagctcagtcagtgrcycagcc

SEQ ID NO: 56 - DNA, 41 bp, synthetic construct
  misc_feature 1..41: note = Description of Artificial Sequence: Synthetic primer
  source 1..41: mol_type = other DNA
ccagcagctagcgttttagcagatgctaagaccacmcagcc

SEQ ID NO: 57 - DNA, 43 bp, synthetic construct
  misc_feature 1..43: note = Description of Artificial Sequence: Synthetic primer
  source 1..43: mol_type = other DNA
ccagcagctagcgttttagcaagaaaasawstggagcagagtc

SEQ ID NO: 58 - DNA, 41 bp, synthetic construct
  misc_feature 1..41: note = Description of Artificial Sequence: Synthetic primer
  source 1..41: mol_type = other DNA
ccagcagctagcgttttagcaagccaaaagatagaacagaa

SEQ ID NO: 59 - DNA, 41 bp, synthetic construct
  misc_feature 1..41: note = Description of Artificial Sequence: Synthetic primer
  source 1..41: mol_type = other DNA
ccagcagctagcgttttagcagaaaaccaggtggagcacag

SEQ ID NO: 60 - DNA, 41 bp, synthetic construct
  misc_feature 1..41: note = Description of Artificial Sequence: Synthetic primer
  source 1..41: mol_type = other DNA
ccagcagctagcgttttagcagcccagtckgtgasccagcw

SEQ ID NO: 61 - DNA, 41 bp, synthetic construct
  misc_feature 1..41: note = Description of Artificial Sequence: Synthetic primer
  source 1..41: mol_type = other DNA
ccagcagctagcgttttagcaggaaattcagtgryccagay

SEQ ID NO: 62 - DNA, 44 bp, synthetic construct
  misc_feature 1..44: note = Description of Artificial Sequence: Synthetic primer
  source 1..44: mol_type = other DNA
ccagcagctagcgttttagcacagaaggaggtggagcagratyc

SEQ ID NO: 63 - DNA, 41 bp, synthetic construct
  misc_feature 1..41: note = Description of Artificial Sequence: Synthetic primer
  source 1..41: mol_type = other DNA
ccagcagctagcgttttagcaggagagartgtggrgcwgca

SEQ ID NO: 64 - DNA, 41 bp, synthetic construct
  misc_feature 1..41: note = Description of Artificial Sequence: Synthetic primer
  source 1..41: mol_type = other DNA
ccagcagctagcgttttagcagcccagaagrtwactcaarc

SEQ ID NO: 65 - DNA, 41 bp, synthetic construct
  misc_feature 1..41: note = Description of Artificial Sequence: Synthetic primer
  source 1..41: mol_type = other DNA
ccagcagctagcgttttagcagcccagasagtsactcagyc

SEQ ID NO: 66 - DNA, 41 bp, synthetic construct
  misc_feature 1..41: note = Description of Artificial Sequence: Synthetic primer
  source 1..41: mol_type = other DNA
ccagcagctagcgttttagcaagtcaacagggagaagagga

SEQ ID NO: 67 - DNA, 41 bp, synthetic construct
  misc_feature 1..41: note = Description of Artificial Sequence: Synthetic primer
  source 1..41: mol_type = other DNA
ccagcagctagcgttttagcaggagactcggttacccagac

SEQ ID NO: 68 - DNA, 44 bp, synthetic construct
  misc_feature 1..44: note = Description of Artificial Sequence: Synthetic primer
  source 1..44: mol_type = other DNA
ccagcagctagcgttttagcaaaacaggaggtgacgcagaktcc

SEQ ID NO: 69 - DNA, 41 bp, synthetic construct
  misc_feature 1..41: note = Description of Artificial Sequence: Synthetic primer
  source 1..41: mol_type = other DNA
ccagcagctagcgttttagcaggccaacagaaggagaaaag

SEQ ID NO: 70 - DNA, 41 bp, synthetic construct
  misc_feature 1..41: note = Description of Artificial Sequence: Synthetic primer
  source 1..41: mol_type = other DNA
ccagcagctagcgttttagcagagctgaamgtggaacaaar

SEQ ID NO: 71 - DNA, 41 bp, synthetic construct
  misc_feature 1..41: note = Description of Artificial Sequence: Synthetic primer
  source 1..41: mol_type = other DNA
ccagcagctagcgttttagcaggacaacaggtaatgcaaat

SEQ ID NO: 72 - DNA, 41 bp, synthetic construct
  misc_feature 1..41: note = Description of Artificial Sequence: Synthetic primer
  source 1..41: mol_type = other DNA
ccagcagctagcgttttagcaacccagctgctggagcagag

SEQ ID NO: 73 - DNA, 41 bp, synthetic construct
  misc_feature 1..41: note = Description of Artificial Sequence: Synthetic primer
  source 1..41: mol_type = other DNA
ccagcagctagcgttttagcaagtcaacagaagaatgatga

SEQ ID NO: 74 - DNA, 41 bp, synthetic construct
  misc_feature 1..41: note = Description of Artificial Sequence: Synthetic primer
  source 1..41: mol_type = other DNA
ccagcagctagcgttttagcacaacaaccagtgcagagtcc

SEQ ID NO: 75 - DNA, 41 bp, synthetic construct
  misc_feature 1..41: note = Description of Artificial Sequence: Synthetic primer
  source 1..41: mol_type = other DNA
ccagcagctagcgttttagcaggtcaacagctgaatcagag

SEQ ID NO: 76 - DNA, 41 bp, synthetic construct
  misc_feature 1..41: note = Description of Artificial Sequence: Synthetic primer
  source 1..41: mol_type = other DNA
ccagcagctagcgttttagcagaagacaaggtggtacaaag

SEQ ID NO: 77 - DNA, 41 bp, synthetic construct
  misc_feature 1..41: note = Description of Artificial Sequence: Synthetic primer
  source 1..41: mol_type = other DNA
ccagcagctagcgttttagcaagcaattcagtcaagcagac

SEQ ID NO: 78 - DNA, 20 bp, synthetic construct
  misc_feature 1..20: note = Description of Artificial Sequence: Synthetic primer
  source 1..20: mol_type = other DNA
cgaccagcttgacatcacag

SEQ ID NO: 79 - protein, 9 aa, Epstein-Barr virus
FLRGRAYGL